European Patent Application EP 4 183 408 A1, published May 24, 2023. Title: COMBINED ENTEROTOXIGENIC ESCHERICHIA COLI AND SHIGELLA. Applicant: THE UNITED STATES OF AMERICA AS REPRESENTED BY THE SECRETARY OF THE NAVY. Application EP. The sequence listing filed with the application follows.

SEQUENCE LISTING (143 sequences)

SEQ ID NO: 1 - protein, 414 aa, Escherichia coli
ATGAGAACAGAAATAGCGACTAAAAACTTCCCAGTATCAACGACTATTTCAAAAAGTTTTTTTGCGCCTGAACCACAAATCCAGCCTTCTTTTGGTAAAAATGTTGGAAAGGAAGGAGATTTATTATTTAGTGTGAGCTTAATTGTTCCTGAAAATGTATCCCAGGTAACGGTCTACCCTGTTTATGATGAAGATTATGGATTAGGACGACTCGTAAATACCGCTGATGATTCCCAATCAATAATCTACCAGATTGTTGATGATAAAGGGAAAAAAATGTTAAAAGATCATGGTACAGAGGTTACGCCTAATCAACAAATAACTTTTAAAGCGCTGAATTATACTAGCGGAGATAAAGAAATACCTCCTGGGATATATAACGATCAGGTTATGGTTGGTTACTATGTAAACTAA

SEQ ID NO: 2 - protein, 137 aa, Escherichia coli
MRTEIATKNFPVSTTISKSFFAPEPQIQPSFGKNVGKEGDLLFSVSLIVPENVSQVTVYPVYDEDYGLGRLVNTADDSQSIIYQIVDDKGKKMLKDHGTEVTPNQQITFKALNYTSGDKEIPPGIYNDQVMVGYYVN

SEQ ID NO: 3 - protein, 444 aa, Escherichia coli
ATGGGAAACTGGCAATATAAATCTCTGGATGTAAATGTAAATATTGAGCAAAATTTTATTCCAGATATTGATTCCGCTGTTCGTATAATACCTGTTAATTACGATTCGGATCCGAAACTGAATTCACAGTTATATACGGTTGAGATGACGATCCCTGCAGGTGTAAGCGCAGTTAAAATCGTACCAACAGATAGTCTGACATCTTCTGGACAGCAGATCGGAAAGCTGGTTAATGTAAACAATCCAGATCAAAATATGAATTATTATATCAGAAAGGATTCTGGCGCTGGTAAGTTTATGGCAGGGCAAAAAGGATCCTTTTCTGTCAAAGAGAATACGTCATACACATTCTCAGCAATTTATACTGGTGGCGAATACCCTAATAGCGGATATTCGTCTGGTACTTATGCAGGACATTTGACTGTATCATTTTACAGCAATTAA

SEQ ID NO: 4 - protein, 147 aa, Escherichia coli
MGNWQYKSLDVNVNIEQNFIPDIDSAVRIIPVNYDSDPKLNSQLYTVEMTIPAGVSAVKIVPTDSLTSSGQQIGKLVNVNNPDQNMNYYIRKDSGAGKFMAGQKGSFSVKENTSYTFSAIYTGGEYPNSGYSSGTYAGHLTVSFYSN

SEQ ID NO: 5 - protein, 4 aa, Escherichia coli
DNKQ

SEQ ID NO: 6 - DNA, 2502 bp, Escherichia coli
  source 1..2502: mol_type = unassigned DNA
atgaataaaattttatttatttttacattgtttttttcttcagggttttttacatttgccgtatcggcagataaaaatcccggaagtgaaaacatgactaatactattggtccccatgacagggggggatcttcccccatatataatatcttaaattcctatcttacagcatacaatggaagccatcatctgtatgataggatgagttttttatgtttgtcttctcaaaatacactgaatggagcatgcccaagcagtgatgcccctggcactgctacaattgatggcgaaacaaatataacattacaatttacggaaaaaagaagtctaattaaaagagaactgcaaattaaaggctataaacaatttttgttcaaaaatgctaattgcccatctaaactagcacttaactcatctcattttcaatgtaatagagaacaagcttcaggtgctactttatcgttatacataccagctggtgaattaaataaattaccttttgggggggtctggaatgccgttctgaagctaaatgtaaaaagacgatatgatacaacctatgggacttacactataaacatcacagttaatttaactgataagggaaatattcagatatggttaccacagttcaaaagtaacgctcgtgtcgatcttaacttgcgtccaactggtggtggtacatatatcggaagaaattctgttgatatgtgcttttatgatggatatagtactaacagcagctctttagagataagatttcaggatgataattctaaatctgatggaaaattttatctaaagaaaataaatgatgactccaaagaacttgtatacactttgtcacttctcctggcaggtaaaaatttaacaccaacaaatggacaggcattaaatattaacactgcttctctggaaacaaactggaatagaattacagctgtcaccatgccagaaatcagtgttccggtgttgtgttggcctggacgtttgcaattggatgcaaaagtgaaaaatcccgaggctggacaatatatggggaatattaaaattactttcacaccaagtagtcaaacactcgacaataaacaagtagagaaaaatattactgtaacagctagtgttgatcctgcaattgatcttttgcaagctgatggcaatgctctgccatcagctgtaaagttagcttattctcccgcatcaaaaacttttgaaagttacagagtaatgactcaagttcatacaaacgatgcaactaaaaaagtaattgttaaacttgctgatacaccacagcttacagatgttctgaattcaactgttcaaatgcctatcagtgtgtcatggggaggacaagtattatctacaacagccaaagaatttgaagctgctgctttgggatattctgcatccggtgtaaatggcgtatcatcttctcaagagttagtaattagcgctgcacctaaaactgccggtaccgccccaactgcaggaaactattcaggagtagtatctcttgtaatgactttgggatccgacaataaacaagtagagaaaaatattactgtaacagctagtgtcgaccctgcagggacattagctattgattttacgcctattgaaaatatttatgtaggtgccaattatggtaaagatattggaacccttgttttcacaacaaatgatttaacagatattacattgatgtcatctcgcagcgttgttgatggtcgccagactggtttttttaccttcatggactcatcagccacttacaaaattagtacaaaactgggatcatcgaatgatgtaaacattcaagaaattactcaaggagctaaaattactcctgttagtggagagaaaactttgcctaaaaaattcactcttaagctacatgcacacaggagtagcagtacagttccaggtacgtatactgttggtcttaacgtaaccagtaacgttattgataacaagcaggcagcggggcccactctaaccaaagaactggcattaaatgtgctttctcctgcagctctggatgcaacttgggctcctcaggataatttaacattatccaatactggcgtttctaatactttggtgggtgttttgactctttcaaataccagtattgatacagttagcattgcgagtacaaatgtttctgatacatctaagaatggtacagtaacttttgcacatgagacaaataactctgctagctttgccaccaccatttcaacagataatgccaacattacgttggataaaaatgctggaaatacgattgttaaaactacaaatgggagtcagttgccaactaatttaccacttaagtttattaccactgaaggtaacgaacatttagtttcaggtaattaccgtgcaaatataacaattacttcgacaattaaagataacaagcaggcggcaggtccaaccctgactaaggagttagcgctgaacgttctgagcctcgagcaccaccaccaccaccactga

SEQ ID NO: 7 - protein, 833 aa, Escherichia coli
MNKILFIFTLFFSSGFFTFAVSADKNPGSENMTNTIGPHDRGGSSPIYNILNSYLTAYNGSHHLYDRMSFLCLSSQNTLNGACPSSDAPGTATIDGETNITLQFTEKRSLIKRELQIKGYKQFLFKNANCPSKLALNSSHFQCNREQASGATLSLYIPAGELNKLPFGGVWNAVLKLNVKRRYDTTYGTYTINITVNLTDKGNIQIWLPQFKSNARVDLNLRPTGGGTYIGRNSVDMCFYDGYSTNSSSLEIRFQDDNSKSDGKFYLKKINDDSKELVYTLSLLLAGKNLTPTNGQALNINTASLETNWNRITAVTMPEISVPVLCWPGRLQLDAKVKNPEAGQYMGNIKITFTPSSQTLDNKQVEKNITVTASVDPAIDLLQADGNALPSAVKLAYSPASKTFESYRVMTQVHTNDATKKVIVKLADTPQLTDVLNSTVQMPISVSWGGQVLSTTAKEFEAAALGYSASGVNGVSSSQELVISAAPKTAGTAPTAGNYSGVVSLVMTLGSDNKQVEKNITVTASVDPAGTLAIDFTPIENIYVGANYGKDIGTLVFTTNDLTDITLMSSRSVVDGRQTGFFTFMDSSATYKISTKLGSSNDVNIQEITQGAKITPVSGEKTLPKKFTLKLHAHRSSSTVPGTYTVGLNVTSNVIDNKQAAGPTLTKELALNVLSPAALDATWAPQDNLTLSNTGVSNTLVGVLTLSNTSIDTVSIASTNVSDTSKNGTVTFAHETNNSASFATTISTDNANITLDKNAGNTIVKTTNGSQLPTNLPLKFITTEGNEHLVSGNYRANITITSTIKDNKQAAGPTLTKELALNVLSLEHHHHHH

SEQ ID NO: 8 - DNA, 3414 bp, Escherichia coli
  source 1..3414: mol_type = unassigned DNA
atgaataaaattttatttatttttacattgtttttttcttcagggttttttacatttgccgtatcggcagataaaaatcccggaagtgaaaacatgactaatactattggtccccatgacagggggggatcttcccccatatataatatcttaaattcctatcttacagcatacaatggaagccatcatctgtatgataggatgagttttttatgtttgtcttctcaaaatacactgaatggagcatgcccaagcagtgatgcccctggcactgctacaattgatggcgaaacaaatataacattacaatttacggaaaaaagaagtctaattaaaagagaactgcaaattaaaggctataaacaatttttgttcaaaaatgctaattgcccatctaaactagcacttaactcatctcattttcaatgtaatagagaacaagcttcaggtgctactttatcgttatacataccagctggtgaattaaataaattaccttttgggggggtctggaatgccgttctgaagctaaatgtaaaaagacgatatgatacaacctatgggacttacactataaacatcacagttaatttaactgataagggaaatattcagatatggttaccacagttcaaaagtaacgctcgtgtcgatcttaacttgcgtccaactggtggtggtacatatatcggaagaaattctgttgatatgtgcttttatgatggatatagtactaacagcagctctttagagataagatttcaggatgataattctaaatctgatggaaaattttatctaaagaaaataaatgatgactccaaagaacttgtatacactttgtcacttctcctggcaggtaaaaatttaacaccaacaaatggacaggcattaaatattaacactgcttctctggaaacaaactggaatagaattacagctgtcaccatgccagaaatcagtgttccggtgttgtgttggcctggacgtttgcaattggatgcaaaagtgaaaaatcccgaggctggacaatatatggggaatattaaaattactttcacaccaagtagtcaaacactcgacaataaacaagtagagaaaaatattactgtaacagctagtgttgatcctgcaattgatcttttgcaagctgatggcaatgctctgccatcagctgtaaagttagcttattctcccgcatcaaaaacttttgaaagttacagagtaatgactcaagttcatacaaacgatgcaactaaaaaagtaattgttaaacttgctgatacaccacagcttacagatgttctgaattcaactgttcaaatgcctatcagtgtgtcatggggaggacaagtattatctacaacagccaaagaatttgaagctgctgctttgggatattctgcatccggtgtaaatggcgtatcatcttctcaagagttagtaattagcgctgcacctaaaactgccggtaccgccccaactgcaggaaactattcaggagtagtatctcttgtaatgactttgggatccgacaataaacaagtagagaaaaatattactgtaacagctagtgtcgaccctactattgatattcttcaagcaaatggttctgcgctaccgacagctgtagatttaacttatctacctggtgcaaaaacttttgaaaattacagtgttctaacccagatttacacaaatgacccttcaaaaggtttagatgttcgactggttgatacaccgaaacttacaaatattttgcaaccgacatctaccattcctcttactgtctcatgggcagggaagacattaagtacaagtgctcagaagattgcagttggcgatctgggttttggttccaccggaacggcaggtgtttcgaatagtaaagaattagtaattggagcaactacatccggaactgcaccaagtgcaggtaagtatcaaggcgtcgtttccattgtaatgactcaatcgaccgacacagccgcgcctgttcctgacaataaacaagtagagaaaaatattactgtgacagccagtgttgatcctactattgacattttgcaagctgatggtagtagtttacctactgctgtagaattaacctattcacctgcggcaagtcgttttgaaaattataaaatcgcaactaaagttcatacaaatgttataaataaaaatgtactagttaagcttgtaaatgatccaaaacttacaaatgttttggattctacaaaacaactccccattactgtatcatatggaggaaagactctatcaaccgcagatgtgacttttgaacctgcagaattaaattttggaacgtcaggtgtaactggtgtatcttcttcccaagatttagtgattggtgcgactacagcacaagcaccaacggcgggaaattatagtggggtcgtttctatcttaatgaccttagcatcagacaataaacaagtggaaaaaaatatcactgtaacagctagtgttgatcctacgggcacattagctattgattttacgcctattgaaaatatttatgtaggtgccaattatggtaaagatattggaacccttgttttcacaacaaatgatttaacagatattacattgatgtcatctcgcagcgttgttgatggtcgccagactggtttttttaccttcatggactcatcagccacttacaaaattagtacaaaactgggatcatcgaatgatgtaaacattcaagaaattactcaaggagctaaaattactcctgttagtggagagaaaactttgcctaaaaaattcactcttaagctacatgcacacaggagtagcagtacagttccaggtacgtatactgttggtcttaacgtaaccagtaacgttattgataacaagcaggcagcggggcccactctaaccaaagaactggcattaaatgtgctttctcctgcagctctggatgcaacttgggctcctcaggataatttaacattatccaatactggcgtttctaatactttggtgggtgttttgactctttcaaataccagtattgatacagttagcattgcgagtacaaatgtttctgatacatctaagaatggtacagtaacttttgcacatgagacaaataactctgctagctttgccaccaccatttcaacagataatgccaacattacgttggataaaaatgctggaaatacgattgttaaaactacaaatgggagtcagttgccaactaatttaccacttaagtttattaccactgaaggtaacgaacatttagtttcaggtaattaccgtgcaaatataacaattacttcgacaattaaagataacaagcaggcggcaggtccaaccctgactaaggagttagcgctgaacgttctgagcctcgagcaccaccaccaccaccactga

SEQ ID NO: 9 - protein, 1137 aa, Escherichia coli
MNKILFIFTLFFSSGFFTFAVSADKNPGSENMTNTIGPHDRGGSSPIYNILNSYLTAYNGSHHLYDRMSFLCLSSQNTLNGACPSSDAPGTATIDGETNITLQFTEKRSLIKRELQIKGYKQFLFKNANCPSKLALNSSHFQCNREQASGATLSLYIPAGELNKLPFGGVWNAVLKLNVKRRYDTTYGTYTINITVNLTDKGNIQIWLPQFKSNARVDLNLRPTGGGTYIGRNSVDMCFYDGYSTNSSSLEIRFQDDNSKSDGKFYLKKINDDSKELVYTLSLLLAGKNLTPTNGQALNINTASLETNWNRITAVTMPEISVPVLCWPGRLQLDAKVKNPEAGQYMGNIKITFTPSSQTLDNKQVEKNITVTASVDPAIDLLQADGNALPSAVKLAYSPASKTFESYRVMTQVHTNDATKKVIVKLADTPQLTDVLNSTVQMPISVSWGGQVLSTTAKEFEAAALGYSASGVNGVSSSQELVISAAPKTAGTAPTAGNYSGVVSLVMTLGSDNKQVEKNITVTASVDPTIDILQANGSALPTAVDLTYLPGAKTFENYSVLTQIYTNDPSKGLDVRLVDTPKLTNILQPTSTIPLTVSWAGKTLSTSAQKIAVGDLGFGSTGTAGVSNSKELVIGATTSGTAPSAGKYQGVVSIVMTQSTDTAAPVPDNKQVEKNITVTASVDPTIDILQADGSSLPTAVELTYSPAASRFENYKIATKVHTNVINKNVLVKLVNDPKLTNVLDSTKQLPITVSYGGKTLSTADVTFEPAELNFGTSGVTGVSSSQDLVIGATTAQAPTAGNYSGVVSILMTLASDNKQVEKNITVTASVDPTGTLAIDFTPIENIYVGANYGKDIGTLVFTTNDLTDITLMSSRSVVDGRQTGFFTFMDSSATYKISTKLGSSNDVNIQEITQGAKITPVSGEKTLPKKFTLKLHAHRSSSTVPGTYTVGLNVTSNVIDNKQAAGPTLTKELALNVLSPAALDATWAPQDNLTLSNTGVSNTLVGVLTLSNTSIDTVSIASTNVSDTSKNGTVTFAHETNNSASFATTISTDNANITLDKNAGNTIVKTTNGSQLPTNLPLKFITTEGNEHLVSGNYRANITITSTIKDNKQAAGPTLTKELALNVLSLEHHHHHH

SEQ ID NO: 10 - DNA, 2952 bp, Escherichia coli
  source 1..2952: mol_type = unassigned DNA
atgaaaaagatatttatttttttgtctatcatattttctgcggtggtcagtgccgggcgatacccggaaactacagtaggtaatctgacgaagagttttcaagcccctcgtcaggatagaagcgtacaatcaccaatatataacatctttacgaatcatgtggctggatatagtttgagtcataacttatatgacaggattgtttttttatgtacatcctcgtcgaatccggttaatggtgcttgcccaaccattggaacatctggagttcaatacggtactacaaccataaccttgcagtttacagaaaaaagaagtctgataaaaagaaatattaatcttgcaggtaataagaaaccaatatgggagaatcagagttgcgacactagcaatctaatggtgttgaattcgaagtcttggtcctgtggggcttacggaaatgctaacggaacacttctaaatctgtatatccctgcaggagaaatcaacaaattgccttttggagggatatgggaggcaactctgatcttacgcttatcaagatatggcgaagtcagtagcacccattacggcaattataccgtaaatattacggttgatttaactgataaaggtaatattcaggtatggcttccagggtttcacagcaacccgcgtgtagacctgaatctgcaccctatcggtaattataaatatagtggtagtaattcactcgacatgtgtttctatgatggatatagtacaaacagtgatagcatggtaataaagttccaggatgataatcctacctattcatctgaatataatctttataagatagggggcactgaaaaattaccctatgctgtttcactgcttatgggagaaaaaatattttatccagtgaatggtcaatcatttactatcaatgacagtagtgtactcgaaacaaactggaatcgagtaaccgcagttgctatgccggaagttaatgttccagtattatgctggccagcaagattgctattaaatgctgatgtaaatgctcccgatgcaggacagtattcaggacagatatatataacatttacacccagtgtcgaaaatttaggcggtggagtcgaaaaaaatattactgtgagggcaagtgttgaccctaaacttgatcttctgcaagcagatggaacttcactgccggactctatcgcattaacctattcttcggcttcaaataattttgaagtttactctcttaatactgctattcatacaaatgacaaaagcaagggagttgtagtgaagctgtcagcttcaccagttctgtccaatattatgaagccaaactcgcaaattccgatgaaagtgactttgggggggaagacgctgaatacaactgatactgagtttactgttgatactctgaactttggtacatctggtgttgaaaacgtttcttccactcaacagcttacgattcatgcagacacacaaggaactgcgcctgaggcaggcaattaccaaggtattatttctcttatcatgactcaaaaaacagggggcggtgtcgaaaaaaatattactgtgagggcaagtgtcgaccctaaacttgaccttctgcaatctgatggctctgcgctgccgaactctgtcgcattaacctattctccggctgtaaataattttgaagctcacaccatcaacaccgttgttcatacaaatgactcagataaaggtgttgttgtgaagctgtcagcagatccagtcctgtccaatgttctgaatccaaccctgcaaattcctgtttctgtgaatttcgcaggaaaaccactgagcacaacaggcattaccatcgactccaatgatctgaactttgcttcgagtggtgttaataaagtttcttctacgcagaaactttcaatccatgcagatgctactcgggtaactggcggcgcactaacagctggtcaatatcagggactcgtatcaattatcctgactaagtcaacggggggcggtgtcgagaagaccattagcgttacggcgagtgttgacccgacgggcacattagctattgattttacgcctattgaaaatatttatgtaggtgccaattatggtaaagatattggaacccttgttttcacaacaaatgatttaacagatattacattgatgtcatctcgcagcgttgttgatggtcgccagactggtttttttaccttcatggactcatcagccacttacaaaattagtacaaaactgggatcatcgaatgatgtaaacattcaagaaattactcaaggagctaaaattactcctgttagtggagagaaaactttgcctaaaaaattcactcttaagctacatgcacacaggagtagcagtacagttccaggtacgtatactgttggtcttaacgtaaccagtaacgttattgataacaagcaggcagcggggcccactctaaccaaagaactggcattaaatgtgctttctcctgcagctctggatgcaacttgggctcctcaggataatttaacattatccaatactggcgtttctaatactttggtgggtgttttgactctttcaaataccagtattgatacagttagcattgcgagtacaaatgtttctgatacatctaagaatggtacagtaacttttgcacatgagacaaataactctgctagctttgccaccaccatttcaacagataatgccaacattacgttggataaaaatgctggaaatacgattgttaaaactacaaatgggagtcagttgccaactaatttaccacttaagtttattaccactgaaggtaacgaacatttagtttcaggtaattaccgtgcaaatataacaattacttcgacaattaaagataacaagcaggcggcaggtccaaccctgactaaggagttagcgctgaacgttctgagcctcgagcaccaccaccaccaccactga

SEQ ID NO: 11 - protein, 983 aa, Escherichia coli
MKKIFIFLSIIFSAVVSAGRYPETTVGNLTKSFQAPRQDRSVQSPIYNIFTNHVAGYSLSHNLYDRIVFLCTSSSNPVNGACPTIGTSGVQYGTTTITLQFTEKRSLIKRNINLAGNKKPIWENQSCDTSNLMVLNSKSWSCGAYGNANGTLLNLYIPAGEINKLPFGGIWEATLILRLSRYGEVSSTHYGNYTVNITVDLTDKGNIQVWLPGFHSNPRVDLNLHPIGNYKYSGSNSLDMCFYDGYSTNSDSMVIKFQDDNPTYSSEYNLYKIGGTEKLPYAVSLLMGEKIFYPVNGQSFTINDSSVLETNWNRVTAVAMPEVNVPVLCWPARLLLNADVNAPDAGQYSGQIYITFTPSVENLGGGVEKNITVRASVDPKLDLLQADGTSLPDSIALTYSSASNNFEVYSLNTAIHTNDKSKGVVVKLSASPVLSNIMKPNSQIPMKVTLGGKTLNTTDTEFTVDTLNFGTSGVENVSSTQQLTIHADTQGTAPEAGNYQGIISLIMTQKTGGGVEKNITVRASVDPKLDLLQSDGSALPNSVALTYSPAVNNFEAHTINTVVHTNDSDKGVVVKLSADPVLSNVLNPTLQIPVSVNFAGKPLSTTGITIDSNDLNFASSGVNKVSSTQKLSIHADATRVTGGALTAGQYQGLVSIILTKSTGGGVEKTISVTASVDPTGTLAIDFTPIENIYVGANYGKDIGTLVFTTNDLTDITLMSSRSVVDGRQTGFFTFMDSSATYKISTKLGSSNDVNIQEITQGAKITPVSGEKTLPKKFTLKLHAHRSSSTVPGTYTVGLNVTSNVIDNKQAAGPTLTKELALNVLSPAALDATWAPQDNLTLSNTGVSNTLVGVLTLSNTSIDTVSIASTNVSDTSKNGTVTFAHETNNSASFATTISTDNANITLDKNAGNTIVKTTNGSQLPTNLPLKFITTEGNEHLVSGNYRANITITSTIKDNKQAAGPTLTKELALNVLSLEHHHHHH

SEQ ID NO: 12 - DNA, 2514 bp, Escherichia coli
  source 1..2514: mol_type = unassigned DNA
atgaaaaaagtgatttttgttttatccatgtttctatgttctcaggtttacgggcaatcatggcatacgaacgtagaggctggttcaataaataaaacagagtcgataggccccatagaccgaagtgctgctgcatcgtatcctgctcattatatatttcatgaacatgttgctggttacaataaagatcactctctttttgacaggatgacgtttttatgtatgtcatcaacagatgcatctaaaggtgcatgtccgacaggagaaaactccaaatcctctcaaggggagactaatattaagctaatatttactgaaaagaaaagtctggccagaaaaacattaaacttaaaaggatataagagatttttatatgaatcagatagatgcattcattatgtcgataaaatgaatctcaattctcatactgttaaatgtgtaggttcattcacaagaggagtagatttcactttatatatcccacaaggtgaaattgatgggcttctaactggaggtatatgggaggcaacactagagttacgagtcaaaaggcattacgactataatcatggtacttacaaagttaatatcacagttgatttgacagacaaaggaaatattcaggtctggacaccaaagtttcatagcgatcctagaattgatctgaatttacgtcctgaaggtaatggtaaatattctggtagtaacgtgcttgagatgtgtctctatgatggctatagtacacatagtcaaagtatagaaatgaggtttcaggatgactcacaaacaggaaataatgaatataatcttataaaaactggagagccattaaaaaaattgccatataaactttctcttcttttaggaggacgagagttttatccaaataatggagaggcttttactattaatgatacttcgtcattgtttataaactggaatcgtattaagtctgtatccttaccacagattagtattccagtactatgctggccagcaaacttgacatttatgtcagagctaaataatccagaagcgggtgagtattcaggaatacttaacgtaacatttactcctagtagttcaagcctagacaataaacaagccgagaaaaatatcactgtaactgctagcgttgatccaactatcgatctgatgcaatctgatggcacagcgttaccaagtgcagttaatattgcatatcttccaggagagaaaagatttgaatctgctcgtatcaatacccaagttcataccaataataaaactaagggtattcagataaagcttactaatgataatgtggtaatgactaacttatctgatccaagcaagactattcctttagaggtttcattcgctggcactaagctgagcacagctgcaacatctattactgccgatcaattaaattttggcgcagctggtgtagagacagtttctgcaactaaggaactcgttattaatgcaggaagcacccagcaaactaatattgtagctggtaactatcaaggattggtgtcaattgtgcttactcaagaacctgacaataaacaagccgagaaaaatatcactgtaactgctagcgttgatccgacgggcacattagctattgattttacgcctattgaaaatatttatgtaggtgccaattatggtaaagatattggaacccttgttttcacaacaaatgatttaacagatattacattgatgtcatctcgcagcgttgttgatggtcgccagactggtttttttaccttcatggactcatcagccacttacaaaattagtacaaaactgggatcatcgaatgatgtaaacattcaagaaattactcaaggagctaaaattactcctgttagtggagagaaaactttgcctaaaaaattcactcttaagctacatgcacacaggagtagcagtacagttccaggtacgtatactgttggtcttaacgtaaccagtaacgttattgataacaagcaggcagcggggcccactctaaccaaagaactggcattaaatgtgctttctcctgcagctctggatgcaacttgggctcctcaggataatttaacattatccaatactggcgtttctaatactttggtgggtgttttgactctttcaaataccagtattgatacagttagcattgcgagtacaaatgtttctgatacatctaagaatggtacagtaacttttgcacatgagacaaataactctgctagctttgccaccaccatttcaacagataatgccaacattacgttggataaaaatgctggaaatacgattgttaaaactacaaatgggagtcagttgccaactaatttaccacttaagtttattaccactgaaggtaacgaacatttagtttcaggtaattaccgtgcaaatataacaattacttcgacaattaaagataacaagcaggcggcaggtccaaccctgactaaggagttagcgctgaacgttctgagcctcgagcaccaccaccaccaccactga

SEQ ID NO: 13 - protein, 837 aa, Escherichia coli
MKKVIFVLSMFLCSQVYGQSWHTNVEAGSINKTESIGPIDRSAAASYPAHYIFHEHVAGYNKDHSLFDRMTFLCMSSTDASKGACPTGENSKSSQGETNIKLIFTEKKSLARKTLNLKGYKRFLYESDRCIHYVDKMNLNSHTVKCVGSFTRGVDFTLYIPQGEIDGLLTGGIWEATLELRVKRHYDYNHGTYKVNITVDLTDKGNIQVWTPKFHSDPRIDLNLRPEGNGKYSGSNVLEMCLYDGYSTHSQSIEMRFQDDSQTGNNEYNLIKTGEPLKKLPYKLSLLLGGREFYPNNGEAFTINDTSSLFINWNRIKSVSLPQISIPVLCWPANLTFMSELNNPEAGEYSGILNVTFTPSSSSLDNKQAEKNITVTASVDPTIDLMQSDGTALPSAVNIAYLPGEKRFESARINTQVHTNNKTKGIQIKLTNDNVVMTNLSDPSKTIPLEVSFAGTKLSTAATSITADQLNFGAAGVETVSATKELVINAGSTQQTNIVAGNYQGLVSIVLTQEPDNKQAEKNITVTASVDPTGTLAIDFTPIENIYVGANYGKDIGTLVFTTNDLTDITLMSSRSVVDGRQTGFFTFMDSSATYKISTKLGSSNDVNIQEITQGAKITPVSGEKTLPKKFTLKLHAHRSSSTVPGTYTVGLNVTSNVIDNKQAAGPTLTKELALNVLSPAALDATWAPQDNLTLSNTGVSNTLVGVLTLSNTSIDTVSIASTNVSDTSKNGTVTFAHETNNSASFATTISTDNANITLDKNAGNTIVKTTNGSQLPTNLPLKFITTEGNEHLVSGNYRANITITSTIKDNKQAAGPTLTKELALNVLSLEHHHHHH

SEQ ID NO: 14 - DNA, 1845 bp, Escherichia coli
  source 1..1845: mol_type = unassigned DNA
atggcagtgggcccaacgaaagatatgagtttaggtgcaaatttaacttcagagcctacattagctattgattttacgcctattgaaaatatttatgtaggtgccaattatggtaaagatattggaacccttgttttcacaacaaatgatttaacagatattacattgatgtcatctcgcagcgttgttgatggtcgccagactggtttttttaccttcatggactcatcagccacttacaaaattagtacaaaactgggatcatcgaatgatgtaaacattcaagaaattactcaaggagctaaaattactcctgttagtggagagaaaactttgcctaaaaaattcactcttaagctacatgcacacaggagtagcagtacagttccaggtacgtatactgttggtcttaacgtaaccagtaacgttattgataacaagcaggcagcggggcccactctaaccaaagaactggcattaaatgtgctttctcctgcagctctggatgcaacttgggctcctcaggataatttaacattatccaatactggcgtttctaatactttggtgggtgttttgactctttcaaataccagtattgatacagttagcattgcgagtacaaatgtttctgatacatctaagaatggtacagtaacttttgcacatgagacaaataactctgctagctttgccaccaccatttcaacagataatgccaacattacgttggataaaaatgctggaaatacgattgttaaaactacaaatgggagtcagttgccaactaatttaccacttaagtttattaccactgaaggtaacgaacatttagtttcaggtaattaccgtgcaaatataacaattacttcgacaattaaagataacaagcaggcggcaggtccaaccctgactaaggagttagcgctgaacgttttaagcggctcaaaaagtttttttgcacctgaaccacgaatacagccttcttttggtgaaaatgttggaaaggaaggagctttattatttagtgtgaacttaactgttcctgaaaatgtatcccaggtaacggtctaccctgtttatgatgaagattatgggttaggacgactagtaaataccgctgatgcttcccaatcaataatctaccagattgttgatgagaaagggaaaaaaatgttaaaagatcatggtgcagaggttacacctaatcaacaaataacttttaaagcgctgaattatactagcggggaaaaaaaaatatctcctggaatatataacgatcaggttatggttggttactacgtcaacgacaataaacaaggaaactggcaatataaatctctggatgtaaatgtaaatattgagcaaaattttattccagatattgattccgctgttcgtataatacctgttaattacgattcggacccgaaactggattcacagttatatacggttgagatgacgatccctgcaggtgtaagcgcagttaaaatcgcaccaacagatagtctgacatcttctggacagcagatcggaaagctggttaatgtaaacaatccagatcaaaatatgaattattatatcagaaaggattctggcgctggtaactttatggcaggacaaaaaggatcctttcctgtcaaagagaatacgtcatacacattctcagcaatttatactggtggcgaataccctaatagcggatattcgtctggtacttatgcaggaaatttgactgtatcattttacagcaatgacaataaacaaagaacagaaatagcgactaaaaacttcccagtatcaacgactatttcactcgagcaccaccaccaccaccactga

SEQ ID NO: 15 - protein, 614 aa, Escherichia coli
MAVGPTKDMSLGANLTSEPTLAIDFTPIENIYVGANYGKDIGTLVFTTNDLTDITLMSSRSVVDGRQTGFFTFMDSSATYKISTKLGSSNDVNIQEITQGAKITPVSGEKTLPKKFTLKLHAHRSSSTVPGTYTVGLNVTSNVIDNKQAAGPTLTKELALNVLSPAALDATWAPQDNLTLSNTGVSNTLVGVLTLSNTSIDTVSIASTNVSDTSKNGTVTFAHETNNSASFATTISTDNANITLDKNAGNTIVKTTNGSQLPTNLPLKFITTEGNEHLVSGNYRANITITSTIKDNKQAAGPTLTKELALNVLSGSKSFFAPEPRIQPSFGENVGKEGALLFSVNLTVPENVSQVTVYPVYDEDYGLGRLVNTADASQSIIYQIVDEKGKKMLKDHGAEVTPNQQITFKALNYTSGEKKISPGIYNDQVMVGYYVNDNKQGNWQYKSLDVNVNIEQNFIPDIDSAVRIIPVNYDSDPKLDSQLYTVEMTIPAGVSAVKIAPTDSLTSSGQQIGKLVNVNNPDQNMNYYIRKDSGAGNFMAGQKGSFPVKENTSYTFSAIYTGGEYPNSGYSSGTYAGNLTVSFYSNDNKQRTEIATKNFPVSTTISLEHHHHHH

SEQ ID NO: 16 - DNA, 2487 bp, Escherichia coli
  source 1..2487: mol_type = unassigned DNA
atgaataaaattttatttatttttacattgtttttttcttcagggttttttacatttgccgtatcggcagataaaaatcccggaagtgaaaacatgactaatactattggtccccatgacagggggggatcttcccccatatataatatcttaaattcctatcttacagcatacaatggaagccatcatctgtatgataggatgagttttttatgtttgtcttctcaaaatacactgaatggagcatgcccaagcagtgatgcccctggcactgctacaattgatggcgaaacaaatataacattacaatttacggaaaaaagaagtctaattaaaagagaactgcaaattaaaggctataaacaatttttgttcaaaaatgctaattgcccatctaaactagcacttaactcatctcattttcaatgtaatagagaacaagcttcaggtgctactttatcgttatacataccagctggtgaattaaataaattaccttttgggggggtctggaatgccgttctgaagctaaatgtaaaaagacgatatgatacaacctatgggacttacactataaacatcacagttaatttaactgataagggaaatattcagatatggttaccacagttcaaaagtaacgctcgtgtcgatcttaacttgcgtccaactggtggtggtacatatatcggaagaaattctgttgatatgtgcttttatgatggatatagtactaacagcagctctttagagataagatttcaggatgataattctaaatctgatggaaaattttatctaaagaaaataaatgatgactccaaagaacttgtatacactttgtcacttctcctggcaggtaaaaatttaacaccaacaaatggacaggcattaaatattaacactgcttctctggaaacaaactggaatagaattacagctgtcaccatgccagaaatcagtgttccggtgttgtgttggcctggacgtttgcaattggatgcaaaagtgaaaaatcccgaggctggacaatatatggggaatattaaaattactttcacaccaagtagtcaaacactcgacaataaacaagtagagaaaaatattactgtaacagctagtgttgatcctgcaattgatcttttgcaagctgatggcaatgctctgccatcagctgtaaagttagcttattctcccgcatcaaaaacttttgaaagttacagagtaatgactcaagttcatacaaacgatgcaactaaaaaagtaattgttaaacttgctgatacaccacagcttacagatgttctgaattcaactgttcaaatgcctatcagtgtgtcatggggaggacaagtattatctacaacagccaaagaatttgaagctgctgctttgggatattctgcatccggtgtaaatggcgtatcatcttctcaagagttagtaattagcgctgcacctaaaactgccggtaccgccccaactgcaggaaactattcaggagtagtatctcttgtaatgactttgggatccgacaataaacaagtagagaaaaatattactgtaacagctagtgtcgaccctgcagggaattttattccagatattgattccgctgttcgtataatacctgttaattacgattcggacccgaaactggattcacagttatatacggttgagatgacgatccctgcaggtgtaagcgcagttaaaatcgcaccaacagatagtctgacatcttctggacagcagatcggaaagctggttaatgtaaacaatccagatcaaaatatgaattattatatcagaaaggattctggcgctggtaactttatggcaggacaaaaaggatcctttcctgtcaaagagaatacgtcatacacattctcagcaatttatactggtggcgaataccctaatagcggatattcgtctggtacttatgcaggaaatttgactgtatcattttacagcaatgacaataaacaaagaacagaaatagcgactaaaaacttcccagtatcaacgactatttcaaaaagtttttttgcacctgaaccacgaatacagccttcttttggtgaaaatgttggaaaggaaggagctttattatttagtgtgaacttaactgttcctgaaaatgtatcccaggtaacggtctaccctgtttatgatgaagattatgggttaggacgactagtaaataccgctgatgcttcccaatcaataatctaccagattgttgatgagaaagggaaaaaaatgttaaaagatcatggtgcagaggttacacctaatcaacaaataacttttaaagcgctgaattatactagcggggaaaaaaaaatatctcctggaatatataacgatcaggttatggttggttactacgtaaacgacaataaacaacgtaccgagattgccaccaagaattttccggtgagcaccaccatcagcctcgagcaccaccaccaccaccactga

SEQ ID NO: 17 - protein, 828 aa, Escherichia coli
MNKILFIFTLFFSSGFFTFAVSADKNPGSENMTNTIGPHDRGGSSPIYNILNSYLTAYNGSHHLYDRMSFLCLSSQNTLNGACPSSDAPGTATIDGETNITLQFTEKRSLIKRELQIKGYKQFLFKNANCPSKLALNSSHFQCNREQASGATLSLYIPAGELNKLPFGGVWNAVLKLNVKRRYDTTYGTYTINITVNLTDKGNIQIWLPQFKSNARVDLNLRPTGGGTYIGRNSVDMCFYDGYSTNSSSLEIRFQDDNSKSDGKFYLKKINDDSKELVYTLSLLLAGKNLTPTNGQALNINTASLETNWNRITAVTMPEISVPVLCWPGRLQLDAKVKNPEAGQYMGNIKITFTPSSQTLDNKQVEKNITVTASVDPAIDLLQADGNALPSAVKLAYSPASKTFESYRVMTQVHTNDATKKVIVKLADTPQLTDVLNSTVQMPISVSWGGQVLSTTAKEFEAAALGYSASGVNGVSSSQELVISAAPKTAGTAPTAGNYSGVVSLVMTLGSDNKQVEKNITVTASVDPAGNFIPDIDSAVRIIPVNYDSDPKLDSQLYTVEMTIPAGVSAVKIAPTDSLTSSGQQIGKLVNVNNPDQNMNYYIRKDSGAGNFMAGQKGSFPVKENTSYTFSAIYTGGEYPNSGYSSGTYAGNLTVSFYSNDNKQRTEIATKNFPVSTTISKSFFAPEPRIQPSFGENVGKEGALLFSVNLTVPENVSQVTVYPVYDEDYGLGRLVNTADASQSIIYQIVDEKGKKMLKDHGAEVTPNQQITFKALNYTSGEKKISPGIYNDQVMVGYYVNDNKQRTEIATKNFPVSTTISLEHHHHHH

SEQ ID NO: 18 - DNA, 2490 bp, Escherichia coli
  source 1..2490: mol_type = unassigned DNA
atgaataaaattttatttatttttacattgtttttttcttcagggttttttacatttgccgtatcggcagataaaaatcccggaagtgaaaacatgactaatactattggtccccatgacagggggggatcttcccccatatataatatcttaaattcctatcttacagcatacaatggaagccatcatctgtatgataggatgagttttttatgtttgtcttctcaaaatacactgaatggagcatgcccaagcagtgatgcccctggcactgctacaattgatggcgaaacaaatataacattacaatttacggaaaaaagaagtctaattaaaagagaactgcaaattaaaggctataaacaatttttgttcaaaaatgctaattgcccatctaaactagcacttaactcatctcattttcaatgtaatagagaacaagcttcaggtgctactttatcgttatacataccagctggtgaattaaataaattaccttttgggggggtctggaatgccgttctgaagctaaatgtaaaaagacgatatgatacaacctatgggacttacactataaacatcacagttaatttaactgataagggaaatattcagatatggttaccacagttcaaaagtaacgctcgtgtcgatcttaacttgcgtccaactggtggtggtacatatatcggaagaaattctgttgatatgtgcttttatgatggatatagtactaacagcagctctttagagataagatttcaggatgataattctaaatctgatggaaaattttatctaaagaaaataaatgatgactccaaagaacttgtatacactttgtcacttctcctggcaggtaaaaatttaacaccaacaaatggacaggcattaaatattaacactgcttctctggaaacaaactggaatagaattacagctgtcaccatgccagaaatcagtgttccggtgttgtgttggcctggacgtttgcaattggatgcaaaagtgaaaaatcccgaggctggacaatatatggggaatattaaaattactttcacaccaagtagtcaaacactcgacaataaacaagtagagaaaaatattactgtaacagctagtgttgatcctgcaattgatcttttgcaagctgatggcaatgctctgccatcagctgtaaagttagcttattctcccgcatcaaaaacttttgaaagttacagagtaatgactcaagttcatacaaacgatgcaactaaaaaagtaattgttaaacttgctgatacaccacagcttacagatgttctgaattcaactgttcaaatgcctatcagtgtgtcatggggaggacaagtattatctacaacagccaaagaatttgaagctgctgctttgggatattctgcatccggtgtaaatggcgtatcatcttctcaagagttagtaattagcgctgcacctaaaactgccggtaccgccccaactgcaggaaactattcaggagtagtatctcttgtaatgactttgggatccgacaataaacaagtagagaaaaatattactgtaacagctagtgtcgaccctgcagggtcaaaaagtttttttgcacctgaaccacgaatacagccttcttttggtgaaaatgttggaaaggaaggagctttattatttagtgtgaacttaactgttcctgaaaatgtatcccaggtaacggtctaccctgtttatgatgaagattatgggttaggacgactagtaaataccgctgatgcttcccaatcaataatctaccagattgttgatgagaaagggaaaaaaatgttaaaagatcatggtgcagaggttacacctaatcaacaaataacttttaaagcgctgaattatactagcggggaaaaaaaaatatctcctggaatatataacgatcaggttatggttggttactacgtcaacgacaataaacaaggaaactggcaatataaatctctggatgtaaatgtaaatattgagcaaaattttattccagatattgattccgctgttcgtataatacctgttaattacgattcggacccgaaactggattcacagttatatacggttgagatgacgatccctgcaggtgtaagcgcagttaaaatcgcaccaacagatagtctgacatcttctggacagcagatcggaaagctggttaatgtaaacaatccagatcaaaatatgaattattatatcagaaaggattctggcgctggtaactttatggcaggacaaaaaggatcctttcctgtcaaagagaatacgtcatacacattctcagcaatttatactggtggcgaataccctaatagcggatattcgtctggtacttatgcaggaaatttgactgtatcattttacagcaatgacaataaacaaggcaattggcagtacaagagcctcgacgtgaacgtgaacatcgaacagctcgagcaccaccaccaccaccactga

SEQ ID NO: 19 - protein, 829 aa, Escherichia coli
MNKILFIFTLFFSSGFFTFAVSADKNPGSENMTNTIGPHDRGGSSPIYNILNSYLTAYNGSHHLYDRMSFLCLSSQNTLNGACPSSDAPGTATIDGETNITLQFTEKRSLIKRELQIKGYKQFLFKNANCPSKLALNSSHFQCNREQASGATLSLYIPAGELNKLPFGGVWNAVLKLNVKRRYDTTYGTYTINITVNLTDKGNIQIWLPQFKSNARVDLNLRPTGGGTYIGRNSVDMCFYDGYSTNSSSLEIRFQDDNSKSDGKFYLKKINDDSKELVYTLSLLLAGKNLTPTNGQALNINTASLETNWNRITAVTMPEISVPVLCWPGRLQLDAKVKNPEAGQYMGNIKITFTPSSQTLDNKQVEKNITVTASVDPAIDLLQADGNALPSAVKLAYSPASKTFESYRVMTQVHTNDATKKVIVKLADTPQLTDVLNSTVQMPISVSWGGQVLSTTAKEFEAAALGYSASGVNGVSSSQELVISAAPKTAGTAPTAGNYSGVVSLVMTLGSDNKQVEKNITVTASVDPAGSKSFFAPEPRIQPSFGENVGKEGALLFSVNLTVPENVSQVTVYPVYDEDYGLGRLVNTADASQSIIYQIVDEKGKKMLKDHGAEVTPNQQITFKALNYTSGEKKISPGIYNDQVMVGYYVNDNKQGNWQYKSLDVNVNIEQNFIPDIDSAVRIIPVNYDSDPKLDSQLYTVEMTIPAGVSAVKIAPTDSLTSSGQQIGKLVNVNNPDQNMNYYIRKDSGAGNFMAGQKGSFPVKENTSYTFSAIYTGGEYPNSGYSSGTYAGNLTVSFYSNDNKQGNWQYKSLDVNVNIEQLEHHHHHH

SEQ ID NO: 20 - DNA, 3405 bp, Escherichia coli
  source 1..3405: mol_type = unassigned DNA
atgaataaaattttatttatttttacattgtttttttcttcagggttttttacatttgccgtatcggcagataaaaatcccggaagtgaaaacatgactaatactattggtccccatgacagggggggatcttcccccatatataatatcttaaattcctatcttacagcatacaatggaagccatcatctgtatgataggatgagttttttatgtttgtcttctcaaaatacactgaatggagcatgcccaagcagtgatgcccctggcactgctacaattgatggcgaaacaaatataacattacaatttacggaaaaaagaagtctaattaaaagagaactgcaaattaaaggctataaacaatttttgttcaaaaatgctaattgcccatctaaactagcacttaactcatctcattttcaatgtaatagagaacaagcttcaggtgctactttatcgttatacataccagctggtgaattaaataaattaccttttgggggggtctggaatgccgttctgaagctaaatgtaaaaagacgatatgatacaacctatgggacttacactataaacatcacagttaatttaactgataagggaaatattcagatatggttaccacagttcaaaagtaacgctcgtgtcgatcttaacttgcgtccaactggtggtggtacatatatcggaagaaattctgttgatatgtgcttttatgatggatatagtactaacagcagctctttagagataagatttcaggatgataattctaaatctgatggaaaattttatctaaagaaaataaatgatgactccaaagaacttgtatacactttgtcacttctcctggcaggtaaaaatttaacaccaacaaatggacaggcattaaatattaacactgcttctctggaaacaaactggaatagaattacagctgtcaccatgccagaaatcagtgttccggtgttgtgttggcctggacgtttgcaattggatgcaaaagtgaaaaatcccgaggctggacaatatatggggaatattaaaattactttcacaccaagtagtcaaacactcgacaataaacaagtagagaaaaatattactgtaacagctagtgttgatcctgcaattgatcttttgcaagctgatggcaatgctctgccatcagctgtaaagttagcttattctcccgcatcaaaaacttttgaaagttacagagtaatgactcaagttcatacaaacgatgcaactaaaaaagtaattgttaaacttgctgatacaccacagcttacagatgttctgaattcaactgttcaaatgcctatcagtgtgtcatggggaggacaagtattatctacaacagccaaagaatttgaagctgctgctttgggatattctgcatccggtgtaaatggcgtatcatcttctcaagagttagtaattagcgctgcacctaaaactgccggtaccgccccaactgcaggaaactattcaggagtagtatctcttgtaatgactttgggatccgacaataaacaagtagagaaaaatattactgtaacagctagtgtcgaccctactattgatattcttcaagcaaatggttctgcgctaccgacagctgtagatttaacttatctacctggtgcaaaaacttttgaaaattacagtgttctaacccagatttacacaaatgacccttcaaaaggtttagatgttcgactggttgatacaccgaaacttacaaatattttgcaaccgacatctaccattcctcttactgtctcatgggcagggaagacattaagtacaagtgctcagaagattgcagttggcgatctgggttttggttccaccggaacggcaggtgtttcgaatagtaaagaattagtaattggagcaactacatccggaactgcaccaagtgcaggtaagtatcaaggcgtcgtttccattgtaatgactcaatcgaccgacacagccgcgcctgttcctgacaataaacaagtagagaaaaatattactgtgacagccagtgttgatcctactattgacattttgcaagctgatggtagtagtttacctactgctgtagaattaacctattcacctgcggcaagtcgttttgaaaattataaaatcgcaactaaagttcatacaaatgttataaataaaaatgtactagttaagcttgtaaatgatccaaaacttacaaatgttttggattctacaaaacaactccccattactgtatcatatggaggaaagactctatcaaccgcagatgtgacttttgaacctgcagaattaaattttggaacgtcaggtgtaactggtgtatcttcttcccaagatttagtgattggtgcgactacagcacaagcaccaacggcgggaaattatagtggggtcgtttctatcttaatgaccttagcatcagacaataaacaagtggaaaaaaatatcactgtaacagctagtgttgatcctacgggcgagcaaaattttattccagatattgattccgctgttcgtataatacctgttaattacgattcggatccgaaactgaattcacagttatatacggttgagatgacgatccctgcaggtgtaagcgcagttaaaatcgtaccaacagatagtctgacatcttctggacagcagatcggaaagctggttaatgtaaacaatccagatcaaaatatgaattattatatcagaaaggattctggcgctggtaagtttatggcagggcaaaaaggatccttttctgtcaaagagaatacgtcatacacattctcagcaatttatactggtggcgaataccctaatagcggatattcgtctggtacttatgcaggacatttgactgtatcattttacagcaatgacaataaacaaagaacagaaatagcgactaaaaacttcccagtatcaacgactatttcaaaaagtttttttgcgcctgaaccacaaatccagccttcttttggtaaaaatgttggaaaggaaggagatttattatttagtgtgagcttaattgttcctgaaaatgtatcccaggtaacggtctaccctgtttatgatgaagattatggattaggacgactcgtaaataccgctgatgattcccaatcaataatctaccagattgttgatgataaagggaaaaaaatgttaaaagatcatggtacagaggttacgcctaatcaacaaataacttttaaagcgctgaattatactagcggagataaagaaatacctcctgggatatataacgatcaggttatggttggttactacgtaaacgacaataaacaaggaaactggcaatataaatctctggatgtaaatgtaaatattgagcaactcgagcaccaccaccaccaccactga

SEQ ID NO: 21 - protein, 1134 aa, Escherichia coli
MNKILFIFTLFFSSGFFTFAVSADKNPGSENMTNTIGPHDRGGSSPIYNILNSYLTAYNGSHHLYDRMSFLCLSSQNTLNGACPSSDAPGTATIDGETNITLQFTEKRSLIKRELQIKGYKQFLFKNANCPSKLALNSSHFQCNREQASGATLSLYIPAGELNKLPFGGVWNAVLKLNVKRRYDTTYGTYTINITVNLTDKGNIQIWLPQFKSNARVDLNLRPTGGGTYIGRNSVDMCFYDGYSTNSSSLEIRFQDDNSKSDGKFYLKKINDDSKELVYTLSLLLAGKNLTPTNGQALNINTASLETNWNRITAVTMPEISVPVLCWPGRLQLDAKVKNPEAGQYMGNIKITFTPSSQTLDNKQVEKNITVTASVDPAIDLLQADGNALPSAVKLAYSPASKTFESYRVMTQVHTNDATKKVIVKLADTPQLTDVLNSTVQMPISVSWGGQVLSTTAKEFEAAALGYSASGVNGVSSSQELVISAAPKTAGTAPTAGNYSGVVSLVMTLGSDNKQVEKNITVTASVDPTIDILQANGSALPTAVDLTYLPGAKTFENYSVLTQIYTNDPSKGLDVRLVDTPKLTNILQPTSTIPLTVSWAGKTLSTSAQKIAVGDLGFGSTGTAGVSNSKELVIGATTSGTAPSAGKYQGVVSIVMTQSTDTAAPVPDNKQVEKNITVTASVDPTIDILQADGSSLPTAVELTYSPAASRFENYKIATKVHTNVINKNVLVKLVNDPKLTNVLDSTKQLPITVSYGGKTLSTADVTFEPAELNFGTSGVTGVSSSQDLVIGATTAQAPTAGNYSGVVSILMTLASDNKQVEKNITVTASVDPTGEQNFIPDIDSAVRIIPVNYDSDPKLNSQLYTVEMTIPAGVSAVKIVPTDSLTSSGQQIGKLVNVNNPDQNMNYYIRKDSGAGKFMAGQKGSFSVKENTSYTFSAIYTGGEYPNSGYSSGTYAGHLTVSFYSNDNKQRTEIATKNFPVSTTISKSFFAPEPQIQPSFGKNVGKEGDLLFSVSLIVPENVSQVTVYPVYDEDYGLGRLVNTADDSQSIIYQIVDDKGKKMLKDHGTEVTPNQQITFKALNYTSGDKEIPPGIYNDQVMVGYYVNDNKQGNWQYKSLDVNVNIEQLEHHHHHH

SEQ ID NO: 22 - DNA, 3342 bp, Escherichia coli
  source 1..3342: mol_type = unassigned DNA
atggcagataaaaatcccggaagtgaaaacatgactaatactattggtccccatgacagggggggatcttcccccatatataatatcttaaattcctatcttacagcatacaatggaagccatcatctgtatgataggatgagttttttatgtttgtcttctcaaaatacactgaatggagcatgcccaagcagtgatgcccctggcactgctacaattgatggcgaaacaaatataacattacaatttacggaaaaaagaagtctaattaaaagagaactgcaaattaaaggctataaacaatttttgttcaaaaatgctaattgcccatctaaactagcacttaactcatctcattttcaatgtaatagagaacaagcttcaggtgctactttatcgttatacataccagctggtgaattaaataaattaccttttgggggggtctggaatgccgttctgaagctaaatgtaaaaagacgatatgatacaacctatgggacttacactataaacatcacagttaatttaactgataagggaaatattcagatatggttaccacagttcaaaagtaacgctcgtgtcgatcttaacttgcgtccaactggtggtggtacatatatcggaagaaattctgttgatatgtgcttttatgatggatatagtactaacagcagctctttagagataagatttcaggatgataattctaaatctgatggaaaattttatctaaagaaaataaatgatgactccaaagaacttgtatacactttgtcacttctcctggcaggtaaaaatttaacaccaacaaatggacaggcattaaatattaacactgcttctctggaaacaaactggaatagaattacagctgtcaccatgccagaaatcagtgttccggtgttgtgttggcctggacgtttgcaattggatgcaaaagtgaaaaatcccgaggctggacaatatatggggaatattaaaattactttcacaccaagtagtcaaacactcgacaataaacaagtagagaaaaatattactgtaacagctagtgttgatcctgcaattgatcttttgcaagctgatggcaatgctctgccatcagctgtaaagttagcttattctcccgcatcaaaaacttttgaaagttacagagtaatgactcaagttcatacaaacgatgcaactaaaaaagtaattgttaaacttgctgatacaccacagcttacagatgttctgaattcaactgttcaaatgcctatcagtgtgtcatggggaggacaagtattatctacaacagccaaagaatttgaagctgctgctttgggatattctgcatccggtgtaaatggcgtatcatcttctcaagagttagtaattagcgctgcacctaaaactgccggtaccgccccaactgcaggaaactattcaggagtagtatctcttgtaatgactttgggatccgacaataaacaagtagagaaaaatattactgtaacagctagtgtcgaccctactattgatattcttcaagcaaatggttctgcgctaccgacagctgtagatttaacttatctacctggtgcaaaaacttttgaaaattacagtgttctaacccagatttacacaaatgacccttcaaaaggtttagatgttcgactggttgatacaccgaaacttacaaatattttgcaaccgacatctaccattcctcttactgtctcatgggcagggaagacattaagtacaagtgctcagaagattgcagttggcgatctgggttttggttccaccggaacggcaggtgtttcgaatagtaaagaattagtaattggagcaactacatccggaactgcaccaagtgcaggtaagtatcaaggcgtcgtttccattgtaatgactcaatcgaccgacacagccgcgcctgttcctgacaataaacaagtagagaaaaatattactgtgacagccagtgttgatcctactattgacattttgcaagctgatggtagtagtttacctactgctgtagaattaacctattcacctgcggcaagtcgttttgaaaattataaaatcgcaactaaagttcatacaaatgttataaataaaaatgtactagttaagcttgtaaatgatccaaaacttacaaatgttttggattctacaaaacaactccccattactgtatcatatggaggaaagactctatcaaccgcagatgtgacttttgaacctgcagaattaaattttggaacgtcaggtgtaactggtgtatcttcttcccaagatttagtgattggtgcgactacagcacaagcaccaacggcgggaaattatagtggggtcgtttctatcttaatgaccttagcatcagacaataaacaagtggaaaaaaatatcactgtaacagctagtgttgatcctacgggcgagcaaaattttattccagatattgattccgctgttcgtataatacctgttaattacgattcggatccgaaactgaattcacagttatatacggttgagatgacgatccctgcaggtgtaagcgcagttaaaatcgtaccaacagatagtctgacatcttctggacagcagatcggaaagctggttaatgtaaacaatccagatcaaaatatgaattattatatcagaaaggattctggcgctggtaagtttatggcagggcaaaaaggatccttttctgtcaaagagaatacgtcatacacattctcagcaatttatactggtggcgaataccctaatagcggatattcgtctggtacttatgcaggacatttgactgtatcattttacagcaatgacaataaacaaagaacagaaatagcgactaaaaacttcccagtatcaacgactatttcaaaaagtttttttgcgcctgaaccacaaatccagccttcttttggtaaaaatgttggaaaggaaggagatttattatttagtgtgagcttaattgttcctgaaaatgtatcccaggtaacggtctaccctgtttatgatgaagattatggattaggacgactcgtaaataccgctgatgattcccaatcaataatctaccagattgttgatgataaagggaaaaaaatgttaaaagatcatggtacagaggttacgcctaatcaacaaataacttttaaagcgctgaattatactagcggagataaagaaatacctcctgggatatataacgatcaggttatggttggttactacgtaaacgacaataaacaaggaaactggcaatataaatctctggatgtaaatgtaaatattgagcaactcgagcaccaccaccaccaccactga

SEQ ID NO: 23 - protein, 1113 aa, Escherichia coli
MADKNPGSENMTNTIGPHDRGGSSPIYNILNSYLTAYNGSHHLYDRMSFLCLSSQNTLNGACPSSDAPGTATIDGETNITLQFTEKRSLIKRELQIKGYKQFLFKNANCPSKLALNSSHFQCNREQASGATLSLYIPAGELNKLPFGGVWNAVLKLNVKRRYDTTYGTYTINITVNLTDKGNIQIWLPQFKSNARVDLNLRPTGGGTYIGRNSVDMCFYDGYSTNSSSLEIRFQDDNSKSDGKFYLKKINDDSKELVYTLSLLLAGKNLTPTNGQALNINTASLETNWNRITAVTMPEISVPVLCWPGRLQLDAKVKNPEAGQYMGNIKITFTPSSQTLDNKQVEKNITVTASVDPAIDLLQADGNALPSAVKLAYSPASKTFESYRVMTQVHTNDATKKVIVKLADTPQLTDVLNSTVQMPISVSWGGQVLSTTAKEFEAAALGYSASGVNGVSSSQELVISAAPKTAGTAPTAGNYSGVVSLVMTLGSDNKQVEKNITVTASVDPTIDILQANGSALPTAVDLTYLPGAKTFENYSVLTQIYTNDPSKGLDVRLVDTPKLTNILQPTSTIPLTVSWAGKTLSTSAQKIAVGDLGFGSTGTAGVSNSKELVIGATTSGTAPSAGKYQGVVSIVMTQSTDTAAPVPDNKQVEKNITVTASVDPTIDILQADGSSLPTAVELTYSPAASRFENYKIATKVHTNVINKNVLVKLVNDPKLTNVLDSTKQLPITVSYGGKTLSTADVTFEPAELNFGTSGVTGVSSSQDLVIGATTAQAPTAGNYSGVVSILMTLASDNKQVEKNITVTASVDPTGEQNFIPDIDSAVRIIPVNYDSDPKLNSQLYTVEMTIPAGVSAVKIVPTDSLTSSGQQIGKLVNVNNPDQNMNYYIRKDSGAGKFMAGQKGSFSVKENTSYTFSAIYTGGEYPNSGYSSGTYAGHLTVSFYSNDNKQRTEIATKNFPVSTTISKSFFAPEPQIQPSFGKNVGKEGDLLFSVSLIVPENVSQVTVYPVYDEDYGLGRLVNTADDSQSIIYQIVDDKGKKMLKDHGTEVTPNQQITFKALNYTSGDKEIPPGIYNDQVMVGYYVNDNKQGNWQYKSLDVNVNIEQLEHHHHHH

SEQ ID NO: 24 - DNA, 2943 bp, Escherichia coli
  source 1..2943: mol_type = unassigned DNA
atgaaaaagatatttatttttttgtctatcatattttctgcggtggtcagtgccgggcgatacccggaaactacagtaggtaatctgacgaagagttttcaagcccctcgtcaggatagaagcgtacaatcaccaatatataacatctttacgaatcatgtggctggatatagtttgagtcataacttatatgacaggattgtttttttatgtacatcctcgtcgaatccggttaatggtgcttgcccaaccattggaacatctggagttcaatacggtactacaaccataaccttgcagtttacagaaaaaagaagtctgataaaaagaaatattaatcttgcaggtaataagaaaccaatatgggagaatcagagttgcgacactagcaatctaatggtgttgaattcgaagtcttggtcctgtggggcttacggaaatgctaacggaacacttctaaatctgtatatccctgcaggagaaatcaacaaattgccttttggagggatatgggaggcaactctgatcttacgcttatcaagatatggcgaagtcagtagcacccattacggcaattataccgtaaatattacggttgatttaactgataaaggtaatattcaggtatggcttccagggtttcacagcaacccgcgtgtagacctgaatctgcaccctatcggtaattataaatatagtggtagtaattcactcgacatgtgtttctatgatggatatagtacaaacagtgatagcatggtaataaagttccaggatgataatcctacctattcatctgaatataatctttataagatagggggcactgaaaaattaccctatgctgtttcactgcttatgggagaaaaaatattttatccagtgaatggtcaatcatttactatcaatgacagtagtgtactcgaaacaaactggaatcgagtaaccgcagttgctatgccggaagttaatgttccagtattatgctggccagcaagattgctattaaatgctgatgtaaatgctcccgatgcaggacagtattcaggacagatatatataacatttacacccagtgtcgaaaatttaggcggtggagtcgaaaaaaatattactgtgagggcaagtgttgaccctaaacttgatcttctgcaagcagatggaacttcactgccggactctatcgcattaacctattcttcggcttcaaataattttgaagtttactctcttaatactgctattcatacaaatgacaaaagcaagggagttgtagtgaagctgtcagcttcaccagttctgtccaatattatgaagccaaactcgcaaattccgatgaaagtgactttgggggggaagacgctgaatacaactgatactgagtttactgttgatactctgaactttggtacatctggtgttgaaaacgtttcttccactcaacagcttacgattcatgcagacacacaaggaactgcgcctgaggcaggcaattaccaaggtattatttctcttatcatgactcaaaaaacagggggcggtgtcgaaaaaaatattactgtgagggcaagtgtcgaccctaaacttgaccttctgcaatctgatggctctgcgctgccgaactctgtcgcattaacctattctccggctgtaaataattttgaagctcacaccatcaacaccgttgttcatacaaatgactcagataaaggtgttgttgtgaagctgtcagcagatccagtcctgtccaatgttctgaatccaaccctgcaaattcctgtttctgtgaatttcgcaggaaaaccactgagcacaacaggcattaccatcgactccaatgatctgaactttgcttcgagtggtgttaataaagtttcttctacgcagaaactttcaatccatgcagatgctactcgggtaactggcggcgcactaacagctggtcaatatcagggactcgtatcaattatcctgactaagtcaacggggggcggtgtcgagaagaccattagcgttacggcgagtgttgacccgacgggcgagcaaaattttattccagatattgattccgctgttcgtataatacctgttaattacgattcggatccgaaactgaattcacagttatatacggttgagatgacgatccctgcaggtgtaagcgcagttaaaatcgtaccaacagatagtctgacatcttctggacagcagatcggaaagctggttaatgtaaacaatccagatcaaaatatgaattattatatcagaaaggattctggcgctggtaagtttatggcagggcaaaaaggatccttttctgtcaaagagaatacgtcatacacattctcagcaatttatactggtggcgaataccctaatagcggatattcgtctggtacttatgcaggacatttgactgtatcattttacagcaatgacaataaacaaagaacagaaatagcgactaaaaacttcccagtatcaacgactatttcaaaaagtttttttgcgcctgaaccacaaatccagccttcttttggtaaaaatgttggaaaggaaggagatttattatttagtgtgagcttaattgttcctgaaaatgtatcccaggtaacggtctaccctgtttatgatgaagattatggattaggacgactcgtaaataccgctgatgattcccaatcaataatctaccagattgttgatgataaagggaaaaaaatgttaaaagatcatggtacagaggttacgcctaatcaacaaataacttttaaagcgctgaattatactagcggagataaagaaatacctcctgggatatataacgatcaggttatggttggttactacgtaaacgacaataaacaaggaaactggcaatataaatctctggatgtaaatgtaaatattgagcaactcgagcaccaccaccaccaccactga

SEQ ID NO: 25 - protein, 980 aa, Escherichia coli
MKKIFIFLSIIFSAVVSAGRYPETTVGNLTKSFQAPRQDRSVQSPIYNIFTNHVAGYSLSHNLYDRIVFLCTSSSNPVNGACPTIGTSGVQYGTTTITLQFTEKRSLIKRNINLAGNKKPIWENQSCDTSNLMVLNSKSWSCGAYGNANGTLLNLYIPAGEINKLPFGGIWEATLILRLSRYGEVSSTHYGNYTVNITVDLTDKGNIQVWLPGFHSNPRVDLNLHPIGNYKYSGSNSLDMCFYDGYSTNSDSMVIKFQDDNPTYSSEYNLYKIGGTEKLPYAVSLLMGEKIFYPVNGQSFTINDSSVLETNWNRVTAVAMPEVNVPVLCWPARLLLNADVNAPDAGQYSGQIYITFTPSVENLGGGVEKNITVRASVDPKLDLLQADGTSLPDSIALTYSSASNNFEVYSLNTAIHTNDKSKGVVVKLSASPVLSNIMKPNSQIPMKVTLGGKTLNTTDTEFTVDTLNFGTSGVENVSSTQQLTIHADTQGTAPEAGNYQGIISLIMTQKTGGGVEKNITVRASVDPKLDLLQSDGSALPNSVALTYSPAVNNFEAHTINTVVHTNDSDKGVVVKLSADPVLSNVLNPTLQIPVSVNFAGKPLSTTGITIDSNDLNFASSGVNKVSSTQKLSIHADATRVTGGALTAGQYQGLVSIILTKSTGGGVEKTISVTASVDPTGEQNFIPDIDSAVRIIPVNYDSDPKLNSQLYTVEMTIPAGVSAVKIVPTDSLTSSGQQIGKLVNVNNPDQNMNYYIRKDSGAGKFMAGQKGSFSVKENTSYTFSAIYTGGEYPNSGYSSGTYAGHLTVSFYSNDNKQRTEIATKNFPVSTTISKSFFAPEPQIQPSFGKNVGKEGDLLFSVSLIVPENVSQVTVYPVYDEDYGLGRLVNTADDSQSIIYQIVDDKGKKMLKDHGTEVTPNQQITFKALNYTSGDKEIPPGIYNDQVMVGYYVNDNKQGNWQYKSLDVNVNIEQLEHHHHHH

SEQ ID NO: 26 - DNA, 2795 bp, Escherichia coli
  source 1..2795: mol_type = unassigned DNA
ttacgaatcatgtggctggatatagtttgagtcataacttatatgacaggattgtttttttatgtacatcctcgtcgaatccggttaatggtgcttgcccaaccattggaacatctggagttcaatacggtactacaaccataaccttgcagtttacagaaaaaagaagtctgataaaaagaaatattaatcttgcaggtaataagaaaccaatatgggagaatcagagttgcgacactagcaatctaatggtgttgaattcgaagtcttggtcctgtggggcttacggaaatgctaacggaacacttctaaatctgtatatccctgcaggagaaatcaacaaattgccttttggagggatatgggaggcaactctgatcttacgcttatcaagatatggcgaagtcagtagcacccattacggcaattataccgtaaatattacggttgatttaactgataaaggtaatattcaggtatggcttccagggtttcacagcaacccgcgtgtagacctgaatctgcaccctatcggtaattataaatatagtggtagtaattcactcgacatgtgtttctatgatggatatagtacaaacagtgatagcatggtaataaagttccaggatgataatcctacctattcatctgaatataatctttataagatagggggcactgaaaaattaccctatgctgtttcactgcttatgggagaaaaaatattttatccagtgaatggtcaatcatttactatcaatgacagtagtgtactcgaaacaaactggaatcgagtaaccgcagttgctatgccggaagttaatgttccagtattatgctggccagcaagattgctattaaatgctgatgtaaatgctcccgatgcaggacagtattcaggacagatatatataacatttacacccagtgtcgaaaatttaggcggtggagtcgaaaaaaatattactgtgagggcaagtgttgaccctaaacttgatcttctgcaagcagatggaacttcactgccggactctatcgcattaacctattcttcggcttcaaataattttgaagtttactctcttaatactgctattcatacaaatgacaaaagcaagggagttgtagtgaagctgtcagcttcaccagttctgtccaatattatgaagccaaactcgcaaattccgatgaaagtgactttgggggggaagacgctgaatacaactgatactgagtttactgttgatactctgaactttggtacatctggtgttgaaaacgtttcttccactcaacagcttacgattcatgcagacacacaaggaactgcgcctgaggcaggcaattaccaaggtattatttctcttatcatgactcaaaaaacagggggcggtgtcgaaaaaaatattactgtgagggcaagtgtcgaccctaaacttgaccttctgcaatctgatggctctgcgctgccgaactctgtcgcattaacctattctccggctgtaaataattttgaagctcacaccatcaacaccgttgttcatacaaatgactcagataaaggtgttgttgtgaagctgtcagcagatccagtcctgtccaatgttctgaatccaaccctgcaaattcctgtttctgtgaatttcgcaggaaaaccactgagcacaacaggcattaccatcgactccaatgatctgaactttgcttcgagtggtgttaataaagtttcttctacgcagaaactttcaatccatgcagatgctactcgggtaactggcggcgcactaacagctggtcaatatcagggactcgtatcaattatcctgactaagtcaacggggggcggtgtcgagaagaccattagcgttacggcgagtgttgacccgacgggcgagcaaaattttattccagatattgattccgctgttcgtataatacctgttaattacgattcggatccgaaactgaattcacagttatatacggttgagatgacgatccctgcaggtgtaagcgcagttaaaatcgtaccaacagatagtctgacatcttctggacagcagatcggaaagctggttaatgtaaacaatccagatcaaaatatgaattattatatcagaaaggattctggcgctggtaagtttatggcagggcaaaaaggatccttttctgtcaaagagaatacgtcatacacattctcagcaatttatactggtggcgaataccctaatagcggatattcgtctggtacttatgcaggacatttgactgtatcattttacagcaatgacaataaacaaagaacagaaatagcgactaaaaacttcccagtatcaacgactatttcaaaaagtttttttgcgcctgaaccacaaatccagccttcttttggtaaaaatgttggaaaggaaggagatttattatttagtgtgagcttaattgttcctgaaaatgtatcccaggtaacggtctaccctgtttatgatgaagattatggattaggacgactcgtaaataccgctgatgattcccaatcaataatctaccagattgttgatgataaagggaaaaaaatgttaaaagatcatggtacagaggttacgcctaatcaacaaataacttttaaagcgctgaattatactagcggagataaagaaatacctcctgggatatataacgatcaggttatggttggttactacgtaaacgacaataaacaaggaaactggcaatataaatctctggatgtaaatgtaaatattgagcaactcgagcaccaccaccaccaccactga

SEQ ID NO: 27 - protein, 963 aa, Escherichia coli
MGRYPETTVGNLTKSFQAPRQDRSVQSPIYNIFTNHVAGYSLSHNLYDRIVFLCTSSSNPVNGACPTIGTSGVQYGTTTITLQFTEKRSLIKRNINLAGNKKPIWENQSCDTSNLMVLNSKSWSCGAYGNANGTLLNLYIPAGEINKLPFGGIWEATLILRLSRYGEVSSTHYGNYTVNITVDLTDKGNIQVWLPGFHSNPRVDLNLHPIGNYKYSGSNSLDMCFYDGYSTNSDSMVIKFQDDNPTYSSEYNLYKIGGTEKLPYAVSLLMGEKIFYPVNGQSFTINDSSVLETNWNRVTAVAMPEVNVPVLCWPARLLLNADVNAPDAGQYSGQIYITFTPSVENLGGGVEKNITVRASVDPKLDLLQADGTSLPDSIALTYSSASNNFEVYSLNTAIHTNDKSKGVVVKLSASPVLSNIMKPNSQIPMKVTLGGKTLNTTDTEFTVDTLNFGTSGVENVSSTQQLTIHADTQGTAPEAGNYQGIISLIMTQKTGGGVEKNITVRASVDPKLDLLQSDGSALPNSVALTYSPAVNNFEAHTINTVVHTNDSDKGVVVKLSADPVLSNVLNPTLQIPVSVNFAGKPLSTTGITIDSNDLNFASSGVNKVSSTQKLSIHADATRVTGGALTAGQYQGLVSIILTKSTGGGVEKTISVTASVDPTGEQNFIPDIDSAVRIIPVNYDSDPKLNSQLYTVEMTIPAGVSAVKIVPTDSLTSSGQQIGKLVNVNNPDQNMNYYIRKDSGAGKFMAGQKGSFSVKENTSYTFSAIYTGGEYPNSGYSSGTYAGHLTVSFYSNDNKQRTEIATKNFPVSTTISKSFFAPEPQIQPSFGKNVGKEGDLLFSVSLIVPENVSQVTVYPVYDEDYGLGRLVNTADDSQSIIYQIVDDKGKKMLKDHGTEVTPNQQITFKALNYTSGDKEIPPGIYNDQVMVGYYVNDNKQGNWQYKSLDVNVNIEQLEHHHHHH

SEQ ID NO: 28 - DNA, 2505 bp, Escherichia coli
  source 1..2505: mol_type = unassigned DNA
atgaaaaaagtgatttttgttttatccatgtttctatgttctcaggtttacgggcaatcatggcatacgaacgtagaggctggttcaataaataaaacagagtcgataggccccatagaccgaagtgctgctgcatcgtatcctgctcattatatatttcatgaacatgttgctggttacaataaagatcactctctttttgacaggatgacgtttttatgtatgtcatcaacagatgcatctaaaggtgcatgtccgacaggagaaaactccaaatcctctcaaggggagactaatattaagctaatatttactgaaaagaaaagtctggccagaaaaacattaaacttaaaaggatataagagatttttatatgaatcagatagatgcattcattatgtcgataaaatgaatctcaattctcatactgttaaatgtgtaggttcattcacaagaggagtagatttcactttatatatcccacaaggtgaaattgatgggcttctaactggaggtatatgggaggcaacactagagttacgagtcaaaaggcattacgactataatcatggtacttacaaagttaatatcacagttgatttgacagacaaaggaaatattcaggtctggacaccaaagtttcatagcgatcctagaattgatctgaatttacgtcctgaaggtaatggtaaatattctggtagtaacgtgcttgagatgtgtctctatgatggctatagtacacatagtcaaagtatagaaatgaggtttcaggatgactcacaaacaggaaataatgaatataatcttataaaaactggagagccattaaaaaaattgccatataaactttctcttcttttaggaggacgagagttttatccaaataatggagaggcttttactattaatgatacttcgtcattgtttataaactggaatcgtattaagtctgtatccttaccacagattagtattccagtactatgctggccagcaaacttgacatttatgtcagagctaaataatccagaagcgggtgagtattcaggaatacttaacgtaacatttactcctagtagttcaagcctagacaataaacaagccgagaaaaatatcactgtaactgctagcgttgatccaactatcgatctgatgcaatctgatggcacagcgttaccaagtgcagttaatattgcatatcttccaggagagaaaagatttgaatctgctcgtatcaatacccaagttcataccaataataaaactaagggtattcagataaagcttactaatgataatgtggtaatgactaacttatctgatccaagcaagactattcctttagaggtttcattcgctggcactaagctgagcacagctgcaacatctattactgccgatcaattaaattttggcgcagctggtgtagagacagtttctgcaactaaggaactcgttattaatgcaggaagcacccagcaaactaatattgtagctggtaactatcaaggattggtgtcaattgtgcttactcaagaacctgacaataaacaagccgagaaaaatatcactgtaactgctagcgttgatccgacgggcgagcaaaattttattccagatattgattccgctgttcgtataatacctgttaattacgattcggatccgaaactgaattcacagttatatacggttgagatgacgatccctgcaggtgtaagcgcagttaaaatcgtaccaacagatagtctgacatcttctggacagcagatcggaaagctggttaatgtaaacaatccagatcaaaatatgaattattatatcagaaaggattctggcgctggtaagtttatggcagggcaaaaaggatccttttctgtcaaagagaatacgtcatacacattctcagcaatttatactggtggcgaataccctaatagcggatattcgtctggtacttatgcaggacatttgactgtatcattttacagcaatgacaataaacaaagaacagaaatagcgactaaaaacttcccagtatcaacgactatttcaaaaagtttttttgcgcctgaaccacaaatccagccttcttttggtaaaaatgttggaaaggaaggagatttattatttagtgtgagcttaattgttcctgaaaatgtatcccaggtaacggtctaccctgtttatgatgaagattatggattaggacgactcgtaaataccgctgatgattcccaatcaataatctaccagattgttgatgataaagggaaaaaaatgttaaaagatcatggtacagaggttacgcctaatcaacaaataacttttaaagcgctgaattatactagcggagataaagaaatacctcctgggatatataacgatcaggttatggttggttactacgtaaacgacaataaacaaggaaactggcaatataaatctctggatgtaaatgtaaatattgagcaactcgagcaccaccaccaccaccactga

SEQ ID NO: 29 - protein, 834 aa, Escherichia coli
MKKVIFVLSMFLCSQVYGQSWHTNVEAGSINKTESIGPIDRSAAASYPAHYIFHEHVAGYNKDHSLFDRMTFLCMSSTDASKGACPTGENSKSSQGETNIKLIFTEKKSLARKTLNLKGYKRFLYESDRCIHYVDKMNLNSHTVKCVGSFTRGVDFTLYIPQGEIDGLLTGGIWEATLELRVKRHYDYNHGTYKVNITVDLTDKGNIQVWTPKFHSDPRIDLNLRPEGNGKYSGSNVLEMCLYDGYSTHSQSIEMRFQDDSQTGNNEYNLIKTGEPLKKLPYKLSLLLGGREFYPNNGEAFTINDTSSLFINWNRIKSVSLPQISIPVLCWPANLTFMSELNNPEAGEYSGILNVTFTPSSSSLDNKQAEKNITVTASVDPTIDLMQSDGTALPSAVNIAYLPGEKRFESARINTQVHTNNKTKGIQIKLTNDNVVMTNLSDPSKTIPLEVSFAGTKLSTAATSITADQLNFGAAGVETVSATKELVINAGSTQQTNIVAGNYQGLVSIVLTQEPDNKQAEKNITVTASVDPTGEQNFIPDIDSAVRIIPVNYDSDPKLNSQLYTVEMTIPAGVSAVKIVPTDSLTSSGQQIGKLVNVNNPDQNMNYYIRKDSGAGKFMAGQKGSFSVKENTSYTFSAIYTGGEYPNSGYSSGTYAGHLTVSFYSNDNKQRTEIATKNFPVSTTISKSFFAPEPQIQPSFGKNVGKEGDLLFSVSLIVPENVSQVTVYPVYDEDYGLGRLVNTADDSQSIIYQIVDDKGKKMLKDHGTEVTPNQQITFKALNYTSGDKEIPPGIYNDQVMVGYYVNDNKQGNWQYKSLDVNVNIEQLEHHHHHH

SEQ ID NO: 30 - DNA, 2454 bp, Escherichia coli
  source 1..2454: mol_type = unassigned DNA
atgcaatcatggcatacgaacgtagaggctggttcaataaataaaacagagtcgataggccccatagaccgaagtgctgctgcatcgtatcctgctcattatatatttcatgaacatgttgctggttacaataaagatcactctctttttgacaggatgacgtttttatgtatgtcatcaacagatgcatctaaaggtgcatgtccgacaggagaaaactccaaatcctctcaaggggagactaatattaagctaatatttactgaaaagaaaagtctggccagaaaaacattaaacttaaaaggatataagagatttttatatgaatcagatagatgcattcattatgtcgataaaatgaatctcaattctcatactgttaaatgtgtaggttcattcacaagaggagtagatttcactttatatatcccacaaggtgaaattgatgggcttctaactggaggtatatgggaggcaacactagagttacgagtcaaaaggcattacgactataatcatggtacttacaaagttaatatcacagttgatttgacagacaaaggaaatattcaggtctggacaccaaagtttcatagcgatcctagaattgatctgaatttacgtcctgaaggtaatggtaaatattctggtagtaacgtgcttgagatgtgtctctatgatggctatagtacacatagtcaaagtatagaaatgaggtttcaggatgactcacaaacaggaaataatgaatataatcttataaaaactggagagccattaaaaaaattgccatataaactttctcttcttttaggaggacgagagttttatccaaataatggagaggcttttactattaatgatacttcgtcattgtttataaactggaatcgtattaagtctgtatccttaccacagattagtattccagtactatgctggccagcaaacttgacatttatgtcagagctaaataatccagaagcgggtgagtattcaggaatacttaacgtaacatttactcctagtagttcaagcctagacaataaacaagccgagaaaaatatcactgtaactgctagcgttgatccaactatcgatctgatgcaatctgatggcacagcgttaccaagtgcagttaatattgcatatcttccaggagagaaaagatttgaatctgctcgtatcaatacccaagttcataccaataataaaactaagggtattcagataaagcttactaatgataatgtggtaatgactaacttatctgatccaagcaagactattcctttagaggtttcattcgctggcactaagctgagcacagctgcaacatctattactgccgatcaattaaattttggcgcagctggtgtagagacagtttctgcaactaaggaactcgttattaatgcaggaagcacccagcaaactaatattgtagctggtaactatcaaggattggtgtcaattgtgcttactcaagaacctgacaataaacaagccgagaaaaatatcactgtaactgctagcgttgatccgacgggcgagcaaaattttattccagatattgattccgctgttcgtataatacctgttaattacgattcggatccgaaactgaattcacagttatatacggttgagatgacgatccctgcaggtgtaagcgcagttaaaatcgtaccaacagatagtctgacatcttctggacagcagatcggaaagctggttaatgtaaacaatccagatcaaaatatgaattattatatcagaaaggattctggcgctggtaagtttatggcagggcaaaaaggatccttttctgtcaaagagaatacgtcatacacattctcagcaatttatactggtggcgaataccctaatagcggatattcgtctggtacttatgcaggacatttgactgtatcattttacagcaatgacaataaacaaagaacagaaatagcgactaaaaacttcccagtatcaacgactatttcaaaaagtttttttgcgcctgaaccacaaatccagccttcttttggtaaaaatgttggaaaggaaggagatttattatttagtgtgagcttaattgttcctgaaaatgtatcccaggtaacggtctaccctgtttatgatgaagattatggattaggacgactcgtaaataccgctgatgattcccaatcaataatctaccagattgttgatgataaagggaaaaaaatgttaaaagatcatggtacagaggttacgcctaatcaacaaataacttttaaagcgctgaattatactagcggagataaagaaatacctcctgggatatataacgatcaggttatggttggttactacgtaaacgacaataaacaaggaaactggcaatataaatctctggatgtaaatgtaaatattgagcaactcgagcaccaccaccaccaccactga

SEQ ID NO: 31 - protein, 817 aa, Escherichia coli
MQSWHTNVEAGSINKTESIGPIDRSAAASYPAHYIFHEHVAGYNKDHSLFDRMTFLCMSSTDASKGACPTGENSKSSQGETNIKLIFTEKKSLARKTLNLKGYKRFLYESDRCIHYVDKMNLNSHTVKCVGSFTRGVDFTLYIPQGEIDGLLTGGIWEATLELRVKRHYDYNHGTYKVNITVDLTDKGNIQVWTPKFHSDPRIDLNLRPEGNGKYSGSNVLEMCLYDGYSTHSQSIEMRFQDDSQTGNNEYNLIKTGEPLKKLPYKLSLLLGGREFYPNNGEAFTINDTSSLFINWNRIKSVSLPQISIPVLCWPANLTFMSELNNPEAGEYSGILNVTFTPSSSSLDNKQAEKNITVTASVDPTIDLMQSDGTALPSAVNIAYLPGEKRFESARINTQVHTNNKTKGIQIKLTNDNVVMTNLSDPSKTIPLEVSFAGTKLSTAATSITADQLNFGAAGVETVSATKELVINAGSTQQTNIVAGNYQGLVSIVLTQEPDNKQAEKNITVTASVDPTGEQNFIPDIDSAVRIIPVNYDSDPKLNSQLYTVEMTIPAGVSAVKIVPTDSLTSSGQQIGKLVNVNNPDQNMNYYIRKDSGAGKFMAGQKGSFSVKENTSYTFSAIYTGGEYPNSGYSSGTYAGHLTVSFYSNDNKQRTEIATKNFPVSTTISKSFFAPEPQIQPSFGKNVGKEGDLLFSVSLIVPENVSQVTVYPVYDEDYGLGRLVNTADDSQSIIYQIVDDKGKKMLKDHGTEVTPNQQITFKALNYTSGDKEIPPGIYNDQVMVGYYVNDNKQGNWQYKSLDVNVNIEQLEHHHHHH

SEQ ID NO: 32 - DNA, 1848 bp, Escherichia coli
  source 1..1848: mol_type = unassigned DNA
atggcagtgggcccaacgaaagatatgagtttaggtgcaaatttaacttcagagcctacattagctattgattttacgcctattgaaaatatttatgtaggtgccaattatggtaaagatattggaacccttgttttcacaacaaatgatttaacagatattacattgatgtcatctcgcagcgttgttgatggtcgccagactggtttttttaccttcatggactcatcagccacttacaaaattagtacaaaactgggatcatcgaatgatgtaaacattcaagaaattactcaaggagctaaaattactcctgttagtggagagaaaactttgcctaaaaaattcactcttaagctacatgcacacaggagtagcagtacagttccaggtacgtatactgttggtcttaacgtaaccagtaacgttattgataacaagcaggcagcggggcccactctaaccaaagaactggcattaaatgtgctttctcctgcagctctggatgcaacttgggctcctcaggataatttaacattatccaatactggcgtttctaatactttggtgggtgttttgactctttcaaataccagtattgatacagttagcattgcgagtacaaatgtttctgatacatctaagaatggtacagtaacttttgcacatgagacaaataactctgctagctttgccaccaccatttcaacagataatgccaacattacgttggataaaaatgctggaaatacgattgttaaaactacaaatgggagtcagttgccaactaatttaccacttaagtttattaccactgaaggtaacgaacatttagtttcaggtaattaccgtgcaaatataacaattacttcgacaattaaagataacaagcaggcggcaggtccaaccctgactaaggagttagcgctgaacgttttaagcggcgagcaaaattttattccagatattgattccgctgttcgtataatacctgttaattacgattcggatccgaaactgaattcacagttatatacggttgagatgacgatccctgcaggtgtaagcgcagttaaaatcgtaccaacagatagtctgacatcttctggacagcagatcggaaagctggttaatgtaaacaatccagatcaaaatatgaattattatatcagaaaggattctggcgctggtaagtttatggcagggcaaaaaggatccttttctgtcaaagagaatacgtcatacacattctcagcaatttatactggtggcgaataccctaatagcggatattcgtctggtacttatgcaggacatttgactgtatcattttacagcaatgacaataaacaaagaacagaaatagcgactaaaaacttcccagtatcaacgactatttcaaaaagtttttttgcgcctgaaccacaaatccagccttcttttggtaaaaatgttggaaaggaaggagatttattatttagtgtgagcttaattgttcctgaaaatgtatcccaggtaacggtctaccctgtttatgatgaagattatggattaggacgactcgtaaataccgctgatgattcccaatcaataatctaccagattgttgatgataaagggaaaaaaatgttaaaagatcatggtacagaggttacgcctaatcaacaaataacttttaaagcgctgaattatactagcggagataaagaaatacctcctgggatatataacgatcaggttatggttggttactacgtaaacgacaataaacaaggaaactggcaatataaatctctggatgtaaatgtaaatattgagcaactcgagcaccaccaccaccaccactga

SEQ ID NO: 33 - protein, 615 aa, Escherichia coli
MAVGPTKDMSLGANLTSEPTLAIDFTPIENIYVGANYGKDIGTLVFTTNDLTDITLMSSRSVVDGRQTGFFTFMDSSATYKISTKLGSSNDVNIQEITQGAKITPVSGEKTLPKKFTLKLHAHRSSSTVPGTYTVGLNVTSNVIDNKQAAGPTLTKELALNVLSPAALDATWAPQDNLTLSNTGVSNTLVGVLTLSNTSIDTVSIASTNVSDTSKNGTVTFAHETNNSASFATTISTDNANITLDKNAGNTIVKTTNGSQLPTNLPLKFITTEGNEHLVSGNYRANITITSTIKDNKQAAGPTLTKELALNVLSGEQNFIPDIDSAVRIIPVNYDSDPKLNSQLYTVEMTIPAGVSAVKIVPTDSLTSSGQQIGKLVNVNNPDQNMNYYIRKDSGAGKFMAGQKGSFSVKENTSYTFSAIYTGGEYPNSGYSSGTYAGHLTVSFYSNDNKQRTEIATKNFPVSTTISKSFFAPEPQIQPSFGKNVGKEGDLLFSVSLIVPENVSQVTVYPVYDEDYGLGRLVNTADDSQSIIYQIVDDKGKKMLKDHGTEVTPNQQITFKALNYTSGDKEIPPGIYNDQVMVGYYVNDNKQGNWQYKSLDVNVNIEQLEHHHHHH

SEQ ID NO: 34 - DNA, 1794 bp, Escherichia coli
  source 1..1794: mol_type = unassigned DNA
atggagcaaaattttattccagatattgattccgctgttcgtataatacctgttaattacgattcggatccgaaactgaattcacagttatatacggttgagatgacgatccctgcaggtgtaagcgcagttaaaatcgtaccaacagatagtctgacatcttctggacagcagatcggaaagctggttaatgtaaacaatccagatcaaaatatgaattattatatcagaaaggattctggcgctggtaagtttatggcagggcaaaaaggatccttttctgtcaaagagaatacgtcatacacattctcagcaatttatactggtggcgaataccctaatagcggatattcgtctggtacttatgcaggacatttgactgtatcattttacagcaatgacaataaacaaagaacagaaatagcgactaaaaacttcccagtatcaacgactatttcaaaaagtttttttgcgcctgaaccacaaatccagccttcttttggtaaaaatgttggaaaggaaggagatttattatttagtgtgagcttaattgttcctgaaaatgtatcccaggtaacggtctaccctgtttatgatgaagattatggattaggacgactcgtaaataccgctgatgattcccaatcaataatctaccagattgttgatgataaagggaaaaaaatgttaaaagatcatggtacagaggttacgcctaatcaacaaataacttttaaagcgctgaattatactagcggagataaagaaatacctcctgggatatataacgatcaggttatggttggttactacgtaaacgacaataaacaaggaaactggcaatataaatctctggacgtgaatgtaaatattgagcaaggcacattagctattgattttacgcctattgaaaatatttatgtaggtgccaattatggtaaagatattggaacccttgttttcacaacaaatgatttaacagatattacattgatgtcatctcgcagcgttgttgatggtcgccagactggtttttttaccttcatggactcatcagccacttacaaaattagtacaaaactgggatcatcgaatgatgtaaacattcaagaaattactcaaggagctaaaattactcctgttagtggagagaaaactttgcctaaaaaattcactcttaagctacatgcacacaggagtagcagtacagttccaggtacgtatactgttggtcttaacgtaaccagtaacgttattgataacaagcaggcagcggggcccactctaaccaaagaactggcattaaatgtgctttctcctgcagctctggatgcaacttgggctcctcaggataatttaacattatccaatactggcgtttctaatactttggtgggtgttttgactctttcaaataccagtattgatacagttagcattgcgagtacaaatgtttctgatacatctaagaatggtacagtaacttttgcacatgagacaaataactctgctagctttgccaccaccatttcaacagataatgccaacattacgttggataaaaatgctggaaatacgattgttaaaactacaaatgggagtcagttgccaactaatttaccacttaagtttattaccactgaaggtaacgaacatttagtttcaggtaattaccgtgcaaatataacaattacttcgacaattaaagataacaagcaggcggcaggtccaaccctgactaaggagttagcgctgaacgttctgagcctcgagcaccaccaccaccaccactga

SEQ ID NO: 35 - protein, 597 aa, Escherichia coli
MEQNFIPDIDSAVRIIPVNYDSDPKLNSQLYTVEMTIPAGVSAVKIVPTDSLTSSGQQIGKLVNVNNPDQNMNYYIRKDSGAGKFMAGQKGSFSVKENTSYTFSAIYTGGEYPNSGYSSGTYAGHLTVSFYSNDNKQRTEIATKNFPVSTTISKSFFAPEPQIQPSFGKNVGKEGDLLFSVSLIVPENVSQVTVYPVYDEDYGLGRLVNTADDSQSIIYQIVDDKGKKMLKDHGTEVTPNQQITFKALNYTSGDKEIPPGIYNDQVMVGYYVNDNKQGNWQYKSLDVNVNIEQGTLAIDFTPIENIYVGANYGKDIGTLVFTTNDLTDITLMSSRSVVDGRQTGFFTFMDSSATYKISTKLGSSNDVNIQEITQGAKITPVSGEKTLPKKFTLKLHAHRSSSTVPGTYTVGLNVTSNVIDNKQAAGPTLTKELALNVLSPAALDATWAPQDNLTLSNTGVSNTLVGVLTLSNTSIDTVSIASTNVSDTSKNGTVTFAHETNNSASFATTISTDNANITLDKNAGNTIVKTTNGSQLPTNLPLKFITTEGNEHLVSGNYRANITITSTIKDNKQAAGPTLTKELALNVLSLEHHHHHH

SEQ ID NO: 36 - DNA, 1104 bp, Escherichia coli
  source 1..1104: mol_type = unassigned DNA
atgaaatacctgctgccgaccgctgctgctggtctgctgctcctcgctgcccagccggcgatggccatggcagtgggcccaacgaaagatatgagtttaggtgcaaatttaacttcagagcctacattagctattgattttacgcctattgaaaatatttatgtaggtgccaattatggtaaagatattggaacccttgttttcacaacaaatgatttaacagatattacattgatgtcatctcgcagcgttgttgatggtcgccagactggtttttttaccttcatggactcatcagccacttacaaaattagtacaaaactgggatcatcgaatgatgtaaacattcaagaaattactcaaggagctaaaattactcctgttagtggagagaaaactttgcctaaaaaattcactcttaagctacatgcacacaggagtagcagtacagttccaggtacgtatactgttggtcttaacgtaaccagtaacgttattgataacaagcaggcagcggggcccactctaaccaaagaactggcattaaatgtgctttctcctgcagctctggatgcaacttgggctcctcaggataatttaacattatccaatactggcgtttctaatactttggtgggtgttttgactctttcaaataccagtattgatacagttagcattgcgagtacaaatgtttctgatacatctaagaatggtacagtaacttttgcacatgagacaaataactctgctagctttgccaccaccatttcaacagataatgccaacattacgttggataaaaatgctggaaatacgattgttaaaactacaaatgggagtcagttgccaactaatttaccacttaagtttattaccactgaaggtaacgaacatttagtttcaggtaattaccgtgcaaatataacaattacttcgacaattaaagataacaagcaggcggcaggtccaaccctgactaaggagttagcgctgaacgttctatcgatacttgacgaataccaatctaaagttaaaagacaaatattttcaggctatcaatctgatattgatacacataatagaattaaggatgaattatga

SEQ ID NO: 37 - protein, 367 aa, Escherichia coli
MKYLLPTAAAGLLLLAAQPAMAMAVGPTKDMSLGANLTSEPTLAIDFTPIENIYVGANYGKDIGTLVFTTNDLTDITLMSSRSVVDGRQTGFFTFMDSSATYKISTKLGSSNDVNIQEITQGAKITPVSGEKTLPKKFTLKLHAHRSSSTVPGTYTVGLNVTSNVIDNKQAAGPTLTKELALNVLSPAALDATWAPQDNLTLSNTGVSNTLVGVLTLSNTSIDTVSIASTNVSDTSKNGTVTFAHETNNSASFATTISTDNANITLDKNAGNTIVKTTNGSQLPTNLPLKFITTEGNEHLVSGNYRANITITSTIKDNKQAAGPTLTKELALNVLSILDEYQSKVKRQIFSGYQSDIDTHNRIKDEL

SEQ ID NO: 38 - DNA, 381 bp, Escherichia coli
  source 1..381: mol_type = unassigned DNA
atgagctttaagaaaattatcaaggcatttgttatcatggctgctttggtatctgttcaggcgcatgccgctccccagtctattacagaactatgttcggaatatcacaacacacaaatatatacgataaatgacaagatactatcatatacggaatccatggcaggcaaaagagaaatggttatcattacatttaagagcggcgcaacatttcaggtcgaagtcccgggcagtcaacatatagactcccaaaaaaaagccattgaaaggatgaaggacacattaagaatcgcatatctgaccgagaccaaaattgataaattatgtgtatggaataataaaaccccgcattcaattgcggcaatcagtatggaaaactaa

SEQ ID NO: 39 - protein, 126 aa, Escherichia coli
MSFKKIIKAFVIMAALVSVQAHAAPQSITELCSEYHNTQIYTINDKILSYTESMAGKREMVIITFKSGATFQVEVPGSQHIDSQKKAIERMKDTLRIAYLTETKIDKLCVWNNKTPHSIAAISMEN

SEQ ID NO: 40 - DNA, 1038 bp, Escherichia coli
  source 1..1038: mol_type = unassigned DNA
atgaaatacctgctgccgaccgctgctgctggtctgctgctcctcgctgcccagccggcgatggccatgtcaaaaagtttttttgcacctgaaccacgaatacagccttcttttggtgaaaatgttggaaaggaaggagctttattatttagtgtgaacttaactgttcctgaaaatgtatcccaggtaacggtctaccctgtttatgatgaagattatgggttaggacgactagtaaataccgctgatgcttcccaatcaataatctaccagattgttgatgagaaagggaaaaaaatgttaaaagatcatggtgcagaggttacacctaatcaacaaataacttttaaagcgctgaattatactagcggggaaaaaaaaatatctcctggaatatataacgatcaggttatggttggttactacgtcaacgacaataaacaaggaaactggcaatataaatctctggatgtaaatgtaaatattgagcaaaattttattccagatattgattccgctgttcgtataatacctgttaattacgattcggacccgaaactggattcacagttatatacggttgagatgacgatccctgcaggtgtaagcgcagttaaaatcgcaccaacagatagtctgacatcttctggacagcagatcggaaagctggttaatgtaaacaatccagatcaaaatatgaattattatatcagaaaggattctggcgctggtaactttatggcaggacaaaaaggatcctttcctgtcaaagagaatacgtcatacacattctcagcaatttatactggtggcgaataccctaatagcggatattcgtctggtacttatgcaggaaatttgactgtatcattttacagcaatgacaataaacaaagaacagaaatagcgactaaaaacttcccagtatcaacgactatatcgatacttgacgaataccaatctaaagttaaaagacaaatattttcaggctatcaatctgatattgatacacataatagaattaaggatgaattatga

SEQ ID NO: 41 - protein, 347 aa, Escherichia coli
MKYLLPTAAAGLLLLAAQPAMAMEQNFIPDIDSAVRIIPVNYDSDPKLNSQLYTVEMTIPAGVSAVKIVPTDSLTSSGQQIGKLVNVNNPDQNMNYYIRKDSGAGKFMAGQKGSFSVKENTSYTFSAIYTGGEYPNSGYSSGTYAGHLTVSFYSNDNKQRTEIATKNFPVSTTISKSFFAPEPQIQPSFGKNVGKEGDLLFSVSLIVPENVSQVTVYPVYDEDYGLGRLVNTADDSQSIIYQIVDDKGKKMLKDHGTEVTPNQQITFKALNYTSGDKEIPPGIYNDQVMVGYYVNDNKQGNWQYKSLDVNVNIEQSILDEYQSKVKRQIFSGYQSDIDTHNRIKDEL

SEQ ID NO: 42 - DNA, 1038 bp, Escherichia coli; identical to SEQ ID NO: 40
  source 1..1038: mol_type = unassigned DNA

SEQ ID NO: 43 - protein, 345 aa, Escherichia coli
MKYLLPTAAAGLLLLAAQPAMAMSKSFFAPEPRIQPSFGENVGKEGALLFSVNLTVPENVSQVTVYPVYDEDYGLGRLVNTADASQSIIYQIVDEKGKKMLKDHGAEVTPNQQITFKALNYTSGEKKISPGIYNDQVMVGYYVNDNKQGNWQYKSLDVNVNIEQNFIPDIDSAVRIIPVNYDSDPKLDSQLYTVEMTIPAGVSAVKIAPTDSLTSSGQQIGKLVNVNNPDQNMNYYIRKDSGAGNFMAGQKGSFPVKENTSYTFSAIYTGGEYPNSGYSSGTYAGNLTVSFYSNDNKQRTEIATKNFPVSTTISILDEYQSKVKRQIFSGYQSDIDTHNRIKDEL

SEQ ID NO: 44 - DNA, 1092 bp, Escherichia coli
  source 1..1092: mol_type = unassigned DNA
atgaaaaagatatttatttttttgtctatcatattttctgcggtggtcagtgccgggcgatacccggaaactacagtaggtaatctgacgaagagttttcaagcccctcgtcaggatagaagcgtacaatcaccaatatataacatctttacgaatcatgtggctggatatagtttgagtcataacttatatgacaggattgtttttttatgtacatcctcgtcgaatccggttaatggtgcttgcccaaccattggaacatctggagttcaatacggtactacaaccataaccttgcagtttacagaaaaaagaagtctgataaaaagaaatattaatcttgcaggtaataagaaaccaatatgggagaatcagagttgcgacactagcaatctaatggtgttgaattcgaagtcttggtcctgtggggcttacggaaatgctaacggaacacttctaaatctgtatatccctgcaggagaaatcaacaaattgccttttggagggatatgggaggcaactctgatcttacgcttatcaagatatggcgaagtcagtagcacccattacggcaattataccgtaaatattacggttgatttaactgataaaggtaatattcaggtatggcttccagggtttcacagcaacccgcgtgtagacctgaatctgcaccctatcggtaattataaatatagtggtagtaattcactcgacatgtgtttctatgatggatatagtacaaacagtgatagcatggtaataaagttccaggatgataatcctacctattcatctgaatataatctttataagatagggggcactgaaaaattaccatatgctgtttcactgcttatgggagaaaaaatattttatccagtgaatggtcaatcatttactatcaatgacagtagtgtactcgaaacaaactggaatcgagtaaccgcagttgctatgccggaagttaatgttccagtattatgctggccagcaagattgctattaaatgctgatgtaaatgctcccgatgcaggacagtattcaggacagatatatataacatttacacccagtgtcgaaaatttatga

SEQ ID NO: 45 - protein, 363 aa, Escherichia coli
MKKIFIFLSIIFSAVVSAGRYPETTVGNLTKSFQAPRQDRSVQSPIYNIFTNHVAGYSLSHNLYDRIVFLCTSSSNPVNGACPTIGTSGVQYGTTTITLQFTEKRSLIKRNINLAGNKKPIWENQSCDTSNLMVLNSKSWSCGAYGNANGTLLNLYIPAGEINKLPFGGIWEATLILRLSRYGEVSSTHYGNYTVNITVDLTDKGNIQVWLPGFHSNPRVDLNLHPIGNYKYSGSNSLDMCFYDGYSTNSDSMVIKFQDDNPTYSSEYNLYKIGGTEKLPYAVSLLMGEKIFYPVNGQSFTINDSSVLETNWNRVTAVAMPEVNVPVLCWPARLLLNADVNAPDAGQYSGQIYITFTPSVENL

SEQ ID NO: 46 - protein, 345 aa, Escherichia coli
GRYPETTVGNLTKSFQAPRQDRSVQSPIYNIFTNHVAGYSLSHNLYDRIVFLCTSSSNPVNGACPTIGTSGVQYGTTTITLQFTEKRSLIKRNINLAGNKKPIWENQSCDTSNLMVLNSKSWSCGAYGNANGTLLNLYIPAGEINKLPFGGIWEATLILRLSRYGEVSSTHYGNYTVNITVDLTDKGNIQVWLPGFHSNPRVDLNLHPIGNYKYSGSNSLDMCFYDGYSTNSDSMVIKFQDDNPTYSSEYNLYKIGGTEKLPYAVSLLMGEKIFYPVNGQSFTINDSSVLETNWNRVTAVAMPEVNVPVLCWPARLLLNADVNAPDAGQYSGQIYITFTPSVENL

SEQ ID NO: 47 - DNA, 507 bp, Escherichia coli
  source 1..507: mol_type = unassigned DNA
atgaaactgaagaaaacaattggcgcaatggctatggcgactctgtttgccaccatggctgcctctgcagtcgaaaaaaatattactgtgagggcaagtgttgaccctaaacttgatcttctgcaagcagatggaacttcactgccggactctatcgcattaacctattcttcggcttcaaataattttgaagtttactctcttaatactgctattcatacaaatgacaaaagcaagggagttgtagtgaagctgtcagcttcaccagttctgtccaatattatgaagccaaactcgcaaattccgatgaaagtgactttgggggggaagacgctgaatacaactgatactgagtttactgttgatactctgaactttggtacatctggtgttgaaaacgtttcttccactcaacagcttacgattcatgcagacacacaaggaactgcgcctgaggcaggcaattaccaaggtattatttctcttatcatgactcaaaaaacttaa

SEQ ID NO: 48 - protein, 168 aa, Escherichia coli
MKLKKTIGAMAMATLFATMAASAVEKNITVRASVDPKLDLLQADGTSLPDSIALTYSSASNNFEVYSLNTAIHTNDKSKGVVVKLSASPVLSNIMKPNSQIPMKVTLGGKTLNTTDTEFTVDTLNFGTSGVENVSSTQQLTIHADTQGTAPEAGNYQGIISLIMTQKT

SEQ ID NO: 49 - protein, 145 aa, Escherichia coli
VEKNITVRASVDPKLDLLQADGTSLPDSIALTYSSASNNFEVYSLNTAIHTNDKSKGVVVKLSASPVLSNIMKPNSQIPMKVTLGGKTLNTTDTEFTVDTLNFGTSGVENVSSTQQLTIHADTQGTAPEAGNYQGIISLIMTQKT

SEQ ID NO: 50 - DNA, 1095 bp, Escherichia coli
  source 1..1095: mol_type = unassigned DNA
ttgaaaaaagtgatttttgttttatccatgtttctatgttctcaggtttacgggcaatcatggcatacgaacgtagaggctggttcaataaataaaacagagtcgataggccccatagaccgaagtgctgctgcatcgtatcctgctcattatatatttcatgaacatgttgctggttacaataaagatcactctctttttgacaggatgacgtttttatgtatgtcatcaacagatgcatctaaaggtgcatgtccgacaggagaaaactccaaatcctctcaaggggagactaatattaagctaatatttactgaaaagaaaagtctggccagaaaaacattaaacttaaaaggatataagagatttttatatgaatcagatagatgcattcattatgtcgataaaatgaatctcaattctcatactgttaaatgtgtaggttcattcacaagaggagtagatttcactttatatatcccacaaggtgaaattgatgggcttctaactggaggtatatgggaggcaacactagagttacgagtcaaaaggcattacgactataatcatggtacttacaaagttaatatcacagttgatttgacagacaaaggaaatattcaggtctggacaccaaagtttcatagcgatcctagaattgatctgaatttacgtcctgaaggtaatggtaaatattctggtagtaacgtgcttgagatgtgtctctatgatggctatagtacacatagtcaaagtatagaaatgaggtttcaggatgactcacaaacaggaaataatgaatataatcttataaaaactggagagccattaaaaaaattgccatataaactttctcttcttttaggaggacgagagttttatccaaataatggagaggcttttactattaatgatacttcgtcattgtttataaactggaatcgtattaagtctgtatccttaccacagattagtattccagtactatgctggccagcaaacttgacatttatgtcagagctaaataatccagaagcgggtgagtattcaggaatacttaacgtaacatttactcctagtagttcaagtctgtaa

SEQ ID NO: 51 - protein, 364 aa, Escherichia coli
LKKVIFVLSMFLCSQVYGQSWHTNVEAGSINKTESIGPIDRSAAASYPAHYIFHEHVAGYNKDHSLFDRMTFLCMSSTDASKGACPTGENSKSSQGETNIKLIFTEKKSLARKTLNLKGYKRFLYESDRCIHYVDKMNLNSHTVKCVGSFTRGVDFTLYIPQGEIDGLLTGGIWEATLELRVKRHYDYNHGTYKVNITVDLTDKGNIQVWTPKFHSDPRIDLNLRPEGNGKYSGSNVLEMCLYDGYSTHSQSIEMRFQDDSQTGNNEYNLIKTGEPLKKLPYKLSLLLGGREFYPNNGEAFTINDTSSLFINWNRIKSVSLPQISIPVLCWPANLTFMSELNNPEAGEYSGILNVTFTPSSSSL

SEQ ID NO: 52 - protein, 346 aa, Escherichia coli
QSWHTNVEAGSINKTESIGPIDRSAAASYPAHYIFHEHVAGYNKDHSLFDRMTFLCMSSTDASKGACPTGENSKSSQGETNIKLIFTEKKSLARKTLNLKGYKRFLYESDRCIHYVDKMNLNSHTVKCVGSFTRGVDFTLYIPQGEIDGLLTGGIWEATLELRVKRHYDYNHGTYKVNITVDLTDKGNIQVWTPKFHSDPRIDLNLRPEGNGKYSGSNVLEMCLYDGYSTHSQSIEMRFQDDSQTGNNEYNLIKTGEPLKKLPYKLSLLLGGREFYPNNGEAFTINDTSSLFINWNRIKSVSLPQISIPVLCWPANLTFMSELNNPEAGEYSGILNVTFTPSSSSL

SEQ ID NO: 53 - DNA, 513 bp, Escherichia coli
  source 1..513: mol_type = unassigned DNA
atgaaactcaataagattattggagcattagttctttcatctacatttgttagcatgggggcttctgctgccgagaaaaatatcactgtaactgctagcgttgatccaactatcgatctgatgcaatctgatggcacagcgttaccaagtgcagttaatattgcatatcttccaggagagaaaagatttgaatctgctcgtatcaatacccaagttcataccaataataaaactaagggtattcagataaagcttactaatgataatgtggtaatgactaacttatctgatccaagcaagactattcctttagaggtttcattcgctggcactaagctgagcacagctgcaacatctattactgccgatcaattaaattttggcgcagctggtgtagagacagtttctgcaactaaggaactcgttattaatgcaggaagcacccagcaaactaatattgtagctggtaactatcaaggattggtgtcaattgtgcttactcaagaaccttaa

SEQ ID NO: 54 - protein, 170 aa, Escherichia coli
MKLNKIIGALVLSSTFVSMGASAAEKNITVTASVDPTIDLMQSDGTALPSAVNIAYLPGEKRFESARINTQVHTNNKTKGIQIKLTNDNVVMTNLSDPSKTIPLEVSFAGTKLSTAATSITADQLNFGAAGVETVSATKELVINAGSTQQTNIVAGNYQGLVSIVLTQEP

SEQ ID NO: 55 - protein, 147 aa, Escherichia coli
AEKNITVTASVDPTIDLMQSDGTALPSAVNIAYLPGEKRFESARINTQVHTNNKTKGIQIKLTNDNVVMTNLSDPSKTIPLEVSFAGTKLSTAATSITADQLNFGAAGVETVSATKELVINAGSTQQTNIVAGNYQGLVSIVLTQEP

SEQ ID NO: 56 - DNA, 1083 bp, Escherichia coli
  source 1..1083: mol_type = unassigned DNA
atgaataaaattttatttatttttacattgtttttttcttcagggttttttacatttgccgtatcggcagataaaaatcccggaagtgaaaacatgactaatactattggtccccatgacagggggggatcttcccccatatataatatcttaaattcctatcttacagcatacaatggaagccatcatctgtatgataggatgagttttttatgtttgtcttctcaaaatacactgaatggagcatgcccaagcagtgatgcccctggcactgctacaattgatggcgaaacaaatataacattacaatttacggaaaaaagaagtctaattaaaagagaactgcaaattaaaggctataaacaatttttgttcaaaaatgctaattgcccatctaaactagcacttaactcatctcattttcaatgtaatagagaacaagcttcaggtgctactttatcgttatacataccagctggtgaattaaataaattaccttttgggggggtctggaatgccgttctgaagctaaatgtaaaaagacgatatgatacaacctatgggacttacactataaacatcacagttaatttaactgataagggaaatattcagatatggttaccacagttcaaaagtaacgctcgtgtcgatcttaacttgcgtccaactggtggtggtacatatatcggaagaaattctgttgatatgtgcttttatgatggatatagtactaacagcagctctttggagataagatttcaggatgataattctaaatctgatggaaaattttatctaaagaaaataaatgatgactccaaagaacttgtatacactttgtcacttctcctggcaggtaaaaatttaacaccaacaaatggacaggcattaaatattaacactgcttctctggaaacaaactggaatagaattacagctgtcaccatgccagaaatcagtgttccggtgttgtgttggcctggacgtttgcaattggatgcaaaagtgaaaaatcccgaggctggacaatatatggggaatattaaaattactttcacaccaagtagtcaaacactctag

SEQ ID NO: 57 - protein, 360 aa, Escherichia coli
MNKILFIFTLFFSSGFFTFAVSADKNPGSENMTNTIGPHDRGGSSPIYNILNSYLTAYNGSHHLYDRMSFLCLSSQNTLNGACPSSDAPGTATIDGETNITLQFTEKRSLIKRELQIKGYKQFLFKNANCPSKLALNSSHFQCNREQASGATLSLYIPAGELNKLPFGGVWNAVLKLNVKRRYDTTYGTYTINITVNLTDKGNIQIWLPQFKSNARVDLNLRPTGGGTYIGRNSVDMCFYDGYSTNSSSLEIRFQDDNSKSDGKFYLKKINDDSKELVYTLSLLLAGKNLTPTNGQALNINTASLETNWNRITAVTMPEISVPVLCWPGRLQLDAKVKNPEAGQYMGNIKITFTPSSQTL

SEQ ID NO: 58 - protein, 338 aa, Escherichia coli
ADKNPGSENMTNTIGPHDRGGSSPIYNILNSYLTAYNGSHHLYDRMSFLCLSSQNTLNGACPSSDAPGTATIDGETNITLQFTEKRSLIKRELQIKGYKQFLFKNANCPSKLALNSSHFQCNREQASGATLSLYIPAGELNKLPFGGVWNAVLKLNVKRRYDTTYGTYTINITVNLTDKGNIQIWLPQFKSNARVDLNLRPTGGGTYIGRNSVDMCFYDGYSTNSSSLEIRFQDDNSKSDGKFYLKKINDDSKELVYTLSLLLAGKNLTPTNGQALNINTASLETNWNRITAVTMPEISVPVLCWPGRLQLDAKVKNPEAGQYMGNIKITFTPSSQTL

SEQ ID NO: 59 - DNA, 513 bp, Escherichia coli
  source 1..513: mol_type = unassigned DNA
atgaaatttaaaaaaactattggtgcaatggctctgaccacaatgtttgtagcagtgagtgcttcagcagtagagaaaaatattactgtaacagctagtgttgatcctgcaattgatcttttgcaagctgatggcaatgctctgccatcagctgtaaagttagcttattctcccgcatcaaaaacttttgaaagttacagagtaatgactcaagttcatacaaacgatgcaactaaaaaagtaattgttaaacttgctgatacaccacagcttacagatgttctgaattcaactgttcaaatgcctatcagtgtgtcatggggaggacaagtattatctacaacagccaaagaatttgaagctgctgctttgggatattctgcatccggtgtaaatggcgtatcatcttctcaagagttagtaattagcgctgcacctaaaactgccggtaccgccccaactgcaggaaactattcaggagtagtatctcttgtaatgactttgggatcctga

SEQ ID NO: 60 - protein, 170 aa, Escherichia coli
MKFKKTIGAMALTTMFVAVSASAVEKNITVTASVDPAIDLLQADGNALPSAVKLAYSPASKTFESYRVMTQVHTNDATKKVIVKLADTPQLTDVLNSTVQMPISVSWGGQVLSTTAKEFEAAALGYSASGVNGVSSSQELVISAAPKTAGTAPTAGNYSGVVSLVMTLGS

SEQ ID NO: 61 - protein, 147 aa, Escherichia coli
VEKNITVTASVDPAIDLLQADGNALPSAVKLAYSPASKTFESYRVMTQVHTNDATKKVIVKLADTPQLTDVLNSTVQMPISVSWGGQVLSTTAKEFEAAALGYSASGVNGVSSSQELVISAAPKTAGTAPTAGNYSGVVSLVMTLGS

SEQ ID NO: 62 - DNA, 504 bp, Escherichia coli
  source 1..504: mol_type = unassigned DNA
atgaaattaaaaaaaactattggtgcaatggcactgaccacaatgtttgtagctatgagtgcttctgcagtagagaaaaatatcactgtaacagctagtgttgatcctacaattgatattttgcaagctgatggtagtagtttacctactgctgtagaattaacctattcacctgcggcaagtcgttttgaaaattataaaatcgcaactaaagttcatacaaatgttataaataaaaatgtactagttaagcttgtaaatgatccaaaacttacaaatgttttggattctacaaaacaactccccattactgtatcatatggaggaaagactctatcaaccgcagatgtgacttttgaacctgcagaattaaattttggaacgtcaggtgtaactggtgtatcttcttcccaagatttagtgattggtgcgactacagcacaagcaccaacggcgggaaattatagtggggtcgtttctatcttaatgaccttagcatcataa

SEQ ID NO: 63 - protein, 167 aa, Escherichia coli
MKLKKTIGAMALTTMFVAMSASAVEKNITVTASVDPTIDILQADGSSLPTAVELTYSPAASRFENYKIATKVHTNVINKNVLVKLVNDPKLTNVLDSTKQLPITVSYGGKTLSTADVTFEPAELNFGTSGVTGVSSSQDLVIGATTAQAPTAGNYSGVVSILMTLAS

SEQ ID NO: 64 - DNA, 1086 bp, Escherichia coli
  source 1..1086: mol_type = unassigned DNA
atgaataagattttatttatttttacattgtttttctcttcagtactttttacatttgctgtatcggcagataaaattcccggagatgaaagcataactaatatttttggcccgcgtgacaggaacgaatcttcccccaaacataatatattaaataaccatattacagcatacagtgaaagtcatactctgtatgataggatgacttttttatgtttgtcttctcacaatacacttaatggagcatgtccaaccagtgagaatcctagcagttcatcggtcagcggtgaaacaaatataacattacaatttacggaaaaaagaagtttaataaaaagagagctacaaattaaaggctataaacaattattgttcaaaagtgttaactgcccatccggcctaacacttaactcagctcattttaactgtaataaaaacgcggcttcaggtgcaagtttatatttatatattcctgctggcgaactaaaaaatttgccttttggtggtatctgggatgctactctgaagttaagagtaaaaagacgatatagtgagacctatggaacttacactataaatatcactattaaattaactgataagggaaatattcagatatggttacctcagttcaaaagtgacgctcgcgtcgatcttaacttgcgtccaactggtgggggcacatatattggaagaaattctgttgatatgtgcttttatgatggatatagtactaacagcagctctttggagataagatttcaggataacaatcctaaatctgatgggaaattttatctaaggaaaataaatgatgacaccaaagaaattgcatatactttgtcacttctcttggcgggtaaaagtttaactccaacaaatggaacgtcattaaatattgctgacgcagcttctctggaaacaaactggaatagaattacagctgtcaccatgccagaaatcagtgttccggtgttgtgttggcctggacgtttgcaattggatgcaaaagtggaaaatcccgaggctggacaatatatgggtaatattaatgttactttcacaccaagtagtcaaacactctag

SEQ ID NO: 65 - protein, 361 aa, Escherichia coli
MNKILFIFTLFFSSVLFTFAVSADKIPGDESITNIFGPRDRNESSPKHNILNNHITAYSESHTLYDRMTFLCLSSHNTLNGACPTSENPSSSSVSGETNITLQFTEKRSLIKRELQIKGYKQLLFKSVNCPSGLTLNSAHFNCNKNAASGASLYLYIPAGELKNLPFGGIWDATLKLRVKRRYSETYGTYTINITIKLTDKGNIQIWLPQFKSDARVDLNLRPTGGGTYIGRNSVDMCFYDGYSTNSSSLEIRFQDNNPKSDGKFYLRKINDDTKEIAYTLSLLLAGKSLTPTNGTSLNIADAASLETNWNRITAVTMPEISVPVLCWPGRLQLDAKVENPEAGQYMGNINVTFTPSSQTL

SEQ ID NO: 66 - DNA, 510 bp, Escherichia coli
  source 1..510: mol_type = unassigned DNA
atgaaattaaaaaaaactattggcgcaatggctctgagcacaatatttgtagcggtgagtgcttcagcagtagagaaaaatattactgtgacagccagtgttgatcctactattgatattcttcaagcaaatggttctgcgctaccgacagctgtagatttaacttatctacctggtgcaaaaacttttgaaaattacagtgttctaacccagatttacacaaatgacccttcaaaaggtttagatgttcgactggttgatacaccgaaacttacaaatattttgcaaccgacatctaccattcctcttactgtctcatgggcagggaggacattaagtacaagtgctcagaagatcgcagttggcgatctgggttttggttccaccggaacggcaggtgtttcgaatagtaaagaattagtaattggagcaactacatccggaactgcaccaagtgcaggtaagtatcaaggcgtcgtttccattgtaatgactcaatcgacaaactaa

SEQ ID NO: 67 - protein, 169 aa, Escherichia coli
MKLKKTIGAMALSTIFVAVSASAVEKNITVTASVDPTIDILQANGSALPTAVDLTYLPGAKTFENYSVLTQIYTNDPSKGLDVRLVDTPKLTNILQPTSTIPLTVSWAGRTLSTSAQKIAVGDLGFGSTGTAGVSNSKELVIGATTSGTAPSAGKYQGVVSIVMTQSTN

SEQ ID NO: 68 - DNA, 528 bp, Escherichia coli
  source 1..528: mol_type = unassigned DNA
atgaaattaaaaaaaactattggcgcaatggctctgagcacaatgtttgtagcggtgagtgcttcagcagtagagaaaaatattactgtgacagccagtgttgatcctactattgatattcttcaagcaaatggttctgcgctaccgacagctgtagatttaacttatctacctggtgcaaaaacttttgaaaattacagtgttctaacccagatttacacaaatgacccttcaaaaggtttagatgttcgactggttgatacaccgaaacttacaaatattttgcaaccgacatctaccattcctcttactgtctcatgggcagggaagacattaagtacaagtgctcagaagattgcagttggcgatctgggttttggttccaccggaacggcaggtgtttcgaatagtaaagaattagtaattggagcaactacatccggaactgcaccaagtgcaggtaagtatcaaggcgtcgtttccattgtaatgactcaatcgacagacacagccgcgcctgttccttaa

SEQ ID NO: 69 - protein, 175 aa, Escherichia coli
MKLKKTIGAMALSTMFVAVSASAVEKNITVTASVDPTIDILQANGSALPTAVDLTYLPGAKTFENYSVLTQIYTNDPSKGLDVRLVDTPKLTNILQPTSTIPLTVSWAGKTLSTSAQKIAVGDLGFGSTGTAGVSNSKELVIGATTSGTAPSAGKYQGVVSIVMTQSTDTAAPVP

SEQ ID NO: 70 - DNA, 1086 bp, Escherichia coli
  source 1..1086: mol_type = unassigned DNA
atgaataagattttatttatttttacattgtttttctcttcagtactttttacatttgctgtatcggcagataaaattcccggagatgagaatataactaatatttttggcccgcgtgacaggaacgaatcttcccccaaacataatatattaaatgactatattacagcatacagtgaaagtcatactctgtatgataggatgatttttttatgtttgtcttctcaaaatacacttaatggagcatgtccaaccagtgagaatcctagcagttcatcggtcagtggcgaaacaaatataacattacaatttacggaaaaaagaagtttaattaaaagagagctacaaattaaaggctataaacgattattgttcaaaggtgctaactgcccatcctacctaacacttaactcagctcattatacctgcaatagaaactcggcttcaggtgcaagtttatatttatatattcctgctggcgaactaaaaaatttaccttttggtggtatctgggatgctactctgaagttaagagtaaaaagacgatatgatcagacctatggaacttacactataaatatcactgttaaattaactgataagggaaatattcagatatggttacctcagttcaaaagtgacgctcgcgtcgatcttaacttgcgtccaactggtgggggcacatatattggaagaaattctgttgatatgtgcttttatgatggatatagtactaacagcagctctttggagctaagatttcaggataacaatcctaaatctgatgggaaattttatctaaggaaaataaatgatgacaccaaagaaattgcatatactttgtcacttctcttggcgggtaaaagtttaactccaacaaatggaacgtcattaaatattgctgacgcagcttctctggaaataaactggaatagaattacagctgtcaccatgccagaaatcagtgttccggtgttgtgttggcctggacgtttgcaattggatgcaaaagtggaaaatcccgaggccggacaatatatgggtaatattaatattactttcacaccaagtagtcaaacactctag

SEQ ID NO: 71 - protein, 361 aa, Escherichia coli
MNKILFIFTLFFSSVLFTFAVSADKIPGDENITNIFGPRDRNESSPKHNILNDYITAYSESHTLYDRMIFLCLSSQNTLNGACPTSENPSSSSVSGETNITLQFTEKRSLIKRELQIKGYKRLLFKGANCPSYLTLNSAHYTCNRNSASGASLYLYIPAGELKNLPFGGIWDATLKLRVKRRYDQTYGTYTINITVKLTDKGNIQIWLPQFKSDARVDLNLRPTGGGTYIGRNSVDMCFYDGYSTNSSSLELRFQDNNPKSDGKFYLRKINDDTKEIAYTLSLLLAGKSLTPTNGTSLNIADAASLEINWNRITAVTMPEISVPVLCWPGRLQLDAKVENPEAGQYMGNINITFTPSSQTL

SEQ ID NO: 72 - DNA, 516 bp, Escherichia coli
  source 1..516: mol_type = unassigned DNA
atgaaactaaagaaaacaattggcgcaatggctctggcgacattatttgcaactatgggagcatctgcggtcgagaagaccattagcgttacggcgagtgttgacccgactgttgaccttctgcaatctgatggctctgcgctgccgaactctgtcgcattaacctattctccggctgtaaataattttgaagctcacaccatcaacaccgttgttcatacaaatgactcagataaaggtgttgttgtgaagctgtcagcagatccagtcctgtccaatgttctgaatccaaccctgcaaattcctgtttctgtgaatttcgcaggaaaaccactgagcacaacaggcattaccatcgactccaatgatctgaactttgcttcgagtggtgttaataaagtttcttctacgcagaaactttcaatccatgcagatgctactcgggtaactggcggcgcactaacagctggtcaatatcagggactcgtatcaattatcctgactaagtcaacgtaa

SEQ ID NO: 73 - protein, 171 aa, Escherichia coli
MKLKKTIGAMALATLFATMGASAVEKTISVTASVDPTVDLLQSDGSALPNSVALTYSPAVNNFEAHTINTVVHTNDSDKGVVVKLSADPVLSNVLNPTLQIPVSVNFAGKPLSTTGITIDSNDLNFASSGVNKVSSTQKLSIHADATRVTGGALTAGQYQGLVSIILTKST

SEQ ID NO: 74 - DNA, 1092 bp, Escherichia coli
  source 1..1092: mol_type = unassigned DNA
atgaaaaagatatttatttttttgtctatcatattttctgcggtggtcagtgccgggcgatacccggaaactacagtaggtaatctgacgaagagttttcaagcccctcgtctggatagaagcgtacaatcaccaatatataacatctttacgaatcatgtggctggatatagtttgagtcatagcttatatgacaggattgtttttttatgtacatcctcgtcgaatccggttaatggtgcttgcccaaccattggaacatctggagttcaatacggtactacaaccataaccttgcagtttacagaaaaaagaagtctgataaaaagaaatattaatcttgcaggtaataagaaaccaatatgggagaatcagagttgcgactttagcaatctaatggtgttgaattcgaagtcttggagctgtggggcttacggaaatgctaacggaacacttctaaatctgtatatccctgcaggagaaatcaacaaattgccttttggagggatatgggaggcaactctgatcttacgcttatcaagatatggcgaagtcagtagcacccattacggcaattataccgtaaatattacggttgatttaactgataaaggtaatattcaggtatggcttccagggtttcacagcaacccgcgtgtagacctgaatctgcgccctatcggtaattataaatatagtggtagtaattcactcgacatgtgtttctatgatggatatagtacaaacagtgatagcatggtaataaagttccaggatgataatcctaccaattcatctgaatataatctttataagatagggggcactgaaaaattaccatatgctgtttcactgcttatgggagaaaaaatattttatccagtgaatggtcaatcatttactatcaatgacagtagtgtactcgaaacaaactggaatcgagtaaccgcagttgctatgccggaagttaatgttccagtattatgctggccagcaagattgctattaaatgctgatgtaaatgctcccgatgcaggacagtattcaggacagatatatataacatttacacccagtgtcgaaaatttatga

SEQ ID NO: 75 - protein, 363 aa, Escherichia coli
MKKIFIFLSIIFSAVVSAGRYPETTVGNLTKSFQAPRLDRSVQSPIYNIFTNHVAGYSLSHSLYDRIVFLCTSSSNPVNGACPTIGTSGVQYGTTTITLQFTEKRSLIKRNINLAGNKKPIWENQSCDFSNLMVLNSKSWSCGAYGNANGTLLNLYIPAGEINKLPFGGIWEATLILRLSRYGEVSSTHYGNYTVNITVDLTDKGNIQVWLPGFHSNPRVDLNLRPIGNYKYSGSNSLDMCFYDGYSTNSDSMVIKFQDDNPTNSSEYNLYKIGGTEKLPYAVSLLMGEKIFYPVNGQSFTINDSSVLETNWNRVTAVAMPEVNVPVLCWPARLLLNADVNAPDAGQYSGQIYITFTPSVENL

SEQ ID NO: 76 - DNA, 501 bp, Escherichia coli
  source 1..501: mol_type = unassigned DNA
atgaaactgaagaaaacaattggcgcaatggctatggcgactctgtttgccaccatggctgcctctgcagtcgaaaaaaatattactgtgagggcaagtgttgaccctaaacttgatcttctgcaagcagatggaacttcactgccggactctatcgcattaacctattcttcggcttcaaataattttgaagtttactctcttaatactgctattcatacaaatgacaaaaccaaggcagttgtagtgaagctgtcagctccagcagttctgtccaatattatgaagccaagctcgcaaattccgatgaaagtgactttgggggggaagacgctgagtacagctgatgctgagtttgctgctgatactctgaactttggtgcatctggtgttgaaaacgtttcttccgttcaacagcttacgattcatgcagaagctgctccgcctgaggcaggtaattaccaaggtgttatttctcttatcatgactcaaaaaacttaa

SEQ ID NO: 77 - protein, 166 aa, Escherichia coli
MKLKKTIGAMAMATLFATMAASAVEKNITVRASVDPKLDLLQADGTSLPDSIALTYSSASNNFEVYSLNTAIHTNDKTKAVVVKLSAPAVLSNIMKPSSQIPMKVTLGGKTLSTADAEFAADTLNFGASGVENVSSVQQLTIHAEAAPPEAGNYQGVISLIMTQKT

SEQ ID NO: 78 - DNA, 1092 bp, Escherichia coli
  source 1..1092: mol_type = unassigned DNA
atgaaaaagatatttatttttttgtctatcatattttctgcggtggtcagtgccgggcgatacccggaaactacagtaggtaatctgacgaagagttttcaagcccctcgtctggatagaagcgtacaatcaccaatatataacatctttacgaatcatgtggctggatatagtttgagtcatagattatatgacaggattgtttttgtatgtacatcctcgtcgaatccggttaatggtgcttgcccaaccattggaacatctagagttgaatacggtactacaaccataaccttgcagtttacagaaaaaagaagtctgataaaaagaaatattaatcttgcaggtaataagaaaccaatatgggagaatcagagttgcgacactagcaatctaatggtgttgaattcgaagtcttggtcctgtggggctctaggaaatgctaacggaacacttctaaatctgtatatccctgcaggagaaatcaacaaattgccttttggagggatatgggaggcaactctgatcttacgcttatcaagatatggcgaagtcagtagcacccattacggcaattataccgtaaatattacggttgatttaactgataaaggtaatattcaggtatggcttccagggtttcacagcaacccgcgtgtagacctgaatctgcaccctatcggtaattataaatatagtggtagtaattcactcgacatgtgtttctatgatggatatagtacaaacagtgatagcatggtaataaagttccaggatgataatcctaccaattcatctgaatataatctttataagatagggggcactgaaaaattaccatatgctgtttcactgcttatgggaggaaaaatattttatccagtgaatggtcaatcatttactatcaatgacagtagtgtactcgaaacaaactggaatcgagtaaccgcagttgctatgccggaagttaatgttccagtattatgctggccagcaagattgctattaaatgctgatgtaaatgctcccgatgcaggacagtattcaggacagatatatataacatttacacccagtgtcgaaaatttatga

SEQ ID NO: 79 - protein, 363 aa, Escherichia coli
MKKIFIFLSIIFSAVVSAGRYPETTVGNLTKSFQAPRLDRSVQSPIYNIFTNHVAGYSLSHRLYDRIVFVCTSSSNPVNGACPTIGTSRVEYGTTTITLQFTEKRSLIKRNINLAGNKKPIWENQSCDTSNLMVLNSKSWSCGALGNANGTLLNLYIPAGEINKLPFGGIWEATLILRLSRYGEVSSTHYGNYTVNITVDLTDKGNIQVWLPGFHSNPRVDLNLHPIGNYKYSGSNSLDMCFYDGYSTNSDSMVIKFQDDNPTNSSEYNLYKIGGTEKLPYAVSLLMGGKIFYPVNGQSFTINDSSVLETNWNRVTAVAMPEVNVPVLCWPARLLLNADVNAPDAGQYSGQIYITFTPSVENL

SEQ ID NO: 80 - DNA, 513 bp, Escherichia coli
  source 1..513: mol_type = unassigned DNA
atgaaactaaagaaaacaattggcgcaatggctctggcgacattatttgcaaccatgggagcatctgcggtcgagaagaccattagcgttacggcgagtgttgacccgactgttgaccttctgcaatctgatggctctgcgctgccgaactctgtcgcattaacctattctccggctgtagggggttttgaagctcacaccatcaacaccgttgttcatacaaatgacccagctaaaggtgttattgtgaagctgtcagcagaaccagtcctgtccaatgtactgaatccaaccctgcaaattcctgtttctgtgaatttcgcaggaaaaaaactgaccacaacaggcactaccatcgaatccaataaactgaactttgcttcgagtggtgttgataaagtttcttctacgcagaaactttcaatccatgcagatactactcaggtaactggcggactaacagctggtcaatatcaggggctcgtatcaattatcctgactcagtcaacgtaa

SEQ ID NO: 81 - protein, 170 aa, Escherichia coli
MKLKKTIGAMALATLFATMGASAVEKTISVTASVDPTVDLLQSDGSALPNSVALTYSPAVGGFEAHTINTVVHTNDPAKGVIVKLSAEPVLSNVLNPTLQIPVSVNFAGKKLTTTGTTIESNKLNFASSGVDKVSSTQKLSIHADTTQVTGGLTAGQYQGLVSIILTQST

SEQ ID NO: 82 - DNA, 1092 bp, Escherichia coli
  source 1..1092: mol_type = unassigned DNA
atgaaaaagatatttatttttttgtctatcatattttctgcggtggtcagtgccgggcgatacccggaaactacagtaggtaatctgacgaagagttttcaagcccctcgtctggatagaagcgtacaatcaccaatatataacatctttacgaatcatgtggctggatatagtttgagtcatagattatatgacaggattgtttttgtatgtacatcctcgtcgaatccggttaatggtgcttgcccaaccattggaacatctggagttgaatacggtactacaaccataaccttgcagtttacagaaaaaagaagtctgataaaaagaaatattaatcttgcaggtaataagaaaccaatatgggagaatcagagttgcgactttagcaatctaatggtgttgaattcgaagtcttggtcctgtggggctcaaggaaatgctaacggaacacttctaaatctgtatatccctgcaggagaaatcaacaaattgccttttggagggatatgggaggcaactctgatcttacgcttatcaagatatggcgaagtcagtagcacccattacggcaattataccgtaaatattacggttgatttaactgataaaggtaatattcaggtatggcttccagggtttcacagcaacccgcgtgtagacctgaatctgcaccctatcggtaattataaatatagtggtagtaattcactcgacatgtgtttctatgatggatatagtacaaacagtgatagcatggtaataaagttccaggatgataatcctaccaattcatctgaatataatctttataagagagggggcactgaaaaattaccatatgctgtttcactgcttatgggaggaaaaatattttatccagtgaatggtcaatcatttactatcaatgacagtagtgtactcgaaacaaactggaatcgagtaaccgcagttgctatgccggaagttaatgttccagtattatgctggccagcaagattgctattaaatgctgatgtaaatgctcccgatgcaggacagtattcaggacagatatatataacatttacacccagtgtcgaaaatttatga

SEQ ID NO: 83 - protein, 363 aa, Escherichia coli
MKKIFIFLSIIFSAVVSAGRYPETTVGNLTKSFQAPRLDRSVQSPIYNIFTNHVAGYSLSHRLYDRIVFVCTSSSNPVNGACPTIGTSGVEYGTTTITLQFTEKRSLIKRNINLAGNKKPIWENQSCDFSNLMVLNSKSWSCGAQGNANGTLLNLYIPAGEINKLPFGGIWEATLILRLSRYGEVSSTHYGNYTVNITVDLTDKGNIQVWLPGFHSNPRVDLNLHPIGNYKYSGSNSLDMCFYDGYSTNSDSMVIKFQDDNPTNSSEYNLYKRGGTEKLPYAVSLLMGGKIFYPVNGQSFTINDSSVLETNWNRVTAVAMPEVNVPVLCWPARLLLNADVNAPDAGQYSGQIYITFTPSVENL

SEQ ID NO: 84 - DNA, 507 bp, Escherichia coli
  source 1..507: mol_type = unassigned DNA
atgttaaaaataaaatacttattaataggtctttcactgtcagctatgagttcatactcactagctgcagcggggcccactctaaccaaagaactggcattaaatgtgctttctcctgcagctctggatgcaacttgggctcctcaggataatttaacattatccaatactggcgtttctaatactttggtgggtgttttgactctttcaaataccagtattgatacagttagcattgcgagtacaaatgtttctgatacatctaagaatggtacagtaacttttgcacatgagacaaataactctgctagctttgccaccaccatttcaacagataatgccaacattacgttggataaaaatgctggaaatacgattgttaaaactacaaatgggagtcagttgccaactaatttaccacttaagtttattaccactgaaggtaacgaacatttagtttcaggtaattaccgtgcaaatataacaattacttcgacaattaaataa

SEQ ID NO: 85 - protein, 168 aa, Escherichia coli
MLKIKYLLIGLSLSAMSSYSLAAAGPTLTKELALNVLSPAALDATWAPQDNLTLSNTGVSNTLVGVLTLSNTSIDTVSIASTNVSDTSKNGTVTFAHETNNSASFATTISTDNANITLDKNAGNTIVKTTNGSQLPTNLPLKFITTEGNEHLVSGNYRANITITSTIK

SEQ ID NO: 86 - DNA, 480 bp, Escherichia coli
  source 1..480: mol_type = unassigned DNA
atgattttagcattgactttgatgtcggtgtggggaggtgcgtttgccgcagtgggcccaacgaaagatatgagtttaggtgcaaatttaacttcagagcctacattagctattgattttacgcctattgaaaatatttatgtaggtgccaattatggtaaagatattggaacccttgttttcacaacaaatgatttaacagatattacattgatgtcatctcgcagcgttgttgatggtcgccagactggtttttttaccttcatggactcatcagccacttacaaaattagtacaaaactgggatcatcgaatgatgtaaacattcaagaaattactcaaggagctaaaattactcctgttagtggagagaaaactttgcctaaaaaattcactcttaagctacatgcacacaggagtagcagtacagttccaggtacgtatactgttggtcttaacgtaaccagtaatgttatttaa

SEQ ID NO: 87 - protein, 159 aa, Escherichia coli
MILALTLMSVWGGAFAAVGPTKDMSLGANLTSEPTLAIDFTPIENIYVGANYGKDIGTLVFTTNDLTDITLMSSRSVVDGRQTGFFTFMDSSATYKISTKLGSSNDVNIQEITQGAKITPVSGEKTLPKKFTLKLHAHRSSSTVPGTYTVGLNVTSNVI

SEQ ID NO: 88 - protein, 339 aa, Escherichia coli
ADKIPGDESITNIFGPRDRNESSPKHNILNNHITAYSESHTLYDRMTFLCLSSHNTLNGACPTSENPSSSSVSGETNITLQFTEKRSLIKRELQIKGYKQLLFKSVNCPSGLTLNSAHFNCNKNAASGASLYLYIPAGELKNLPFGGIWDATLKLRVKRRYSETYGTYTINITIKLTDKGNIQIWLPQFKSDARVDLNLRPTGGGTYIGRNSVDMCFYDGYSTNSSSLEIRFQDNNPKSDGKFYLRKINDDTKEIAYTLSLLLAGKSLTPTNGTSLNIADAASLETNWNRITAVTMPEISVPVLCWPGRLQLDAKVENPEAGQYMGNINVTFTPSSQTL

SEQ ID NO: 89 - protein, 144 aa, Escherichia coli
VEKNITVTASVDPTIDILQADGSSLPTAVELTYSPAASRFENYKIATKVHTNVINKNVLVKLVNDPKLTNVLDSTKQLPITVSYGGKTLSTADVTFEPAELNFGTSGVTGVSSSQDLVIGATTAQAPTAGNYSGVVSILMTLAS

SEQ ID NO: 90 - protein, 339 aa, Escherichia coli
ADKIPGDENITNIFGPRDRNESSPKHNILNDYITAYSESHTLYDRMIFLCLSSQNTLNGACPTSENPSSSSVSGETNITLQFTEKRSLIKRELQIKGYKRLLFKGANCPSYLTLNSAHYTCNRNSASGASLYLYIPAGELKNLPFGGIWDATLKLRVKRRYDQTYGTYTINITVKLTDKGNIQIWLPQFKSDARVDLNLRPTGGGTYIGRNSVDMCFYDGYSTNSSSLELRFQDNNPKSDGKFYLRKINDDTKEIAYTLSLLLAGKSLTPTNGTSLNIADAASLEINWNRITAVTMPEISVPVLCWPGRLQLDAKVENPEAGQYMGNINITFTPSSQTL

SEQ ID NO: 91 - protein, 152 aa, Escherichia coli
VEKNITVTASVDPTIDILQANGSALPTAVDLTYLPGAKTFENYSVLTQIYTNDPSKGLDVRLVDTPKLTNILQPTSTIPLTVSWAGKTLSTSAQKIAVGDLGFGSTGTAGVSNSKELVIGATTSGTAPSAGKYQGVVSIVMTQSTDTAAPVP

SEQ ID NO: 92 - protein, 146 aa, Escherichia coli
VEKNITVTASVDPTIDILQANGSALPTAVDLTYLPGAKTFENYSVLTQIYTNDPSKGLDVRLVDTPKLTNILQPTSTIPLTVSWAGRTLSTSAQKIAVGDLGFGSTGTAGVSNSKELVIGATTSGTAPSAGKYQGVVSIVMTQSTN

SEQ ID NO: 93 - protein, 345 aa, Escherichia coli
GRYPETTVGNLTKSFQAPRLDRSVQSPIYNIFTNHVAGYSLSHSLYDRIVFLCTSSSNPVNGACPTIGTSGVQYGTTTITLQFTEKRSLIKRNINLAGNKKPIWENQSCDFSNLMVLNSKSWSCGAYGNANGTLLNLYIPAGEINKLPFGGIWEATLILRLSRYGEVSSTHYGNYTVNITVDLTDKGNIQVWLPGFHSNPRVDLNLRPIGNYKYSGSNSLDMCFYDGYSTNSDSMVIKFQDDNPTNSSEYNLYKIGGTEKLPYAVSLLMGEKIFYPVNGQSFTINDSSVLETNWNRVTAVAMPEVNVPVLCWPARLLLNADVNAPDAGQYSGQIYITFTPSVENL

SEQ ID NO: 94 - protein, 148 aa, Escherichia coli
VEKTISVTASVDPTVDLLQSDGSALPNSVALTYSPAVNNFEAHTINTVVHTNDSDKGVVVKLSADPVLSNVLNPTLQIPVSVNFAGKPLSTTGITIDSNDLNFASSGVNKVSSTQKLSIHADATRVTGGALTAGQYQGLVSIILTKST

SEQ ID NO: 95 - protein, 345 aa, Escherichia coli
GRYPETTVGNLTKSFQAPRLDRSVQSPIYNIFTNHVAGYSLSHRLYDRIVFVCTSSSNPVNGACPTIGTSRVEYGTTTITLQFTEKRSLIKRNINLAGNKKPIWENQSCDTSNLMVLNSKSWSCGALGNANGTLLNLYIPAGEINKLPFGGIWEATLILRLSRYGEVSSTHYGNYTVNITVDLTDKGNIQVWLPGFHSNPRVDLNLHPIGNYKYSGSNSLDMCFYDGYSTNSDSMVIKFQDDNPTNSSEYNLYKIGGTEKLPYAVSLLMGGKIFYPVNGQSFTINDSSVLETNWNRVTAVAMPEVNVPVLCWPARLLLNADVNAPDAGQYSGQIYITFTPSVENL

SEQ ID NO: 96 - protein, 143 aa, Escherichia coli
VEKNITVRASVDPKLDLLQADGTSLPDSIALTYSSASNNFEVYSLNTAIHTNDKTKAVVVKLSAPAVLSNIMKPSSQIPMKVTLGGKTLSTADAEFAADTLNFGASGVENVSSVQQLTIHAEAAPPEAGNYQGVISLIMTQKT

SEQ ID NO: 97 - protein, 345 aa, Escherichia coli
GRYPETTVGNLTKSFQAPRLDRSVQSPIYNIFTNHVAGYSLSHRLYDRIVFVCTSSSNPVNGACPTIGTSGVEYGTTTITLQFTEKRSLIKRNINLAGNKKPIWENQSCDFSNLMVLNSKSWSCGAQGNANGTLLNLYIPAGEINKLPFGGIWEATLILRLSRYGEVSSTHYGNYTVNITVDLTDKGNIQVWLPGFHSNPRVDLNLHPIGNYKYSGSNSLDMCFYDGYSTNSDSMVIKFQDDNPTNSSEYNLYKRGGTEKLPYAVSLLMGGKIFYPVNGQSFTINDSSVLETNWNRVTAVAMPEVNVPVLCWPARLLLNADVNAPDAGQYSGQIYITFTPSVENL

SEQ ID NO: 98 - protein, 147 aa, Escherichia coli
VEKTISVTASVDPTVDLLQSDGSALPNSVALTYSPAVGGFEAHTINTVVHTNDPAKGVIVKLSAEPVLSNVLNPTLQIPVSVNFAGKKLTTTGTTIESNKLNFASSGVDKVSSTQKLSIHADTTQVTGGLTAGQYQGLVSIILTQST

SEQ ID NO: 99 - protein, 146 aa, Escherichia coli
AAGPTLTKELALNVLSPAALDATWAPQDNLTLSNTGVSNTLVGVLTLSNTSIDTVSIASTNVSDTSKNGTVTFAHETNNSASFATTISTDNANITLDKNAGNTIVKTTNGSQLPTNLPLKFITTEGNEHLVSGNYRANITITSTIK

SEQ ID NO: 100 - protein, 143 aa, Escherichia coli
AVGPTKDMSLGANLTSEPTLAIDFTPIENIYVGANYGKDIGTLVFTTNDLTDITLMSSRSVVDGRQTGFFTFMDSSATYKISTKLGSSNDVNIQEITQGAKITPVSGEKTLPKKFTLKLHAHRSSSTVPGTYTVGLNVTSNVI

SEQ ID NO: 101 - DNA, 1836 bp, Escherichia coli
  source 1..1836: mol_type = unassigned DNA
atgagaacagaaatagcgactaaaaacttcccagtatcaacgactatttcaaaaagtttttttgcacctgaaccacgaatacagccttcttttggtgaaaatgttggaaaggaaggagctttattatttagtgtgaacttaactgttcctgaaaatgtatcccaggtaacggtctaccctgtttatgatgaagattatgggttaggacgactagtaaataccgctgatgcttcccaatcaataatctaccagattgttgatgagaaagggaaaaaaatgttaaaagatcatggtgcagaggttacacctaatcaacaaataacttttaaagcgctgaattatactagcggggaaaaaaaaatatctcctggaatatataacgatcaggttatggttggttactacgtcaacgacaataaacaaggaaactggcaatataaatctctggatgtaaatgtaaatattgagcaaaattttattccagatattgattccgctgttcgtataatacctgttaattacgattcggacccgaaactggattcacagttatatacggttgagatgacgatccctgcaggtgtaagcgcagttaaaatcgcaccaacagatagtctgacatcttctggacagcagatcggaaagctggttaatgtaaacaatccagatcaaaatatgaattattatatcagaaaggattctggcgctggtaactttatggcaggacaaaaaggatcctttcctgtcaaagagaatacgtcatacacattctcagcaatttatactggtggcgaataccctaatagcggatattcgtctggtacttatgcaggaaatttgactgtatcattttacagcaatgacaataaacaaagaacagaaatagcgactaaaaacttcccagtatccacgactatttcaggcacattagctattgattttacgcctattgaaaatatttatgtaggtgccaattatggtaaagatattggaacccttgttttcacaacaaatgatttaacagatattacattgatgtcatctcgcagcgttgttgatggtcgccagactggtttttttaccttcatggactcatcagccacttacaaaattagtacaaaactgggatcatcgaatgatgtaaacattcaagaaattactcaaggagctaaaattactcctgttagtggagagaaaactttgcctaaaaaattcactcttaagctacatgcacacaggagtagcagtacagttccaggtacgtatactgttggtcttaacgtaaccagtaacgttattgataacaagcaggcagcggggcccactctaaccaaagaactggcattaaatgtgctttctcctgcagctctggatgcaacttgggctcctcaggataatttaacattatccaatactggcgtttctaatactttggtgggtgttttgactctttcaaataccagtattgatacagttagcattgcgagtacaaatgtttctgatacatctaagaatggtacagtaacttttgcacatgagacaaataactctgctagctttgccaccaccatttcaacagataatgccaacattacgttggataaaaatgctggaaatacgattgttaaaactacaaatgggagtcagttgccaactaatttaccacttaagtttattaccactgaaggtaacgaacatttagtttcaggtaattaccgtgcaaatataacaattacttcgacaattaaagataacaagcaggcggcaggtccaaccctgactaaggagttagcgctgaacgttctgagcctcgagcaccaccaccaccaccactga

SEQ ID NO: 102 - protein, 611 aa, Escherichia coli
MRTEIATKNFPVSTTISKSFFAPEPRIQPSFGENVGKEGALLFSVNLTVPENVSQVTVYPVYDEDYGLGRLVNTADASQSIIYQIVDEKGKKMLKDHGAEVTPNQQITFKALNYTSGEKKISPGIYNDQVMVGYYVNDNKQGNWQYKSLDVNVNIEQNFIPDIDSAVRIIPVNYDSDPKLDSQLYTVEMTIPAGVSAVKIAPTDSLTSSGQQIGKLVNVNNPDQNMNYYIRKDSGAGNFMAGQKGSFPVKENTSYTFSAIYTGGEYPNSGYSSGTYAGNLTVSFYSNDNKQRTEIATKNFPVSTTISGTLAIDFTPIENIYVGANYGKDIGTLVFTTNDLTDITLMSSRSVVDGRQTGFFTFMDSSATYKISTKLGSSNDVNIQEITQGAKITPVSGEKTLPKKFTLKLHAHRSSSTVPGTYTVGLNVTSNVIDNKQAAGPTLTKELALNVLSPAALDATWAPQDNLTLSNTGVSNTLVGVLTLSNTSIDTVSIASTNVSDTSKNGTVTFAHETNNSASFATTISTDNANITLDKNAGNTIVKTTNGSQLPTNLPLKFITTEGNEHLVSGNYRANITITSTIKDNKQAAGPTLTKELALNVLSLEHHHHHH

SEQ ID NO: 103 - DNA, 2526 bp, Escherichia coli
  source 1..2526: mol_type = unassigned DNA
atgaataaaattttatttatttttacattgtttttttcttcagggttttttacatttgccgtatcggcagataaaaatcccggaagtgaaaacatgactaatactattggtccccatgacagggggggatcttcccccatatataatatcttaaattcctatcttacagcatacaatggaagccatcatctgtatgataggatgagttttttatgtttgtcttctcaaaatacactgaatggagcatgcccaagcagtgatgcccctggcactgctacaattgatggcgaaacaaatataacattacaatttacggaaaaaagaagtctaattaaaagagaactgcaaattaaaggctataaacaatttttgttcaaaaatgctaattgcccatctaaactagcacttaactcatctcattttcaatgtaatagagaacaagcttcaggtgctactttatcgttatacataccagctggtgaattaaataaattaccttttgggggggtctggaatgccgttctgaagctaaatgtaaaaagacgatatgatacaacctatgggacttacactataaacatcacagttaatttaactgataagggaaatattcagatatggttaccacagttcaaaagtaacgctcgtgtcgatcttaacttgcgtccaactggtggtggtacatatatcggaagaaattctgttgatatgtgcttttatgatggatatagtactaacagcagctctttagagataagatttcaggatgataattctaaatctgatggaaaattttatctaaagaaaataaatgatgactccaaagaacttgtatacactttgtcacttctcctggcaggtaaaaatttaacaccaacaaatggacaggcattaaatattaacactgcttctctggaaacaaactggaatagaattacagctgtcaccatgccagaaatcagtgttccggtgttgtgttggcctggacgtttgcaattggatgcaaaagtgaaaaatcccgaggctggacaatatatggggaatattaaaattactttcacaccaagtagtcaaacactcgacaataaacaagtagagaaaaatattactgtaacagctagtgttgatcctgcaattgatcttttgcaagctgatggcaatgctctgccatcagctgtaaagttagcttattctcccgcatcaaaaacttttgaaagttacagagtaatgactcaagttcatacaaacgatgcaactaaaaaagtaattgttaaacttgctgatacaccacagcttacagatgttctgaattcaactgttcaaatgcctatcagtgtgtcatggggaggacaagtattatctacaacagccaaagaatttgaagctgctgctttgggatattctgcatccggtgtaaatggcgtatcatcttctcaagagttagtaattagcgctgcacctaaaactgccggtaccgccccaactgcaggaaactattcaggagtagtatctcttgtaatgactttgggatccgacaataaacaagtagagaaaaatattactgtaacagctagtgtcgaccctactattgatattcttcaagcaaatggttctgcgctaccgacagctgtagatttaacttatctacctggtgcaaaaacttttgaaaattacagtgttctaacccagatttacacaaatgacccttcaaaaggtttagatgttcgactggttgatacaccgaaacttacaaatattttgcaaccgacatctaccattcctcttactgtctcatgggcagggaagacattaagtacaagtgctcagaagattgcagttggcgatctgggttttggttccaccggaacggcaggtgtttcgaatagtaaagaattagtaattggagcaactacatccggaactgcaccaagtgcaggtaagtatcaaggcgtcgtttccattgtaatgactcaatcgaccgacacagccgcgcctgttcctgacaataaacaagtagagaaaaatattactgtgacagccagtgttgatcctactattgacattttgcaagctgatggtagtagtttacctactgctgtagaattaacctattcacctgcggcaagtcgttttgaaaattataaaatcgcaactaaagttcatacaaatgttataaataaaaatgtactagttaagcttgtaaatgatccaaaacttacaaatgttttggattctacaaaacaactccccattactgtatcatatggaggaaagactctatcaaccgcagatgtgacttttgaacctgcagaattaaattttggaacgtcaggtgtaactggtgtatcttcttcccaagatttagtgattggtgcgactacagcacaagcaccaacggcgggaaattatagtggggtcgtttctatcttaatgaccttagcatcagacaataaacaagtggaaaaaaatatcactgtaacagctagtgttgatcctacgctcgagcaccaccaccaccaccactga

SEQ ID NO: 104 - protein, 841 aa, Escherichia coli
MNKILFIFTLFFSSGFFTFAVSADKNPGSENMTNTIGPHDRGGSSPIYNILNSYLTAYNGSHHLYDRMSFLCLSSQNTLNGACPSSDAPGTATIDGETNITLQFTEKRSLIKRELQIKGYKQFLFKNANCPSKLALNSSHFQCNREQASGATLSLYIPAGELNKLPFGGVWNAVLKLNVKRRYDTTYGTYTINITVNLTDKGNIQIWLPQFKSNARVDLNLRPTGGGTYIGRNSVDMCFYDGYSTNSSSLEIRFQDDNSKSDGKFYLKKINDDSKELVYTLSLLLAGKNLTPTNGQALNINTASLETNWNRITAVTMPEISVPVLCWPGRLQLDAKVKNPEAGQYMGNIKITFTPSSQTLDNKQVEKNITVTASVDPAIDLLQADGNALPSAVKLAYSPASKTFESYRVMTQVHTNDATKKVIVKLADTPQLTDVLNSTVQMPISVSWGGQVLSTTAKEFEAAALGYSASGVNGVSSSQELVISAAPKTAGTAPTAGNYSGVVSLVMTLGSDNKQVEKNITVTASVDPTIDILQANGSALPTAVDLTYLPGAKTFENYSVLTQIYTNDPSKGLDVRLVDTPKLTNILQPTSTIPLTVSWAGKTLSTSAQKIAVGDLGFGSTGTAGVSNSKELVIGATTSGTAPSAGKYQGVVSIVMTQSTDTAAPVPDNKQVEKNITVTASVDPTIDILQADGSSLPTAVELTYSPAASRFENYKIATKVHTNVINKNVLVKLVNDPKLTNVLDSTKQLPITVSYGGKTLSTADVTFEPAELNFGTSGVTGVSSSQDLVIGATTAQAPTAGNYSGVVSILMTLASDNKQVEKNITVTASVDPTLEHHHHHH

SEQ ID NO: 105 - DNA, 2164 bp, Escherichia coli
  source 1..2164: mol_type = unassigned DNA
atgaaaaagatatttatttttttgtctatcatattttctgcggtggtcagtgccgggcgatacccggaaactacagtaggtaatctgacgaagagttttcaagcccctcgtcaggatagaagcgtacaatcaccaatatataacatctttacgaatcatgtggctggatatagtttgagtcataacttatatgacaggattgtttttttatgtacatcctcgtcgaatccggttaatggtgcttgcccaaccattggaacatctggagttcaatacggtactacaaccataaccttgcagtttacagaaaaaagaagtctgataaaaagaaatattaatcttgcaggtaataagaaaccaatatgggagaatcagagttgcgacactagcaatctaatggtgttgaattcgaagtcttggtcctgtggggcttacggaaatgctaacggaacacttctaaatctgtatatccctgcaggagaaatcaacaaattgccttttggagggatatgggaggcaactctgatcttacgcttatcaagatatggcgaagtcagtagcacccattacggcaattataccgtaaatattacggttgatttaactgataaaggtaatattcaggtatggcttccagggtttcacagcaacccgcgtgtagacctgaatctgcaccctatcggtaattataaatatagtggtagtaattcactcgacatgtgtttctatgatggatatagtacaaacagtgatagcatggtaataaagttccaggatgataatcctacctattcatctgaatataatctttataagatagggggcactgaaaaattaccctatgctgtttcactgcttatgggagaaaaaatattttatccagtgaatggtcaatcatttactatcaatgacagtagtgtactcgaaacaaactggaatcgagtaaccgcagttgctatgccggaagttaatgttccagtattatgctggccagcaagattgctattaaatgctgatgtaaatgctcccgatgcaggacagtattcaggacagatatatataacatttacacccagtgtcgaaaatttaggcggtggagtcgaaaaaaatattactgtgagggcaagtgttgaccctaaacttgatcttctgcaagcagatggaacttcactgccggactctatcgcattaacctattcttcggcttcaaataattttgaagtttactctcttaatactgctattcatacaaatgacaaaagcaagggagttgtagtgaagctgtcagcttcaccagttctgtccaatattatgaagccaaactcgcaaattccgatgaaagtgactttgggggggaagacgctgaatacaactgatactgagtttactgttgatactctgaactttggtacatctggtgttgaaaacgtttcttccactcaacagcttacgattcatgcagacacacaaggaactgcgcctgaggcaggcaattaccaaggtattatttctcttatcatgactcaaaaaacagggggcggtgtcgaaaaaaatattactgtgagggcaagtgtcgaccctaaacttgaccttctgcaatctgatggctctgcgctgccgaactctgtcgcattaacctattctccggctgtaaataattttgaagctcacaccatcaacaccgttgttcatacaaatgactcagataaaggtgttgttgtgaagctgtcagcagatccagtcctgtccaatgttctgaatccaaccctgcaaattcctgtttctgtgaatttcgcaggaaaaccactgagcacaacaggcattaccatcgactccaatgatctgaactttgcttcgagtggtgttaataaagtttcttctacgcagaaactttcaatccatgcagatgctactcgggtaactggcggcgcactaacagctggtcaatatcagggactcgtatcaattatcctgactaagtcaacggggggcggtgtcgagaagaccattagcgttacggcgagtgttgacccgacgggcacattagctattgattttacgcctattgaaaatatttatgtaggtgccaattatggtaaagatattggaacccttgttttcacaacaaatgatttaactcgagcaccaccaccaccaccactga

SEQ ID NO: 106 - protein, 687 aa, Escherichia coli
MKKIFIFLSIIFSAVVSAGRYPETTVGNLTKSFQAPRQDRSVQSPIYNIFTNHVAGYSLSHNLYDRIVFLCTSSSNPVNGACPTIGTSGVQYGTTTITLQFTEKRSLIKRNINLAGNKKPIWENQSCDTSNLMVLNSKSWSCGAYGNANGTLLNLYIPAGEINKLPFGGIWEATLILRLSRYGEVSSTHYGNYTVNITVDLTDKGNIQVWLPGFHSNPRVDLNLHPIGNYKYSGSNSLDMCFYDGYSTNSDSMVIKFQDDNPTYSSEYNLYKIGGTEKLPYAVSLLMGEKIFYPVNGQSFTINDSSVLETNWNRVTAVAMPEVNVPVLCWPARLLLNADVNAPDAGQYSGQIYITFTPSVENLGGGVEKNITVRASVDPKLDLLQADGTSLPDSIALTYSSASNNFEVYSLNTAIHTNDKSKGVVVKLSASPVLSNIMKPNSQIPMKVTLGGKTLNTTDTEFTVDTLNFGTSGVENVSSTQQLTIHADTQGTAPEAGNYQGIISLIMTQKTGGGVEKNITVRASVDPKLDLLQSDGSALPNSVALTYSPAVNNFEAHTINTVVHTNDSDKGVVVKLSADPVLSNVLNPTLQIPVSVNFAGKPLSTTGITIDSNDLNFASSGVNKVSSTQKLSIHADATRVTGGALTAGQYQGLVSIILTKSTGGGVEKTISVTASVDPTLEHHHHHH

SEQ ID NO: 107 - DNA, 2278 bp, Escherichia coli
  source 1..2278: mol_type = unassigned DNA
atgaaaaagatatttatttttttgtctatcatattttctgcggtggtcagtgccgggcgatacccggaaactacagtaggtaatctgacgaagagttttcaagcccctcgtcaggatagaagcgtacaatcaccaatatataacatctttacgaatcatgtggctggatatagtttgagtcataacttatatgacaggattgtttttttatgtacatcctcgtcgaatccggttaatggtgcttgcccaaccattggaacatctggagttcaatacggtactacaaccataaccttgcagtttacagaaaaaagaagtctgataaaaagaaatattaatcttgcaggtaataagaaaccaatatgggagaatcagagttgcgacactagcaatctaatggtgttgaattcgaagtcttggtcctgtggggcttacggaaatgctaacggaacacttctaaatctgtatatccctgcaggagaaatcaacaaattgccttttggagggatatgggaggcaactctgatcttacgcttatcaagatatggcgaagtcagtagcacccattacggcaattataccgtaaatattacggttgatttaactgataaaggtaatattcaggtatggcttccagggtttcacagcaacccgcgtgtagacctgaatctgcaccctatcggtaattataaatatagtggtagtaattcactcgacatgtgtttctatgatggatatagtacaaacagtgatagcatggtaataaagttccaggatgataatcctacctattcatctgaatataatctttataagatagggggcactgaaaaattaccctatgctgtttcactgcttatgggagaaaaaatattttatccagtgaatggtcaatcatttactatcaatgacagtagtgtactcgaaacaaactggaatcgagtaaccgcagttgctatgccggaagttaatgttccagtattatgctggccagcaagattgctattaaatgctgatgtaaatgctcccgatgcaggacagtattcaggacagatatatataacatttacacccagtgtcgaaaatttaggcggtggagtcgaaaaaaatattactgtgagggcaagtgttgaccctaaacttgatcttctgcaagcagatggaacttcactgccggactctatcgcattaacctattcttcggcttcaaataattttgaagtttactctcttaatactgctattcatacaaatgacaaaagcaagggagttgtagtgaagctgtcagcttcaccagttctgtccaatattatgaagccaaactcgcaaattccgatgaaagtgactttgggggggaagacgctgaatacaactgatactgagtttactgttgatactctgaactttggtacatctggtgttgaaaacgtttcttccactcaacagcttacgattcatgcagacacacaaggaactgcgcctgaggcaggcaattaccaaggtattatttctcttatcatgactcaaaaaacagggggcggtgtcgaaaaaaatattactgtgagggcaagtgtcgaccctaaacttaaactaaagaaaacaattggcgcaatggctctggcgacattatttgcaactatgggagcatctgcggtcgagaagaccattagcgttacggcgagtgttgacccgactgttgaccttctgcaatctgatggctctgcgctgccgaactctgtcgcattaacctattctccggctgtaaataattttgaagctcacaccatcaacaccgttgttcatacaaatgactcagataaaggtgttgttgtgaagctgtcagcagatccagtcctgtccaatgttctgaatccaaccctgcaaattcctgtttctgtgaatttcgcaggaaaaccactgagcacaacaggcattaccatcgactccaatgatctgaactttgcttcgagtggtgttaataaagtttcttctacgcagaaactttcaatccatgcagatgctactcgggtaactggcggcgcactaacagctggtcaatatcagggactcgtatcaattatcctgactaagtcaacgtaagggggcggtgtcgagaagaccattagcgttacggcgagtgttgacccgacgggcacattagctattgattttacgcctattgaaaatatttatgtaggtgccaattatggtaaagatattggaacccttgttttcacaacaaatgatttaactcgagcaccaccaccaccaccactga

SEQ ID NO: 108 - protein, 703 aa, Escherichia coli
MKKIFIFLSIIFSAVVSAGRYPETTVGNLTKSFQAPRQDRSVQSPIYNIFTNHVAGYSLSHNLYDRIVFLCTSSSNPVNGACPTIGTSGVQYGTTTITLQFTEKRSLIKRNINLAGNKKPIWENQSCDTSNLMVLNSKSWSCGAYGNANGTLLNLYIPAGEINKLPFGGIWEATLILRLSRYGEVSSTHYGNYTVNITVDLTDKGNIQVWLPGFHSNPRVDLNLHPIGNYKYSGSNSLDMCFYDGYSTNSDSMVIKFQDDNPTYSSEYNLYKIGGTEKLPYAVSLLMGEKIFYPVNGQSFTINDSSVLETNWNRVTAVAMPEVNVPVLCWPARLLLNADVNAPDAGQYSGQIYITFTPSVENLGGGVEKNITVRASVDPKLDLLQADGTSLPDSIALTYSSASNNFEVYSLNTAIHTNDKSKGVVVKLSASPVLSNIMKPNSQIPMKVTLGGKTLNTTDTEFTVDTLNFGTSGVENVSSTQQLTIHADTQGTAPEAGNYQGIISLIMTQKTGGGVEKNITVRASVDPKLDVEKTISVTASVDPTVDLLQSDGSALPNSVALTYSPAVNNFEAHTINTVVHTNDSDKGVVVKLSADPVLSNVLNPTLQIPVSVNFAGKPLSTTGITIDSNDLNFASSGVNKVSSTQKLSIHADATRVTGGALTAGQYQGLVSIILTKSTGGGVEKTISVTASVDPTLEHHHHHH

SEQ ID NO: 109 - DNA, 1620 bp, Escherichia coli
  source 1..1620: mol_type = unassigned DNA
atgaaaaaagtgatttttgttttatccatgtttctatgttctcaggtttacgggcaatcatggcatacgaacgtagaggctggttcaataaataaaacagagtcgataggccccatagaccgaagtgctgctgcatcgtatcctgctcattatatatttcatgaacatgttgctggttacaataaagatcactctctttttgacaggatgacgtttttatgtatgtcatcaacagatgcatctaaaggtgcatgtccgacaggagaaaactccaaatcctctcaaggggagactaatattaagctaatatttactgaaaagaaaagtctggccagaaaaacattaaacttaaaaggatataagagatttttatatgaatcagatagatgcattcattatgtcgataaaatgaatctcaattctcatactgttaaatgtgtaggttcattcacaagaggagtagatttcactttatatatcccacaaggtgaaattgatgggcttctaactggaggtatatgggaggcaacactagagttacgagtcaaaaggcattacgactataatcatggtacttacaaagttaatatcacagttgatttgacagacaaaggaaatattcaggtctggacaccaaagtttcatagcgatcctagaattgatctgaatttacgtcctgaaggtaatggtaaatattctggtagtaacgtgcttgagatgtgtctctatgatggctatagtacacatagtcaaagtatagaaatgaggtttcaggatgactcacaaacaggaaataatgaatataatcttataaaaactggagagccattaaaaaaattgccatataaactttctcttcttttaggaggacgagagttttatccaaataatggagaggcttttactattaatgatacttcgtcattgtttataaactggaatcgtattaagtctgtatccttaccacagattagtattccagtactatgctggccagcaaacttgacatttatgtcagagctaaataatccagaagcgggtgagtattcaggaatacttaacgtaacatttactcctagtagttcaagcctagacaataaacaagccgagaaaaatatcactgtaactgctagcgttgatccaactatcgatctgatgcaatctgatggcacagcgttaccaagtgcagttaatattgcatatcttccaggagagaaaagatttgaatctgctcgtatcaatacccaagttcataccaataataaaactaagggtattcagataaagcttactaatgataatgtggtaatgactaacttatctgatccaagcaagactattcctttagaggtttcattcgctggcactaagctgagcacagctgcaacatctattactgccgatcaattaaattttggcgcagctggtgtagagacagtttctgcaactaaggaactcgttattaatgcaggaagcacccagcaaactaatattgtagctggtaactatcaaggattggtgtcaattgtgcttactcaagaacctgacaataaacaagccgagaaaaatatcactgtaactgctagcgttgatccgacgcaccaccaccaccaccactga

SEQ ID NO: 110 - protein, 539 aa, Escherichia coli
MKKVIFVLSMFLCSQVYGQSWHTNVEAGSINKTESIGPIDRSAAASYPAHYIFHEHVAGYNKDHSLFDRMTFLCMSSTDASKGACPTGENSKSSQGETNIKLIFTEKKSLARKTLNLKGYKRFLYESDRCIHYVDKMNLNSHTVKCVGSFTRGVDFTLYIPQGEIDGLLTGGIWEATLELRVKRHYDYNHGTYKVNITVDLTDKGNIQVWTPKFHSDPRIDLNLRPEGNGKYSGSNVLEMCLYDGYSTHSQSIEMRFQDDSQTGNNEYNLIKTGEPLKKLPYKLSLLLGGREFYPNNGEAFTINDTSSLFINWNRIKSVSLPQISIPVLCWPANLTFMSELNNPEAGEYSGILNVTFTPSSSSLDNKQAEKNITVTASVDPTIDLMQSDGTALPSAVNIAYLPGEKRFESARINTQVHTNNKTKGIQIKLTNDNVVMTNLSDPSKTIPLEVSFAGTKLSTAATSITADQLNFGAAGVETVSATKELVINAGSTQQTNIVAGNYQGLVSIVLTQEPDNKQAEKNITVTASVDPTHHHHHH

SEQ ID NO: 111 - DNA, 2490 bp, Escherichia coli
  source 1..2490: mol_type = unassigned DNA
atgaataaaattttatttatttttacattgtttttttcttcagggttttttacatttgccgtatcggcagataaaaatcccggaagtgaaaacatgactaatactattggtccccatgacagggggggatcttcccccatatataatatcttaaattcctatcttacagcatacaatggaagccatcatctgtatgataggatgagttttttatgtttgtcttctcaaaatacactgaatggagcatgcccaagcagtgatgcccctggcactgctacaattgatggcgaaacaaatataacattacaatttacggaaaaaagaagtctaattaaaagagaactgcaaattaaaggctataaacaatttttgttcaaaaatgctaattgcccatctaaactagcacttaactcatctcattttcaatgtaatagagaacaagcttcaggtgctactttatcgttatacataccagctggtgaattaaataaattaccttttgggggggtctggaatgccgttctgaagctaaatgtaaaaagacgatatgatacaacctatgggacttacactataaacatcacagttaatttaactgataagggaaatattcagatatggttaccacagttcaaaagtaacgctcgtgtcgatcttaacttgcgtccaactggtggtggtacatatatcggaagaaattctgttgatatgtgcttttatgatggatatagtactaacagcagctctttagagataagatttcaggatgataattctaaatctgatggaaaattttatctaaagaaaataaatgatgactccaaagaacttgtatacactttgtcacttctcctggcaggtaaaaatttaacaccaacaaatggacaggcattaaatattaacactgcttctctggaaacaaactggaatagaattacagctgtcaccatgccagaaatcagtgttccggtgttgtgttggcctggacgtttgcaattggatgcaaaagtgaaaaatcccgaggctggacaatatatggggaatattaaaattactttcacaccaagtagtcaaacactcgacaataaacaagtagagaaaaatattactgtaacagctagtgttgatcctgcaattgatcttttgcaagctgatggcaatgctctgccatcagctgtaaagttagcttattctcccgcatcaaaaacttttgaaagttacagagtaatgactcaagttcatacaaacgatgcaactaaaaaagtaattgttaaacttgctgatacaccacagcttacagatgttctgaattcaactgttcaaatgcctatcagtgtgtcatggggaggacaagtattatctacaacagccaaagaatttgaagctgctgctttgggatattctgcatccggtgtaaatggcgtatcatcttctcaagagttagtaattagcgctgcacctaaaactgccggtaccgccccaactgcaggaaactattcaggagtagtatctcttgtaatgactttgggatccgacaataaacaagtagagaaaaatattactgtaacagctagtgtcgaccctgcagggtcaaaaagtttttttgcacctgaaccacgaatacagccttcttttggtgaaaatgttggaaaggaaggagctttattatttagtgtgaacttaactgttcctgaaaatgtatcccaggtaacggtctaccctgtttatgatgaagattatgggttaggacgactagtaaataccgctgatgcttcccaatcaataatctaccagattgttgatgagaaagggaaaaaaatgttaaaagatcatggtgcagaggttacacctaatcaacaaataacttttaaagcgctgaattatactagcggggaaaaaaaaatatctcctggaatatataacgatcaggttatggttggttactacgtcaacgacaataaacaaggaaactggcaatataaatctctggatgtaaatgtaaatattgagcaaaattttattccagatattgattccgctgttcgtataatacctgttaattacgattcggacccgaaactggattcacagttatatacggttgagatgacgatccctgcaggtgtaagcgcagttaaaatcgcaccaacagatagtctgacatcttctggacagcagatcggaaagctggttaatgtaaacaatccagatcaaaatatgaattattatatcagaaaggattctggcgctggtaactttatggcaggacaaaaaggatcctttcctgtcaaagagaatacgtcatacacattctcagcaatttatactggtggcgaataccctaatagcggatattcgtctggtacttatgcaggaaatttgactgtatcattttacagcaatgacaataaacaacgtaccgagattgccaccaagaattttccggtgagcaccaccatcagcctcgagcaccaccaccaccaccactga

SEQ ID NO: 112 - protein, 829 aa, Escherichia coli
MNKILFIFTLFFSSGFFTFAVSADKNPGSENMTNTIGPHDRGGSSPIYNILNSYLTAYNGSHHLYDRMSFLCLSSQNTLNGACPSSDAPGTATIDGETNITLQFTEKRSLIKRELQIKGYKQFLFKNANCPSKLALNSSHFQCNREQASGATLSLYIPAGELNKLPFGGVWNAVLKLNVKRRYDTTYGTYTINITVNLTDKGNIQIWLPQFKSNARVDLNLRPTGGGTYIGRNSVDMCFYDGYSTNSSSLEIRFQDDNSKSDGKFYLKKINDDSKELVYTLSLLLAGKNLTPTNGQALNINTASLETNWNRITAVTMPEISVPVLCWPGRLQLDAKVKNPEAGQYMGNIKITFTPSSQTLDNKQVEKNITVTASVDPAIDLLQADGNALPSAVKLAYSPASKTFESYRVMTQVHTNDATKKVIVKLADTPQLTDVLNSTVQMPISVSWGGQVLSTTAKEFEAAALGYSASGVNGVSSSQELVISAAPKTAGTAPTAGNYSGVVSLVMTLGSDNKQVEKNITVTASVDPAGSKSFFAPEPRIQPSFGENVGKEGALLFSVNLTVPENVSQVTVYPVYDEDYGLGRLVNTADASQSIIYQIVDEKGKKMLKDHGAEVTPNQQITFKALNYTSGEKKISPGIYNDQVMVGYYVNDNKQGNWQYKSLDVNVNIEQNFIPDIDSAVRIIPVNYDSDPKLDSQLYTVEMTIPAGVSAVKIAPTDSLTSSGQQIGKLVNVNNPDQNMNYYIRKDSGAGNFMAGQKGSFPVKENTSYTFSAIYTGGEYPNSGYSSGTYAGNLTVSFYSNDNKQRTEIATKNFPVSTTISLEHHHHHH

SEQ ID NO: 113 - DNA, 2487 bp, Escherichia coli
  source 1..2487: mol_type = unassigned DNA
atgaataaaattttatttatttttacattgtttttttcttcagggttttttacatttgccgtatcggcagataaaaatcccggaagtgaaaacatgactaatactattggtccccatgacagggggggatcttcccccatatataatatcttaaattcctatcttacagcatacaatggaagccatcatctgtatgataggatgagttttttatgtttgtcttctcaaaatacactgaatggagcatgcccaagcagtgatgcccctggcactgctacaattgatggcgaaacaaatataacattacaatttacggaaaaaagaagtctaattaaaagagaactgcaaattaaaggctataaacaatttttgttcaaaaatgctaattgcccatctaaactagcacttaactcatctcattttcaatgtaatagagaacaagcttcaggtgctactttatcgttatacataccagctggtgaattaaataaattaccttttgggggggtctggaatgccgttctgaagctaaatgtaaaaagacgatatgatacaacctatgggacttacactataaacatcacagttaatttaactgataagggaaatattcagatatggttaccacagttcaaaagtaacgctcgtgtcgatcttaacttgcgtccaactggtggtggtacatatatcggaagaaattctgttgatatgtgcttttatgatggatatagtactaacagcagctctttagagataagatttcaggatgataattctaaatctgatggaaaattttatctaaagaaaataaatgatgactccaaagaacttgtatacactttgtcacttctcctggcaggtaaaaatttaacaccaacaaatggacaggcattaaatattaacactgcttctctggaaacaaactggaatagaattacagctgtcaccatgccagaaatcagtgttccggtgttgtgttggcctggacgtttgcaattggatgcaaaagtgaaaaatcccgaggctggacaatatatggggaatattaaaattactttcacaccaagtagtcaaacactcgacaataaacaagtagagaaaaatattactgtaacagctagtgttgatcctgcaattgatcttttgcaagctgatggcaatgctctgccatcagctgtaaagttagcttattctcccgcatcaaaaacttttgaaagttacagagtaatgactcaagttcatacaaacgatgcaactaaaaaagtaattgttaaacttgctgatacaccacagcttacagatgttctgaattcaactgttcaaatgcctatcagtgtgtcatggggaggacaagtattatctacaacagccaaagaatttgaagctgctgctttgggatattctgcatccggtgtaaatggcgtatcatcttctcaagagttagtaattagcgctgcacctaaaactgccggtaccgccccaactgcaggaaactattcaggagtagtatctcttgtaatgactttgggatccgacaataaacaagtagagaaaaatattactgtaacagctagtgtcgaccctgcagggaattttattccagatattgattccgctgttcgtataatacctgttaattacgattcggacccgaaactggattcacagttatatacggttgagatgacgatccctgcaggtgtaagcgcagttaaaatcgcaccaacagatagtctgacatcttctggacagcagatcggaaagctggttaatgtaaacaatccagatcaaaatatgaattattatatcagaaaggattctggcgctggtaactttatggcaggacaaaaaggatcctttcctgtcaaagagaatacgtcatacacattctcagcaatttatactggtggcgaataccctaatagcggatattcgtctggtacttatgcaggaaatttgactgtatcattttacagcaatgacaataaacaaagaacagaaatagcgactaaaaacttcccagtatcaacgactatttcaaaaagtttttttgcacctgaaccacgaatacagccttcttttggtgaaaatgttggaaaggaaggagctttattatttagtgtgaacttaactgttcctgaaaatgtatcccaggtaacggtctaccctgtttatgatgaagattatgggttaggacgactagtaaataccgctgatgcttcccaatcaataatctaccagattgttgatgagaaagggaaaaaaatgttaaaagatcatggtgcagaggttacacctaatcaacaaataacttttaaagcgctgaattatactagcggggaaaaaaaaatatctcctggaatatataacgatcaggttatggttggttactacgtaaacgacaataaacaaaccgagattgccaccaagaattttccggtgagcaccaccatcagcctcctcgagcaccaccaccaccaccactga

SEQ ID NO: 114 - protein, 828 aa, Escherichia coli
MNKILFIFTLFFSSGFFTFAVSADKNPGSENMTNTIGPHDRGGSSPIYNILNSYLTAYNGSHHLYDRMSFLCLSSQNTLNGACPSSDAPGTATIDGETNITLQFTEKRSLIKRELQIKGYKQFLFKNANCPSKLALNSSHFQCNREQASGATLSLYIPAGELNKLPFGGVWNAVLKLNVKRRYDTTYGTYTINITVNLTDKGNIQIWLPQFKSNARVDLNLRPTGGGTYIGRNSVDMCFYDGYSTNSSSLEIRFQDDNSKSDGKFYLKKINDDSKELVYTLSLLLAGKNLTPTNGQALNINTASLETNWNRITAVTMPEISVPVLCWPGRLQLDAKVKNPEAGQYMGNIKITFTPSSQTLDNKQVEKNITVTASVDPAIDLLQADGNALPSAVKLAYSPASKTFESYRVMTQVHTNDATKKVIVKLADTPQLTDVLNSTVQMPISVSWGGQVLSTTAKEFEAAALGYSASGVNGVSSSQELVISAAPKTAGTAPTAGNYSGVVSLVMTLGSDNKQVEKNITVTASVDPAGNFIPDIDSAVRIIPVNYDSDPKLDSQLYTVEMTIPAGVSAVKIAPTDSLTSSGQQIGKLVNVNNPDQNMNYYIRKDSGAGNFMAGQKGSFPVKENTSYTFSAIYTGGEYPNSGYSSGTYAGNLTVSFYSNDNKQRTEIATKNFPVSTTISKSFFAPEPRIQPSFGENVGKEGALLFSVNLTVPENVSQVTVYPVYDEDYGLGRLVNTADASQSIIYQIVDEKGKKMLKDHGAEVTPNQQITFKALNYTSGEKKISPGIYNDQVMVGYYVNDNKQGNWQYKSLDVNVNIEQLEHHHHHH

SEQ ID NO: 115 - DNA, 1014 bp, Escherichia coli
  source 1..1014: mol_type = unassigned DNA
gcagataaaaatcccggaagtgaaaacatgactaatactattggtccccatgacagggggggatcttcccccatatataatatcttaaattcctatcttacagcatacaatggaagccatcatctgtatgataggatgagttttttatgtttgtcttctcaaaatacactgaatggagcatgcccaagcagtgatgcccctggcactgctacaattgatggcgaaacaaatataacattacaatttacggaaaaaagaagtctaattaaaagagaactgcaaattaaaggctataaacaatttttgttcaaaaatgctaattgcccatctaaactagcacttaactcatctcattttcaatgtaatagagaacaagcttcaggtgctactttatcgttatacataccagctggtgaattaaataaattaccttttgggggggtctggaatgccgttctgaagctaaatgtaaaaagacgatatgatacaacctatgggacttacactataaacatcacagttaatttaactgataagggaaatattcagatatggttaccacagttcaaaagtaacgctcgtgtcgatcttaacttgcgtccaactggtggtggtacatatatcggaagaaattctgttgatatgtgcttttatgatggatatagtactaacagcagctctttagagataagatttcaggatgataattctaaatctgatggaaaattttatctaaagaaaataaatgatgactccaaagaacttgtatacactttgtcacttctcctggcaggtaaaaatttaacaccaacaaatggacaggcattaaatattaacactgcttctctggaaacaaactggaatagaattacagctgtcaccatgccagaaatcagtgttccggtgttgtgttggcctggacgtttgcaattggatgcaaaagtgaaaaatcccgaggctggacaatatatggggaatattaaaattactttcacaccaagtagtcaaacactc

SEQ ID NO: 116 - DNA, 441 bp, Escherichia coli
  source 1..441: mol_type = unassigned DNA
gtagagaaaaatattactgtaacagctagtgttgatcctgcaattgatcttttgcaagctgatggcaatgctctgccatcagctgtaaagttagcttattctcccgcatcaaaaacttttgaaagttacagagtaatgactcaagttcatacaaacgatgcaactaaaaaagtaattgttaaacttgctgatacaccacagcttacagatgttctgaattcaactgttcaaatgcctatcagtgtgtcatggggaggacaagtattatctacaacagccaaagaatttgaagctgctgctttgggatattctgcatccggtgtaaatggcgtatcatcttctcaagagttagtaattagcgctgcacctaaaactgccggtaccgccccaactgcaggaaactattcaggagtagtatctcttgtaatgactttgggatcc

SEQ ID NO: 117 - DNA, 1020 bp, Escherichia coli
  source 1..1020: mol_type = unassigned DNA
gcagataaaattcccggagatgaaagcataactaatatttttggcccgcgtgacaggaacgaatcttcccccaaacataatatattaaataaccatattacagcatacagtgaaagtcatactctgtatgataggatgacttttttatgtttgtcttctcacaatacacttaatggagcatgtccaaccagtgagaatcctagcagttcatcggtcagcggtgaaacaaatataacattacaatttacggaaaaaagaagtttaataaaaagagagctacaaattaaaggctataaacaattattgttcaaaagtgttaactgcccatccggcctaacacttaactcagctcattttaactgtaataaaaacgcggcttcaggtgcaagtttatatttatatattcctgctggcgaactaaaaaatttgccttttggtggtatctgggatgctactctgaagttaagagtaaaaagacgatatagtgagacctatggaacttacactataaatatcactattaaattaactgataagggaaatattcagatatggttacctcagttcaaaagtgacgctcgcgtcgatcttaacttgcgtccaactggtgggggcacatatattggaagaaattctgttgatatgtgcttttatgatggatatagtactaacagcagctctttggagataagatttcaggataacaatcctaaatctgatgggaaattttatctaaggaaaataaatgatgacaccaaagaaattgcatatactttgtcacttctcttggcgggtaaaagtttaactccaacaaatggaacgtcattaaatattgctgacgcagcttctctggaaacaaactggaatagaattacagctgtcaccatgccagaaatcagtgttccggtgttgtgttggcctggacgtttgcaattggatgcaaaagtggaaaatcccgaggctggacaatatatgggtaatattaatgttactttcacaccaagtagtcaaacactctag

SEQ ID NO: 118 - DNA, 435 bp, Escherichia coli
  source 1..435: mol_type = unassigned DNA
gtagagaaaaatatcactgtaacagctagtgttgatcctacaattgatattttgcaagctgatggtagtagtttacctactgctgtagaattaacctattcacctgcggcaagtcgttttgaaaattataaaatcgcaactaaagttcatacaaatgttataaataaaaatgtactagttaagcttgtaaatgatccaaaacttacaaatgttttggattctacaaaacaactccccattactgtatcatatggaggaaagactctatcaaccgcagatgtgacttttgaacctgcagaattaaattttggaacgtcaggtgtaactggtgtatcttcttcccaagatttagtgattggtgcgactacagcacaagcaccaacggcgggaaattatagtggggtcgtttctatcttaatgaccttagcatcataa

SEQ ID NO: 119 - DNA, 1020 bp, Escherichia coli
  source 1..1020: mol_type = unassigned DNA
gcagataaaattcccggagatgagaatataactaatatttttggcccgcgtgacaggaacgaatcttcccccaaacataatatattaaatgactatattacagcatacagtgaaagtcatactctgtatgataggatgatttttttatgtttgtcttctcaaaatacacttaatggagcatgtccaaccagtgagaatcctagcagttcatcggtcagtggcgaaacaaatataacattacaatttacggaaaaaagaagtttaattaaaagagagctacaaattaaaggctataaacgattattgttcaaaggtgctaactgcccatcctacctaacacttaactcagctcattatacctgcaatagaaactcggcttcaggtgcaagtttatatttatatattcctgctggcgaactaaaaaatttaccttttggtggtatctgggatgctactctgaagttaagagtaaaaagacgatatgatcagacctatggaacttacactataaatatcactgttaaattaactgataagggaaatattcagatatggttacctcagttcaaaagtgacgctcgcgtcgatcttaacttgcgtccaactggtgggggcacatatattggaagaaattctgttgatatgtgcttttatgatggatatagtactaacagcagctctttggagctaagatttcaggataacaatcctaaatctgatgggaaattttatctaaggaaaataaatgatgacaccaaagaaattgcatatactttgtcacttctcttggcgggtaaaagtttaactccaacaaatggaacgtcattaaatattgctgacgcagcttctctggaaataaactggaatagaattacagctgtcaccatgccagaaatcagtgttccggtgttgtgttggcctggacgtttgcaattggatgcaaaagtggaaaatcccgaggccggacaatatatgggtaatattaatattactttcacaccaagtagtcaaacactctag

SEQ ID NO: 120 - DNA, 459 bp, Escherichia coli
  source 1..459: mol_type = unassigned DNA
gtagagaaaaatattactgtgacagccagtgttgatcctactattgatattcttcaagcaaatggttctgcgctaccgacagctgtagatttaacttatctacctggtgcaaaaacttttgaaaattacagtgttctaacccagatttacacaaatgacccttcaaaaggtttagatgttcgactggttgatacaccgaaacttacaaatattttgcaaccgacatctaccattcctcttactgtctcatgggcagggaagacattaagtacaagtgctcagaagattgcagttggcgatctgggttttggttccaccggaacggcaggtgtttcgaatagtaaagaattagtaattggagcaactacatccggaactgcaccaagtgcaggtaagtatcaaggcgtcgtttccattgtaatgactcaatcgacagacacagccgcgcctgttccttaa

SEQ ID NO: 121 - DNA, 441 bp, Escherichia coli
  source 1..441: mol_type = unassigned DNA
gtagagaaaaatattactgtgacagccagtgttgatcctactattgatattcttcaagcaaatggttctgcgctaccgacagctgtagatttaacttatctacctggtgcaaaaacttttgaaaattacagtgttctaacccagatttacacaaatgacccttcaaaaggtttagatgttcgactggttgatacaccgaaacttacaaatattttgcaaccgacatctaccattcctcttactgtctcatgggcagggaggacattaagtacaagtgctcagaagatcgcagttggcgatctgggttttggttccaccggaacggcaggtgtttcgaatagtaaagaattagtaattggagcaactacatccggaactgcaccaagtgcaggtaagtatcaaggcgtcgtttccattgtaatgactcaatcgacaaactaa

SEQ ID NO: 122 - DNA, 1038 bp, Escherichia coli
  source 1..1038: mol_type = unassigned DNA
gggcgatacccggaaactacagtaggtaatctgacgaagagttttcaagcccctcgtctggatagaagcgtacaatcaccaatatataacatctttacgaatcatgtggctggatatagtttgagtcatagcttatatgacaggattgtttttttatgtacatcctcgtcgaatccggttaatggtgcttgcccaaccattggaacatctggagttcaatacggtactacaaccataaccttgcagtttacagaaaaaagaagtctgataaaaagaaatattaatcttgcaggtaataagaaaccaatatgggagaatcagagttgcgactttagcaatctaatggtgttgaattcgaagtcttggagctgtggggcttacggaaatgctaacggaacacttctaaatctgtatatccctgcaggagaaatcaacaaattgccttttggagggatatgggaggcaactctgatcttacgcttatcaagatatggcgaagtcagtagcacccattacggcaattataccgtaaatattacggttgatttaactgataaaggtaatattcaggtatggcttccagggtttcacagcaacccgcgtgtagacctgaatctgcgccctatcggtaattataaatatagtggtagtaattcactcgacatgtgtttctatgatggatatagtacaaacagtgatagcatggtaataaagttccaggatgataatcctaccaattcatctgaatataatctttataagatagggggcactgaaaaattaccatatgctgtttcactgcttatgggagaaaaaatattttatccagtgaatggtcaatcatttactatcaatgacagtagtgtactcgaaacaaactggaatcgagtaaccgcagttgctatgccggaagttaatgttccagtattatgctggccagcaagattgctattaaatgctgatgtaaatgctcccgatgcaggacagtattcaggacagatatatataacatttacacccagtgtcgaaaatttatga

SEQ ID NO: 123 - DNA, 447 bp, Escherichia coli
  source 1..447: mol_type = unassigned DNA
gtcgagaagaccattagcgttacggcgagtgttgacccgactgttgaccttctgcaatctgatggctctgcgctgccgaactctgtcgcattaacctattctccggctgtaaataattttgaagctcacaccatcaacaccgttgttcatacaaatgactcagataaaggtgttgttgtgaagctgtcagcagatccagtcctgtccaatgttctgaatccaaccctgcaaattcctgtttctgtgaatttcgcaggaaaaccactgagcacaacaggcattaccatcgactccaatgatctgaactttgcttcgagtggtgttaataaagtttcttctacgcagaaactttcaatccatgcagatgctactcgggtaactggcggcgcactaacagctggtcaatatcagggactcgtatcaattatcctgactaagtcaacgtaa

SEQ ID NO: 124 - DNA, 1038 bp, Escherichia coli
  source 1..1038: mol_type = unassigned DNA
gggcgatacccggaaactacagtaggtaatctgacgaagagttttcaagcccctcgtctggatagaagcgtacaatcaccaatatataacatctttacgaatcatgtggctggatatagtttgagtcatagattatatgacaggattgtttttgtatgtacatcctcgtcgaatccggttaatggtgcttgcccaaccattggaacatctagagttgaatacggtactacaaccataaccttgcagtttacagaaaaaagaagtctgataaaaagaaatattaatcttgcaggtaataagaaaccaatatgggagaatcagagttgcgacactagcaatctaatggtgttgaattcgaagtcttggtcctgtggggctctaggaaatgctaacggaacacttctaaatctgtatatccctgcaggagaaatcaacaaattgccttttggagggatatgggaggcaactctgatcttacgcttatcaagatatggcgaagtcagtagcacccattacggcaattataccgtaaatattacggttgatttaactgataaaggtaatattcaggtatggcttccagggtttcacagcaacccgcgtgtagacctgaatctgcaccctatcggtaattataaatatagtggtagtaattcactcgacatgtgtttctatgatggatatagtacaaacagtgatagcatggtaataaagttccaggatgataatcctaccaattcatctgaatataatctttataagatagggggcactgaaaaattaccatatgctgtttcactgcttatgggaggaaaaatattttatccagtgaatggtcaatcatttactatcaatgacagtagtgtactcgaaacaaactggaatcgagtaaccgcagttgctatgccggaagttaatgttccagtattatgctggccagcaagattgctattaaatgctgatgtaaatgctcccgatgcaggacagtattcaggacagatatatataacatttacacccagtgtcgaaaatttatga

SEQ ID NO: 125 - DNA, 432 bp, Escherichia coli
  source 1..432: mol_type = unassigned DNA
gtcgaaaaaaatattactgtgagggcaagtgttgaccctaaacttgatcttctgcaagcagatggaacttcactgccggactctatcgcattaacctattcttcggcttcaaataattttgaagtttactctcttaatactgctattcatacaaatgacaaaaccaaggcagttgtagtgaagctgtcagctccagcagttctgtccaatattatgaagccaagctcgcaaattccgatgaaagtgactttgggggggaagacgctgagtacagctgatgctgagtttgctgctgatactctgaactttggtgcatctggtgttgaaaacgtttcttccgttcaacagcttacgattcatgcagaagctgctccgcctgaggcaggtaattaccaaggtgttatttctcttatcatgactcaaaaaacttaa

SEQ ID NO: 126 - DNA, 444 bp, Escherichia coli
  source 1..444: mol_type = unassigned DNA
gtcgagaagaccattagcgttacggcgagtgttgacccgactgttgaccttctgcaatctgatggctctgcgctgccgaactctgtcgcattaacctattctccggctgtagggggttttgaagctcacaccatcaacaccgttgttcatacaaatgacccagctaaaggtgttattgtgaagctgtcagcagaaccagtcctgtccaatgtactgaatccaaccctgcaaattcctgtttctgtgaatttcgcaggaaaaaaactgaccacaacaggcactaccatcgaatccaataaactgaactttgcttcgagtggtgttgataaagtttcttctacgcagaaactttcaatccatgcagatactactcaggtaactggcggactaacagctggtcaatatcaggggctcgtatcaattatcctgactcagtcaacgtaa

SEQ ID NO: 127 - DNA, 1038 bp, Escherichia coli
  source 1..1038: mol_type = unassigned DNA
gggcgatacccggaaactacagtaggtaatctgacgaagagttttcaagcccctcgtcaggatagaagcgtacaatcaccaatatataacatctttacgaatcatgtggctggatatagtttgagtcataacttatatgacaggattgtttttttatgtacatcctcgtcgaatccggttaatggtgcttgcccaaccattggaacatctggagttcaatacggtactacaaccataaccttgcagtttacagaaaaaagaagtctgataaaaagaaatattaatcttgcaggtaataagaaaccaatatgggagaatcagagttgcgacactagcaatctaatggtgttgaattcgaagtcttggtcctgtggggcttacggaaatgctaacggaacacttctaaatctgtatatccctgcaggagaaatcaacaaattgccttttggagggatatgggaggcaactctgatcttacgcttatcaagatatggcgaagtcagtagcacccattacggcaattataccgtaaatattacggttgatttaactgataaaggtaatattcaggtatggcttccagggtttcacagcaacccgcgtgtagacctgaatctgcaccctatcggtaattataaatatagtggtagtaattcactcgacatgtgtttctatgatggatatagtacaaacagtgatagcatggtaataaagttccaggatgataatcctacctattcatctgaatataatctttataagatagggggcactgaaaaattaccatatgctgtttcactgcttatgggagaaaaaatattttatccagtgaatggtcaatcatttactatcaatgacagtagtgtactcgaaacaaactggaatcgagtaaccgcagttgctatgccggaagttaatgttccagtattatgctggccagcaagattgctattaaatgctgatgtaaatgctcccgatgcaggacagtattcaggacagatatatataacatttacacccagtgtcgaaaatttatga

SEQ ID NO: 128 - DNA, 438 bp, Escherichia coli
  source 1..438: mol_type = unassigned DNA
gtcgaaaaaaatattactgtgagggcaagtgttgaccctaaacttgatcttctgcaagcagatggaacttcactgccggactctatcgcattaacctattcttcggcttcaaataattttgaagtttactctcttaatactgctattcatacaaatgacaaaagcaagggagttgtagtgaagctgtcagcttcaccagttctgtccaatattatgaagccaaactcgcaaattccgatgaaagtgactttgggggggaagacgctgaatacaactgatactgagtttactgttgatactctgaactttggtacatctggtgttgaaaacgtttcttccactcaacagcttacgattcatgcagacacacaaggaactgcgcctgaggcaggcaattaccaaggtattatttctcttatcatgactcaaaaaacttaa

SEQ ID NO: 129 - DNA, 1041 bp, Escherichia coli
  source 1..1041: mol_type = unassigned DNA
caatcatggcatacgaacgtagaggctggttcaataaataaaacagagtcgataggccccatagaccgaagtgctgctgcatcgtatcctgctcattatatatttcatgaacatgttgctggttacaataaagatcactctctttttgacaggatgacgtttttatgtatgtcatcaacagatgcatctaaaggtgcatgtccgacaggagaaaactccaaatcctctcaaggggagactaatattaagctaatatttactgaaaagaaaagtctggccagaaaaacattaaacttaaaaggatataagagatttttatatgaatcagatagatgcattcattatgtcgataaaatgaatctcaattctcatactgttaaatgtgtaggttcattcacaagaggagtagatttcactttatatatcccacaaggtgaaattgatgggcttctaactggaggtatatgggaggcaacactagagttacgagtcaaaaggcattacgactataatcatggtacttacaaagttaatatcacagttgatttgacagacaaaggaaatattcaggtctggacaccaaagtttcatagcgatcctagaattgatctgaatttacgtcctgaaggtaatggtaaatattctggtagtaacgtgcttgagatgtgtctctatgatggctatagtacacatagtcaaagtatagaaatgaggtttcaggatgactcacaaacaggaaataatgaatataatcttataaaaactggagagccattaaaaaaattgccatataaactttctcttcttttaggaggacgagagttttatccaaataatggagaggcttttactattaatgatacttcgtcattgtttataaactggaatcgtattaagtctgtatccttaccacagattagtattccagtactatgctggccagcaaacttgacatttatgtcagagctaaataatccagaagcgggtgagtattcaggaatacttaacgtaacatttactcctagtagttcaagtctgtaa

SEQ ID NO: 130 - DNA, 444 bp, Escherichia coli
  source 1..444: mol_type = unassigned DNA
gccgagaaaaatatcactgtaactgctagcgttgatccaactatcgatctgatgcaatctgatggcacagcgttaccaagtgcagttaatattgcatatcttccaggagagaaaagatttgaatctgctcgtatcaatacccaagttcataccaataataaaactaagggtattcagataaagcttactaatgataatgtggtaatgactaacttatctgatccaagcaagactattcctttagaggtttcattcgctggcactaagctgagcacagctgcaacatctattactgccgatcaattaaattttggcgcagctggtgtagagacagtttctgcaactaaggaactcgttattaatgcaggaagcacccagcaaactaatattgtagctggtaactatcaaggattggtgtcaattgtgcttactcaagaaccttaa

SEQ ID NO: 131 - DNA, 441 bp, Escherichia coli
  source 1..441: mol_type = unassigned DNA
gcagcggggcccactctaaccaaagaactggcattaaatgtgctttctcctgcagctctggatgcaacttgggctcctcaggataatttaacattatccaatactggcgtttctaatactttggtgggtgttttgactctttcaaataccagtattgatacagttagcattgcgagtacaaatgtttctgatacatctaagaatggtacagtaacttttgcacatgagacaaataactctgctagctttgccaccaccatttcaacagataatgccaacattacgttggataaaaatgctggaaatacgattgttaaaactacaaatgggagtcagttgccaactaatttaccacttaagtttattaccactgaaggtaacgaacatttagtttcaggtaattaccgtgcaaatataacaattacttcgacaattaaataa

SEQ ID NO: 132 - DNA, 432 bp, Escherichia coli
  source 1..432: mol_type = unassigned DNA
gcagtgggcccaacgaaagatatgagtttaggtgcaaatttaacttcagagcctacattagctattgattttacgcctattgaaaatatttatgtaggtgccaattatggtaaagatattggaacccttgttttcacaacaaatgatttaacagatattacattgatgtcatctcgcagcgttgttgatggtcgccagactggtttttttaccttcatggactcatcagccacttacaaaattagtacaaaactgggatcatcgaatgatgtaaacattcaagaaattactcaaggagctaaaattactcctgttagtggagagaaaactttgcctaaaaaattcactcttaagctacatgcacacaggagtagcagtacagttccaggtacgtatactgttggtcttaacgtaaccagtaatgttatttaa

SEQ ID NO: 133 - DNA, 1038 bp, Escherichia coli
  source 1..1038: mol_type = unassigned DNA
gggcgatacccggaaactacagtaggtaatctgacgaagagttttcaagcccctcgtctggatagaagcgtacaatcaccaatatataacatctttacgaatcatgtggctggatatagtttgagtcatagattatatgacaggattgtttttgtatgtacatcctcgtcgaatccggttaatggtgcttgcccaaccattggaacatctggagttgaatacggtactacaaccataaccttgcagtttacagaaaaaagaagtctgataaaaagaaatattaatcttgcaggtaataagaaaccaatatgggagaatcagagttgcgactttagcaatctaatggtgttgaattcgaagtcttggtcctgtggggctcaaggaaatgctaacggaacacttctaaatctgtatatccctgcaggagaaatcaacaaattgccttttggagggatatgggaggcaactctgatcttacgcttatcaagatatggcgaagtcagtagcacccattacggcaattataccgtaaatattacggttgatttaactgataaaggtaatattcaggtatggcttccagggtttcacagcaacccgcgtgtagacctgaatctgcaccctatcggtaattataaatatagtggtagtaattcactcgacatgtgtttctatgatggatatagtacaaacagtgatagcatggtaataaagttccaggatgataatcctaccaattcatctgaatataatctttataagagagggggcactgaaaaattaccatatgctgtttcactgcttatgggaggaaaaatattttatccagtgaatggtcaatcatttactatcaatgacagtagtgtactcgaaacaaactggaatcgagtaaccgcagttgctatgccggaagttaatgttccagtattatgctggccagcaagattgctattaaatgctgatgtaaatgctcccgatgcaggacagtattcaggacagatatatataacatttacacccagtgtcgaaaatttatga

SEQ ID NO: 134 - DNA, 465 bp, Escherichia coli
  source 1..465: mol_type = unassigned DNA
atgaagaaaacaattggtttaattctaattcttgcttcattcggcagccatgccagaacagaaatagcgactaaaaacttcccagtatcaacgactatttcaaaaagtttttttgcgcctgaaccacaaatccagccttcttttggtaaaaatgttggaaaggaaggagatttattatttagtgtgagcttaattgttcctgaaaatgtatcccaggtaacggtctaccctgtttatgatgaagattatggattaggacgactcgtaaataccgctgatgattcccaatcaataatctaccagattgttgatgataaagggaaaaaaatgttaaaagatcatggtacagaggttacgcctaatcaacaaataacttttaaagcgctgaattatactagcggagataaagaaatacctcctgggatatataacgatcaggttatggttggttactatgtaaactaa

SEQ ID NO: 135 - protein, 154 aa, Escherichia coli
MKKTIGLILILASFGSHARTEIATKNFPVSTTISKSFFAPEPQIQPSFGKNVGKEGDLLFSVSLIVPENVSQVTVYPVYDEDYGLGRLVNTADDSQSIIYQIVDDKGKKMLKDHGTEVTPNQQITFKALNYTSGDKEIPPGIYNDQVMVGYYVN

SEQ ID NO: 136 - DNA, 504 bp, Escherichia coli
  source 1..504: mol_type = unassigned DNA
atgttgaaaaaaattattccggctattgcattaattgcaggaacttccggagtggtaaatgcaggaaactggcaatataaatctctggatgtaaatgtaaatattgagcaaaattttattccagatattgattccgctgttcgtataatacctgttaattacgattcggatccgaaactgaattcacagttatatacggttgagatgacgatccctgcaggtgtaagcgcagttaaaatcgtaccaacagatagtctgacatcttctggacagcagatcggaaagctggttaatgtaaacaatccagatcaaaatatgaattattatatcagaaaggattctggcgctggtaagtttatggcagggcaaaaaggatccttttctgtcaaagagaatacgtcatacacattctcagcaatttatactggtggcgaataccctaatagcggatattcgtctggtacttatgcaggacatttgactgtatcattttacagcaattaa

SEQ ID NO: 137 - protein, 167 aa, Escherichia coli
MLKKIIPAIALIAGTSGVVNAGNWQYKSLDVNVNIEQNFIPDIDSAVRIIPVNYDSDPKLNSQLYTVEMTIPAGVSAVKIVPTDSLTSSGQQIGKLVNVNNPDQNMNYYIRKDSGAGKFMAGQKGSFSVKENTSYTFSAIYTGGEYPNSGYSSGTYAGHLTVSFYSN

SEQ ID NO: 138 - protein, 384 aa, Escherichia coli
MNKILFIFTLFFSSGFFTFAVSADKNPGSENMTNTIGPHDRGGSSPIYNILNSYLTAYNGSHHLYDRMSFLCLSSQNTLNGACPSSDAPGTATIDGETNITLQFTEKRSLIKRELQIKGYKQFLFKNANCPSKLALNSSHFQCNREQASGATLSLYIPAGELNKLPFGGVWNAVLKLNVKRRYDTTYGTYTINITVNLTDKGNIQIWLPQFKSNARVDLNLRPTGGGTYIGRNSVDMCFYDGYSTNSSSLEIRFQDDNSKSDGKFYLKKINDDSKELVYTLSLLLAGKNLTPTNGQALNINTASLETNWNRITAVTMPEISVPVLCWPGRLQLDAKVKNPEAGQYMGNIKITFTPSSQTLDNKQVEKNITVTASVDPAIDLLQA

SEQ ID NO: 139 - DNA, 1002 bp, Escherichia coli
  source 1..1002: mol_type = unassigned DNA
atgaataaaattttatttatttttacattgtttttttcttcagggttttttacatttgccgtatcggcagataaaaatcccggaagtgaaaacatgactaatactattggtccccatgacagggggggatcttcccccatatataatatcttaaattcctatcttacagcatacaatggaagccatcatctgtatgataggatgagttttttatgtttgtcttctcaaaatacactgaatggagcatgcccaagcagtgatgcccctggcactgctacaattgatggcgaaacaaatataacattacaatttacggaaaaaagaagtctaattaaaagagaactgcaaattaaaggctataaacaatttttgttcaaaaatgctaattgcccatctaaactagcacttaactcatctcattttcaatgtaatagagaacaagcttcaggtgctactttatcgttatacataccagctggtgaattaaataaattaccttttgggggggtctggaatgccgttctgaagctaaatgtaaaaagacgatatgatacaacctatgggacttacactataaacatcacagttaatttaactgataagggaaatattcagatatggttaccacagttcaaaagtaacgctcgtgtcgatcttaacttgcgtccaactggtggtggtacatatatcggaagaaattctgttgatatgtgcttttatgatggatatagtactaacagcagctctttagagataagatttcaggatgataattctaaatctgatggaaaattttatctaaagaaaataaatgatgactccaaagaacttgtatacactttgtcacttctcctggcaggtaaaaatttaacaccaacaaatggacaggcattaaatattaacactgcttctctggaaacaaactggaatagaattacagctgtcaccatgccagaaatcagtgttccggtgttgtgttggcctggacgtttgcaattggat

SEQ ID NO: 140 - DNA, 1629 bp, Escherichia coli
  source 1..1629: mol_type = unassigned DNA
atgaataaaattttatttatttttacattgtttttttcttcagggttttttacatttgccgtatcggcagataaaaatcccggaagtgaaaacatgactaatactattggtccccatgacagggggggatcttcccccatatataatatcttaaattcctatcttacagcatacaatggaagccatcatctgtatgataggatgagttttttatgtttgtcttctcaaaatacactgaatggagcatgcccaagcagtgatgcccctggcactgctacaattgatggcgaaacaaatataacattacaatttacggaaaaaagaagtctaattaaaagagaactgcaaattaaaggctataaacaatttttgttcaaaaatgctaattgcccatctaaactagcacttaactcatctcattttcaatgtaatagagaacaagcttcaggtgctactttatcgttatacataccagctggtgaattaaataaattaccttttgggggggtctggaatgccgttctgaagctaaatgtaaaaagacgatatgatacaacctatgggacttacactataaacatcacagttaatttaactgataagggaaatattcagatatggttaccacagttcaaaagtaacgctcgtgtcgatcttaacttgcgtccaactggtggtggtacatatatcggaagaaattctgttgatatgtgcttttatgatggatatagtactaacagcagctctttagagataagatttcaggatgataattctaaatctgatggaaaattttatctaaagaaaataaatgatgactccaaagaacttgtatacactttgtcacttctcctggcaggtaaaaatttaacaccaacaaatggacaggcattaaatattaacactgcttctctggaaacaaactggaatagaattacagctgtcaccatgccagaaatcagtgttccggtgttgtgttggcctggacgtttgcaattggatgcaaaagtgaaaaatcccgaggctggacaatatatggggaatattaaaattactttcacaccaagtagtcaaacactcgacaataaacaagtagagaaaaatattactgtaacagctagtgttgatcctgcaattgatcttttgcaagctgatggcaatgctctgccatcagctgtaaagttagcttattctcccgcatcaaaaacttttgaaagttacagagtaatgactcaagttcatacaaacgatgcaactaaaaaagtaattgttaaacttgctgatacaccacagcttacagatgttctgaattcaactgttcaaatgcctatcagtgtgtcatggggaggacaagtattatctacaacagccaaagaatttgaagctgctgctttgggatattctgcatccggtgtaaatggcgtatcatcttctcaagagttagtaattagcgctgcacctaaaactgccggtaccgccccaactgcaggaaactattcaggagtagtatctcttgtaatgactttgggatccgacaataaacaagtagagaaaaatattactgtaacagctagtgttgatcctgtgattgatcttttgcaactcgagcaccaccaccaccaccactga

SEQ ID NO: 141 - protein, 542 aa, Escherichia coli
MNKILFIFTLFFSSGFFTFAVSADKNPGSENMTNTIGPHDRGGSSPIYNILNSYLTAYNGSHHLYDRMSFLCLSSQNTLNGACPSSDAPGTATIDGETNITLQFTEKRSLIKRELQIKGYKQFLFKNANCPSKLALNSSHFQCNREQASGATLSLYIPAGELNKLPFGGVWNAVLKLNVKRRYDTTYGTYTINITVNLTDKGNIQIWLPQFKSNARVDLNLRPTGGGTYIGRNSVDMCFYDGYSTNSSSLEIRFQDDNSKSDGKFYLKKINDDSKELVYTLSLLLAGKNLTPTNGQALNINTASLETNWNRITAVTMPEISVPVLCWPGRLQLDAKVKNPEAGQYMGNIKITFTPSSQTLDNKQVEKNITVTASVDPAIDLLQADGNALPSAVKLAYSPASKTFESYRVMTQVHTNDATKKVIVKLADTPQLTDVLNSTVQMPISVSWGGQVLSTTAKEFEAAALGYSASGVNGVSSSQELVISAAPKTAGTAPTAGNYSGVVSLVMTLGSDNKQVEKNITVTASVDPVIDLLQLEHHHHHH

SEQ ID NO: 142 - DNA, 1176 bp, Escherichia coli
  source 1..1176: mol_type = unassigned DNA
atgaataaaattttatttatttttacattgtttttttcttcagggttttttacatttgccgtatcggcagataaaaatcccggaagtgaaaacatgactaatactattggtccccatgacagggggggatcttcccccatatataatatcttaaattcctatcttacagcatacaatggaagccatcatctgtatgataggatgagttttttatgtttgtcttctcaaaatacactgaatggagcatgcccaagcagtgatgcccctggcactgctacaattgatggcgaaacaaatataacattacaatttacggaaaaaagaagtctaattaaaagagaactgcaaattaaaggctataaacaatttttgttcaaaaatgctaattgcccatctaaactagcacttaactcatctcattttcaatgtaatagagaacaagcttcaggtgctactttatcgttatacataccagctggtgaattaaataaattaccttttgggggggtctggaatgccgttctgaagctaaatgtaaaaagacgatatgatacaacctatgggacttacactataaacatcacagttaatttaactgataagggaaatattcagatatggttaccacagttcaaaagtaacgctcgtgtcgatcttaacttgcgtccaactggtggtggtacatatatcggaagaaattctgttgatatgtgcttttatgatggatatagtactaacagcagctctttagagataagatttcaggatgataattctaaatctgatggaaaattttatctaaagaaaataaatgatgactccaaagaacttgtatacactttgtcacttctcctggcaggtaaaaatttaacaccaacaaatggacaggcattaaatattaacactgcttctctggaaacaaactggaatagaattacagctgtcaccatgccagaaatcagtgttccggtgttgtgttggcctggacgtttgcaattggatgcaaaagtgaaaaatcccgaggctggacaatatatggggaatattaaaattactttcacaccaagtagtcaaacactcgacaataaacaagtagagaaaaatattactgtaacagctagtgttgatcctgtgattgatcttttgcaactcgagcaccaccaccaccaccactga

SEQ ID NO: 143 - protein, 391 aa, Escherichia coli
MNKILFIFTLFFSSGFFTFAVSADKNPGSENMTNTIGPHDRGGSSPIYNILNSYLTAYNGSHHLYDRMSFLCLSSQNTLNGACPSSDAPGTATIDGETNITLQFTEKRSLIKRELQIKGYKQFLFKNANCPSKLALNSSHFQCNREQASGATLSLYIPAGELNKLPFGGVWNAVLKLNVKRRYDTTYGTYTINITVNLTDKGNIQIWLPQFKSNARVDLNLRPTGGGTYIGRNSVDMCFYDGYSTNSSSLEIRFQDDNSKSDGKFYLKKINDDSKELVYTLSLLLAGKNLTPTNGQALNINTASLETNWNRITAVTMPEISVPVLCWPGRLQLDAKVKNPEAGQYMGNIKITFTPSSQTLDNKQVEKNITVTASVDPVIDLLQLEHHHHHH